European Patent Specification EP 3 865 147 B1, published August 27, 2025. Title: BI-SPECIFIC THERAPEUTIC PROTEINS FOR TISSUE REPAIR. Applicant: Silver Creek Pharmaceuticals, Inc. Application EP. The sequence listing filed with the application follows.

SEQUENCE LISTING (138 sequences)

SEQ ID NO: 1 - protein, 319 aa, Homo sapiens
AQVLRGTVTDFPGFDERADAETLRKAMKGLGTDEESILTLLTSRSNAQRQEISAAFKTLFGRDLLDDLKSELTGKFEKLIVALMKPSRLYDAYELKHALKGAGTNEKVLTEIIASRTPEELRAIKQVYEEEYGSSLEDDVVGDTSGYYQRMLVVLLQANRDPDAGIDEAQVEQDAQALFQAGELKWGTDEEKFITIFGTRSVSHLRKVFDKYMTISGFQIEETIDRETSGNLEQLLLAVVKSIRSIPAYLAETLYYAMKGAGTDDHTLIRVMVSRSEIDLFNIRKEFRKNFATSLYSMIKGDTSGDYKKALLLLCGEDD

SEQ ID NO: 2 - protein, 319 aa, Artificial Sequence
  Synthetic construct
AQVLRGTVTDFPGFDERADAETLRKAMKGLGTDEESILTLLTSRSNAQRQEISAAFKTLFGRDLLDDLKSELTGKFEKLIVALMKPSRLYDAYELKHALKGAGTNEKVLTEIIASRTPEELRAIKQVYEEEYGSSLEDDVVGDTSGYYQRMLVVLLQANRDPDAGIDEAQVEQDAQALFQAGELKWGTDEEKFITIFGTRSVSHLRKVFDKYMTISGFQIEETIDRETSGNLEQLLLAVVKSIRSIPAYLAETLYYAMKGAGTDDHTLIRVMVSRSEIDLFNIRKEFRKNFATSLYSMIKGDTSGDYKKALLLLSGEDD

SEQ ID NO: 3 - protein, 333 aa, Artificial Sequence
  Synthetic construct
AQVLRGTVTDFPGFDERADAETLRKAMKGLGTDEESILTLLTSRSNAQRQEISAAFKTLFGRDLLDDLKSELTGKFEKLIVALMKPSRLYDAYELKHALKGAGTNEKVLTEIIASRTPEELRAIKQVYEEEYGSSLEDDVVGDTSGYYQRMLVVLLQANRDPDAGIDEAQVEQDAQALFQAGELKWGTDEEKFITIFGTRSVSHLRKVFDKYMTISGFQIEETIDRETSGNLEQLLLAVVKSIRSIPAYLAETLYYAMKGAGTDDHTLIRVMVSRSEIDLFNIRKEFRKNFATSLYSMIKGDTSGDYKKALLLLSGEDDGSGGSGSGHHHHHH

SEQ ID NO: 4 - protein, 319 aa, Artificial Sequence
  Synthetic construct
AQVLRGTVTDFPGFDERADAETLRKAMKGLGTDEESILTLLTSRSNAQRQEISAAFKTLFGADLLDDLASELTGKFEKLIVALMKPSRLYDAYELKHALAGAGTNEKVLTEIIASRTPEELRAIKQVYEEEYGSSLAGDVVGDTSGYYQRMLVVLLQAARDPDAGIDEAQVEQDAQALFQAGELKWGTDEEKFITIFGTRSVSHLRKVFDKYMTISGFQIEETIDRETSGNLEQLLLAVVKSIRSIPAYLAETLYYAMKGAGTDDHTLIRVMVSRSEIDLFNIRKEFRKNFATSLYSMIKGDTSGDYKKALLLLCGEDD

SEQ ID NO: 5 - DNA, 960 bp, Homo sapiens
gctcaagtcttgcgtggtacggtgacagacttcccaggcttcgatgaaagagcggacgcggaaacacttcgaaaggcgatgaaagggctcggtactgacgaagagtccattttgacccttcttacgagcaggtcaaacgctcagaggcaagaaatctctgcagcctttaagacactctttggacgtgaccttcttgatgacctcaaatctgagctgacgggaaagtttgagaaactcatcgtagctttgatgaagcccagccgattgtatgatgcttacgaactgaaacacgccctgaaaggagcgggaacgaacgagaaagttttgactgagatcatcgcatcgcggaccccggaagagctcagagccatcaaacaagtctacgaggaggagtacggatcgtcattggaagatgacgtggtgggggatacgtcgggttactaccaacgaatgcttgtcgtgcttttgcaggcaaatcgcgacccggatgcggggatcgacgaggcccaagtggagcaagatgcgcaagcactcttccaggccggtgaactcaaatgggggaccgatgaagagaagtttatcaccatctttggcacgaggagtgtaagtcatctgcgtaaagtattcgataagtatatgacaatctcagggtttcagattgaggagacaattgacagggaaacctccggtaacttggagcagctcttgcttgccgtcgtcaagtccattcgctcgatccctgcgtatctggctgaaacactgtattacgccatgaaaggggcaggcactgatgaccacaccttgattagagttatggtgtcgcgatcagaaattgacttgttcaatatccggaaagagttccggaagaatttcgcaacgagcctctatagcatgatcaaaggggacacttcgggagattacaagaaagcgttgctccttctttgcggagaggatgactaa

SEQ ID NO: 6 - DNA, 963 bp, Artificial Sequence
  Synthetic construct
gctcaagtcttgcgtggtacggtgacagacttcccaggcttcgatgaaagagcggacgcggaaacacttcgaaaggcgatgaaagggctcggtactgacgaagagtccattttgacccttcttacgagcaggtcaaacgctcagaggcaagaaatctctgcagcctttaagacactctttggacgtgaccttcttgatgacctcaaatctgagctgacgggaaagtttgagaaactcatcgtagctttgatgaagcccagccgattgtatgatgcttacgaactgaaacacgccctgaaaggagcgggaacgaacgagaaagttttgactgagatcatcgcatcgcggaccccggaagagctcagagccatcaaacaagtctacgaggaggagtacggatcgtcattggaagatgacgtggtgggggatacgtcgggttactaccaacgaatgcttgtcgtgcttttgcaggcaaatcgcgacccggatgcggggatcgacgaggcccaagtggagcaagatgcgcaagcactcttccaggccggtgaactcaaatgggggaccgatgaagagaagtttatcaccatctttggcacgaggagtgtaagtcatctgcgtaaagtattcgataagtatatgacaatctcagggtttcagattgaggagacaattgacagggaaacctccggtaacttggagcagctcttgcttgccgtcgtcaagtccattcgctcgatccctgcgtatctggctgaaacactgtattacgccatgaaaggggcaggcactgatgaccacaccttgattagagttatggtgtcgcgatcagaaattgacttgttcaatatccggaaagagttccggaagaatttcgcaacgagcctctatagcatgatcaaaggggacacttcgggagattacaagaaagcgttgctccttctttcaggagaggatgactaatga

SEQ ID NO: 7 - DNA, 1005 bp, Artificial Sequence
  Synthetic construct
gctcaagtcttgcgtggtacggtgacagacttcccaggcttcgatgaaagagcggacgcggaaacacttcgaaaggcgatgaaagggctcggtactgacgaagagtccattttgacccttcttacgagcaggtcaaacgctcagaggcaagaaatctctgcagcctttaagacactctttggacgtgaccttcttgatgacctcaaatctgagctgacgggaaagtttgagaaactcatcgtagctttgatgaagcccagccgattgtatgatgcttacgaactgaaacacgccctgaaaggagcgggaacgaacgagaaagttttgactgagatcatcgcatcgcggaccccggaagagctcagagccatcaaacaagtctacgaggaggagtacggatcgtcattggaagatgacgtggtgggggatacgtcgggttactaccaacgaatgcttgtcgtgcttttgcaggcaaatcgcgacccggatgcggggatcgacgaggcccaagtggagcaagatgcgcaagcactcttccaggccggtgaactcaaatgggggaccgatgaagagaagtttatcaccatctttggcacgaggagtgtaagtcatctgcgtaaagtattcgataagtatatgacaatctcagggtttcagattgaggagacaattgacagggaaacctccggtaacttggagcagctcttgcttgccgtcgtcaagtccattcgctcgatccctgcgtatctggctgaaacactgtattacgccatgaaaggggcaggcactgatgaccacaccttgattagagttatggtgtcgcgatcagaaattgacttgttcaatatccggaaagagttccggaagaatttcgcaacgagcctctatagcatgatcaaaggggacacttcgggagattacaagaaagcgttgctccttctttcaggagaggatgacggcagtggtggctcaggtagcggccaccatcaccatcaccactaatga

SEQ ID NO: 8 - DNA, 963 bp, Artificial Sequence
  Synthetic construct
gctcaagtcttgcgtggtacggtgacagacttcccaggcttcgatgaaagagcggacgcggaaacacttcgaaaggcgatgaaagggctcggtactgacgaagagtccattttgacccttcttacgagcaggtcaaacgctcagaggcaagaaatctctgcagcctttaagacactctttggagctgaccttcttgatgacctcgcatctgagctgacgggaaagtttgagaaactcatcgtagctttgatgaagcccagccgattgtatgatgcttacgaactgaaacacgccctggctggagcgggaacgaacgagaaagttttgactgagatcatcgcatcgcggaccccggaagagctcagagccatcaaacaagtctacgaggaggagtacggatcgtcattggcaggagacgtggtgggggatacgtcgggttactaccaacgaatgcttgtcgtgcttttgcaggcagctcgcgacccggatgcggggatcgacgaggcccaagtggagcaagatgcgcaagcactcttccaggccggtgaactcaaatgggggaccgatgaagagaagtttatcaccatctttggcacgaggagtgtaagtcatctgcgtaaagtattcgataagtatatgacaatctcagggtttcagattgaggagacaattgacagggaaacctccggtaacttggagcagctcttgcttgccgtcgtcaagtccattcgctcgatccctgcgtatctggctgaaacactgtattacgccatgaaaggggcaggcactgatgaccacaccttgattagagttatggtgtcgcgatcagaaattgacttgttcaatatccggaaagagttccggaagaatttcgcaacgagcctctatagcatgatcaaaggggacacttcgggagattacaagaaagcgttgctccttctttgcggagaggatgactaatga

SEQ ID NO: 9 - protein, 70 aa, Homo sapiens
GPETLCGAELVDALQFVCGDRGFYFNKPTGYGSSSRRAPQTGIVDECCFRSCDLRRLEMYCAPLKPAKSA

SEQ ID NO: 10 - protein, 67 aa, Artificial Sequence
  Synthetic construct
TLCGAELVDALQFVCGDRGFYFNKPTGYGSSSRRAPQTGIVDECCFRSCDLRRLEMYCAPLKPAKSA

SEQ ID NO: 11 - protein, 83 aa, Artificial Sequence
  Synthetic construct
MFPAMPLSSLFVNGPETLCGAELVDALQFVCGDRGFYFNKPTGYGSSSRRAPQTGIVDECCFRSCDLRRLEMYCAPLKPAKSA

SEQ ID NO: 12 - protein, 70 aa, Artificial Sequence
  Synthetic construct
GPRTLCGAELVDALQFVCGDRGFYFNKPTGYGSSSRRAPQTGIVDECCFRSCDLRRLEMYCAPLKPAKSA

SEQ ID NO: 13 - protein, 69 aa, Artificial Sequence
  Synthetic construct
GPETLCGAELVDALQFVCGDRGFYFNKPTGYGSSSRAPQTGIVDECCFRSCDLRRLEMYCAPLKPAKSA

SEQ ID NO: 14 - protein, 66 aa, Artificial Sequence
  Synthetic construct
GPETLCGAELVDALQFVCGDRGFYFNKPTGYGSSSRAPQTGIVDECCFRSCDLRRLEMYCAPLKPA

SEQ ID NO: 15 - protein, 83 aa, Artificial Sequence
  Synthetic construct
MFPAMPLSSLFVNGPRTLCGAELVDALQFVCGDRGFYFNKPTGYGSSSRRAPQTGIVDECCFRSCDLRRLEMYCAPLKPAKSA

SEQ ID NO: 16 - protein, 79 aa, Artificial Sequence
  Synthetic construct
MFPAMPLSSLFVNGPRTLCGAELVDALQFVCGDRGFYFNKPTGYGSSSRAPQTGIVDECCFRSCDLRRLEMYCAPLKPA

SEQ ID NO: 17 - protein, 83 aa, Artificial Sequence
  Synthetic construct
MFPAMPLSSLFVNGPRTLCGAELVDALQFVCGDRGFLFNKPTGYGSSSRRAPQTGIVDECCFRSCDLRRLEMYCAPLKPAKSA

SEQ ID NO: 18 - protein, 83 aa, Artificial Sequence
  Synthetic construct
MFPAMPLSSLFVNGPRTLCGAELVDALQFVCGDRGFLFNKPTGAGSSSRRAPQTGIVDECCFRSCDLRRLEMYCAPLKPAKSA

SEQ ID NO: 19 - protein, 83 aa, Artificial Sequence
  Synthetic construct
MFPAMPLSSLFVNGPRTLCGAELVDALQFVCGDRGFYFNKPTGAGSSSRRAPQTGIVDECCFRSCDLRRLEMYCAPLKPAKSA

SEQ ID NO: 20 - protein, 83 aa, Artificial Sequence
  Synthetic construct
MFPAMPLSSLFVNGPRTLCGAELVDALQFVCGDRGFYFNKPTGYGSSSRRAPQTGIVDECCFRSCDLRRLEMLCAPLKPAKSA

SEQ ID NO: 21 - protein, 66 aa, Artificial Sequence; identical to SEQ ID NO: 14
  Synthetic construct

SEQ ID NO: 22 - protein, 70 aa, Artificial Sequence
  Synthetic construct
GPETLCGAELVDALQFVCGDRGFLFNKPTGYGSSSRRAPQTGIVDECCFRSCDLRRLEMYCAPLKPAKSA

SEQ ID NO: 23 - protein, 70 aa, Artificial Sequence
  Synthetic construct
GPETLCGAELVDALQFVCGDRGFLFNKPTGAGSSSRRAPQTGIVDECCFRSCDLRRLEMYCAPLKPAKSA

SEQ ID NO: 24 - protein, 70 aa, Artificial Sequence
  Synthetic construct
GPETLCGAELVDALQFVCGDRGFYFNKPTGAGSSSRRAPQTGIVDECCFRSCDLRRLEMYCAPLKPAKSA

SEQ ID NO: 25 - protein, 70 aa, Artificial Sequence
  Synthetic construct
GPETLCGAELVDALQFVCGDRGFYFNKPTGYGSSSRRAPQTGIVDECCFRSCDLRRLEMLCAPLKPAKSA

SEQ ID NO: 26 - protein, 63 aa, Artificial Sequence
  Synthetic construct
TLCGAELVDALQFVCGDRGFYFNKPTGYGSSSRAPQTGIVDECCFRSCDLRRLEMYCAPLKPA

SEQ ID NO: 27 - protein, 67 aa, Artificial Sequence
  Synthetic construct
TLCGAELVDALQFVCGDRGFLFNKPTGYGSSSRRAPQTGIVDECCFRSCDLRRLEMYCAPLKPAKSA

SEQ ID NO: 28 - protein, 67 aa, Artificial Sequence
  Synthetic construct
TLCGAELVDALQFVCGDRGFLFNKPTGAGSSSRRAPQTGIVDECCFRSCDLRRLEMYCAPLKPAKSA

SEQ ID NO: 29 - protein, 67 aa, Artificial Sequence
  Synthetic construct
TLCGAELVDALQFVCGDRGFYFNKPTGAGSSSRRAPQTGIVDECCFRSCDLRRLEMYCAPLKPAKSA

SEQ ID NO: 30 - protein, 67 aa, Artificial Sequence
  Synthetic construct
TLCGAELVDALQFVCGDRGFYFNKPTGYGSSSRRAPQTGIVDECCFRSCDLRRLEMLCAPLKPAKSA

SEQ ID NO: 31 - DNA, 210 bp, Homo sapiens
ggcccagaaacactttgtggagccgaactggtggatgctctccaattcgtttgcggcgaccgcggattctactttaacaagcccaccggttacgggtcttcaagccggagggccccgcagactggcatcgtcgacgagtgctgttttagaagctgcgatctgcgacggttggagatgtattgtgcacctctgaagcccgcgaaaagtgct

SEQ ID NO: 32 - DNA, 201 bp, Artificial Sequence
  Synthetic construct
acactttgtggagccgaactggtggatgctctccaattcgtttgcggcgaccgcggattctactttaacaagcccaccggttacgggtcttcaagccggagggccccgcagactggcatcgtcgacgagtgctgttttagaagctgcgatctgcgacggttggagatgtattgtgcacctctgaagcccgcgaaaagtgct

SEQ ID NO: 33 - DNA, 249 bp, Artificial Sequence
  Synthetic construct
atgttcccagccatgcccttgtccagcctgtttgttaacggcccagaaacactttgtggagccgaactggtggatgctctccaattcgtttgcggcgaccgcggattctactttaacaagcccaccggttacgggtcttcaagccggagggccccgcagactggcatcgtcgacgagtgctgttttagaagctgcgatctgcgacggttggagatgtattgtgcacctctgaagcccgcgaaaagtgct

SEQ ID NO: 34 - DNA, 210 bp, Artificial Sequence
  Synthetic construct
ggcccaagaacactttgtggagccgaactggtggatgctctccaattcgtttgcggcgaccgcggattctactttaacaagcccaccggttacgggtcttcaagccggagggccccgcagactggcatcgtcgacgagtgctgttttagaagctgcgatctgcgacggttggagatgtattgtgcacctctgaagcccgcgaaaagtgct

SEQ ID NO: 35 - DNA, 207 bp, Artificial Sequence
  Synthetic construct
ggcccagaaacactttgtggagccgaactggtggatgctctccaattcgtttgcggcgaccgcggattctactttaacaagcccaccggttacgggtcttcaagccgggccccgcagactggcatcgtcgacgagtgctgttttagaagctgcgatctgcgacggttggagatgtattgtgcacctctgaagcccgcgaaaagtgct

SEQ ID NO: 36 - DNA, 201 bp, Artificial Sequence
  Synthetic construct
ggcccagaaacactttgtggagccgaactggtggatgctctccaattcgtttgcggcgaccgcggattctactttaacaagcccaccggttacgggtcttcaagccggagggccccgcagactggcatcgtcgacgagtgctgttttagaagctgcgatctgcgacggttggagatgtattgtgcacctctgaagcccgcg

SEQ ID NO: 37 - DNA, 249 bp, Artificial Sequence
  Synthetic construct
atgttcccagccatgcccttgtccagcctgtttgttaacggcccaagaacactttgtggagccgaactggtggatgctctccaattcgtttgcggcgaccgcggattctactttaacaagcccaccggttacgggtcttcaagccggagggccccgcagactggcatcgtcgacgagtgctgttttagaagctgcgatctgcgacggttggagatgtattgtgcacctctgaagcccgcgaaaagtgct

SEQ ID NO: 38 - DNA, 237 bp, Artificial Sequence
  Synthetic construct
atgttcccagccatgcccttgtccagcctgtttgttaacggcccaagaacactttgtggagccgaactggtggatgctctccaattcgtttgcggcgaccgcggattctactttaacaagcccaccggttacgggtcttcaagccgggccccgcagactggcatcgtcgacgagtgctgttttagaagctgcgatctgcgacggttggagatgtattgtgcacctctgaagcccgcg

SEQ ID NO: 39 - DNA, 249 bp, Artificial Sequence
  Syntehtic construct
atgttcccagccatgcccttgtccagcctgtttgttaacggcccaagaacactttgtggagccgaactggtggatgctctccaattcgtttgcggcgaccgcggattcctctttaacaagcccaccggttacgggtcttcaagccggagggccccgcagactggcatcgtcgacgagtgctgttttagaagctgcgatctgcgacggttggagatgtattgtgcacctctgaagcccgcgaaaagtgct

SEQ ID NO: 40 - DNA, 249 bp, Artificial Sequence
  Synthetic construct
atgttcccagccatgcccttgtccagcctgtttgttaacggcccaagaacactttgtggagccgaactggtggatgctctccaattcgtttgcggcgaccgcggattcctctttaacaagcccaccggtgccgggtcttcaagccggagggccccgcagactggcatcgtcgacgagtgctgttttagaagctgcgatctgcgacggttggagatgtattgtgcacctctgaagcccgcgaaaagtgct

SEQ ID NO: 41 - DNA, 249 bp, Artificial Sequence
  Synthetic construct
atgttcccagccatgcccttgtccagcctgtttgttaacggcccaagaacactttgtggagccgaactggtggatgctctccaattcgtttgcggcgaccgcggattctactttaacaagcccaccggtgccgggtcttcaagccggagggccccgcagactggcatcgtcgacgagtgctgttttagaagctgcgatctgcgacggttggagatgtattgtgcacctctgaagcccgcgaaaagtgct

SEQ ID NO: 42 - DNA, 249 bp, Artificial Sequence
  Synthetic construct
atgttcccagccatgcccttgtccagcctgtttgttaacggcccaagaacactttgtggagccgaactggtggatgctctccaattcgtttgcggcgaccgcggattctactttaacaagcccaccggttacgggtcttcaagccggagggccccgcagactggcatcgtcgacgagtgctgttttagaagctgcgatctgcgacggttggagatgttgtgtgcacctctgaagcccgcgaaaagtgct

SEQ ID NO: 43 - DNA, 198 bp, Artificial Sequence
  Synthetic construct
ggcccagaaacactttgtggagccgaactggtggatgctctccaattcgtttgcggcgaccgcggattctactttaacaagcccaccggttacgggtcttcaagccgggccccgcagactggcatcgtcgacgagtgctgttttagaagctgcgatctgcgacggttggagatgtattgtgcacctctgaagcccgcg

SEQ ID NO: 44 - DNA, 210 bp, Artificial Sequence
  Synthetic construct
ggcccagaaacactttgtggagccgaactggtggatgctctccaattcgtttgcggcgaccgcggattcctctttaacaagcccaccggttacgggtcttcaagccggagggccccgcagactggcatcgtcgacgagtgctgttttagaagctgcgatctgcgacggttggagatgtattgtgcacctctgaagcccgcgaaaagtgct

SEQ ID NO: 45 - DNA, 210 bp, Artificial Sequence
  Synthetic construct
ggcccagaaacactttgtggagccgaactggtggatgctctccaattcgtttgcggcgaccgcggattcctctttaacaagcccaccggtgccgggtcttcaagccggagggccccgcagactggcatcgtcgacgagtgctgttttagaagctgcgatctgcgacggttggagatgtattgtgcacctctgaagcccgcgaaaagtgct

SEQ ID NO: 46 - DNA, 210 bp, Artificial Sequence
  Syntehtic construct
ggcccagaaacactttgtggagccgaactggtggatgctctccaattcgtttgcggcgaccgcggattctactttaacaagcccaccggtgccgggtcttcaagccggagggccccgcagactggcatcgtcgacgagtgctgttttagaagctgcgatctgcgacggttggagatgtattgtgcacctctgaagcccgcgaaaagtgct

SEQ ID NO: 47 - DNA, 210 bp, Artificial Sequence
  Synthetic construct
ggcccagaaacactttgtggagccgaactggtggatgctctccaattcgtttgcggcgaccgcggattctactttaacaagcccaccggttacgggtcttcaagccggagggccccgcagactggcatcgtcgacgagtgctgttttagaagctgcgatctgcgacggttggagatgttgtgtgcacctctgaagcccgcgaaaagtgct

SEQ ID NO: 48 - DNA, 189 bp, Artificial Sequence
  Synthetic construct
acactttgtggagccgaactggtggatgctctccaattcgtttgcggcgaccgcggattctactttaacaagcccaccggttacgggtcttcaagccgggccccgcagactggcatcgtcgacgagtgctgttttagaagctgcgatctgcgacggttggagatgtattgtgcacctctgaagcccgcg

SEQ ID NO: 49 - DNA, 201 bp, Artificial Sequence
  Synthetic construct
acactttgtggagccgaactggtggatgctctccaattcgtttgcggcgaccgcggattcctctttaacaagcccaccggttacgggtcttcaagccggagggccccgcagactggcatcgtcgacgagtgctgttttagaagctgcgatctgcgacggttggagatgtattgtgcacctctgaagcccgcgaaaagtgct

SEQ ID NO: 50 - DNA, 201 bp, Artificial Sequence
  Synthetic construct
acactttgtggagccgaactggtggatgctctccaattcgtttgcggcgaccgcggattcctctttaacaagcccaccggtgccgggtcttcaagccggagggccccgcagactggcatcgtcgacgagtgctgttttagaagctgcgatctgcgacggttggagatgtattgtgcacctctgaagcccgcgaaaagtgct

SEQ ID NO: 51 - DNA, 201 bp, Artificial Sequence
  Synthetic construct
acactttgtggagccgaactggtggatgctctccaattcgtttgcggcgaccgcggattctactttaacaagcccaccggtgccgggtcttcaagccggagggccccgcagactggcatcgtcgacgagtgctgttttagaagctgcgatctgcgacggttggagatgtattgtgcacctctgaagcccgcgaaaagtgct

SEQ ID NO: 52 - DNA, 201 bp, Artificial Sequence
  Synthetic construct
acactttgtggagccgaactggtggatgctctccaattcgtttgcggcgaccgcggattctactttaacaagcccaccggttacgggtcttcaagccggagggccccgcagactggcatcgtcgacgagtgctgttttagaagctgcgatctgcgacggttggagatgttgtgtgcacctctgaagcccgcgaaaagtgct

SEQ ID NO: 53 - protein, 226 aa, Artificial Sequence
  Synthetic construct
DKTHTCPPCPAPELLGGPSVFLFPPKPKDTLMISRTPEVTCVVVDVSHEDPEVKFNWYVDGVEVHNAKTKPREEQYQSTYRVVSVLTVLHQDWLNGKEYKCKVSNKALPAPIEKTISKAKGQPREPQVYTLPPSREEMTKNQVSLTCLVKGFYPSDIAVEWESNGQPENNYKTTPPVLDSDGSFFLYSKLTVDKSRWQQGNVFSCSVMHEALHNHYTQKSLSLSPG

SEQ ID NO: 54 - protein, 585 aa, Homor sapiens [sequence omitted]

SEQ ID NO: 55 - protein, 585 aa, Artificial Sequence
  Synthetic construct
DAHKSEVAHRFKDLGEENFKALVLIAFAQYLQQSPFEDHVKLVNEVTEFAKTCVADESAENCDKSLHTLFGDKLCTVATLRETYGEMADCCAKQEPERNECFLQHKDDNPNLPRLVRPEVDVMCTAFHDNEETFLKKYLYEIARRHPYFYAPELLFFAKRYKAAFTECCQAADKAACLLPKLDELRDEGKASSAKQRLKCASLQKFGERAFKAWAVARLSQRFPKAEFAEVSKLVTDLTKVHTECCHGDLLECADDRADLAKYICENQDSISSKLKECCEKPLLEKSHCIAEVENDEMPADLPSLAADFVESKDVCKNYAEAKDVFLGMFLYEYARRHPDYSVVLLLRLAKTYETTLEKCCAAADPHECYAKVFDEFKPLVEEPQNLIKQNCELFEQLGEYKFQNALLVRYTKKVPQVSTPTLVEVSRNLGKVGSKCCKHPEAKRMPCAEDYLSVVLNQLCVLHEKTPVSDRVTKCCTESLVNRRPCFSALEVDETYVPKEFQAETFTFHADICTLSEKERQIKKQTALVELVKHKPKATKEQLKAVMDDFAAFVEKCCKADDKETCFAEEGKKLVAASQAALGL

SEQ ID NO: 56 - protein, 585 aa, Artificial Sequence
  Synthetic construct
DAHKSEVAHRFKDLGEENFKALVLIAFAQYLQQSPFEDHVKLVNEVTEFAKTCVADESAENCDKSLHTLFGDKLCTVATLRETYGEMADCCAKQEPERNECFLQHKDDNPNLPRLVRPEVDVMCTAFHDNEETFLKKYLYEIARRHPYFYAPELLFFAKRYKAAFTECCQAADKAACLLPKLDELRDEGKASSAKQRLKCASLQKFGERAFKAWAVARLSQRFPKAEFAEVSKLVTDLTKVHTECCHGDLLECADDRADLAKYICENQDSISSKLKECCEKPLLEKSHCIAEVENDEMPADLPSLAADFVESKDVCKNYAEAKDVFLGMFLYEYARRHPDYSVVLLLRLAKTYETTLEKCCAAADPHECYAKVFDEFKPLVEEPQNLIKQNCELFEQLGEYKFQNALLVRYTKKVPQVSTPTLVEVSRNLGKVGSKCCKHPEAKRMPCAEDYLSVVLNQLCVLHEKTPVSDRVTKCCTESLVNRRPCFSALEVDETYVPKEFQAGTFTFHADICTLSEKERQIKKQTALVELVKHKPKATKEQLKAAMDDFAAFVEKCCKADDKETCFAEEGKKLVAASQAALGL

SEQ ID NO: 57 - DNA, 1755 bp, Homo sapiens
gacgctcacaagtctgaagtggcacataggttcaaagatctgggcgaagagaactttaaggccctcgtcctgatcgctttcgcacagtacctccagcagtgtccctttgaagatcacgtgaaactggtcaatgaggtgaccgaatttgccaagacatgcgtggctgatgagagtgcagaaaactgtgacaaatcactgcatactctctttggagataagctgtgcaccgtcgccacactcagagagacttatggggaaatggctgactgttgcgcaaaacaggagcctgaacggaatgagtgtttcctccagcacaaggatgacaacccaaatctgccccgcctcgtgcgacctgaggtcgatgtgatgtgcaccgcctttcatgacaacgaagagacattcctgaagaaatacctgtatgaaattgctcgtaggcacccatacttttatgcccccgagctcctgttctttgcaaagagatacaaagctgccttcactgaatgttgccaggcagctgataaggccgcatgtctcctgcctaaactggacgagctccgggatgaaggtaaggcttccagcgccaaacagcgcctgaagtgcgcttctctccagaagtttggcgagcgagcattcaaagcctgggctgtggcccgtctcagtcagaggtttccaaaggcagaatttgctgaggtgtcaaaactggtgaccgacctcacaaaggtccatactgagtgttgccacggagatctgctggaatgtgccgacgatagagcagacctcgctaaatatatctgcgagaatcaggattccattagctctaagctgaaagaatgttgcgagaagcccctcctggaaaagagtcattgtatcgccgaggtggaaaacgacgagatgccagcagatctgccatcactcgctgccgactttgtggaatccaaagatgtctgcaagaattacgcagaggctaaagacgtgttcctggggatgtttctgtatgagtacgcccggcgtcaccccgattatagcgtcgtgctcctgctccgactggcaaagacctacgaaacaactctggagaaatgttgcgctgccgcagaccctcatgaatgttatgctaaggtgttcgatgagtttaagccactcgtcgaagagccccagaacctgattaaacagaattgcgaactgttcgagcagctcggtgaatacaagtttcagaacgccctgctcgtgcgttataccaaaaaggtccctcaggtgtctacaccaactctggtggaggtcagtaggaatctgggcaaagtgggatcaaagtgttgcaaacaccccgaggcaaagagaatgccttgtgctgaagattacctctccgtcgtgctgaaccagctctgcgtgctgcatgaaaagaccccagtcagcgaccgggtgacaaaatgttgcaccgaatctctggtcaatcgccgaccctgtttcagtgccctcgaagtggacgaaacttatgtgcctaaggagtttaatgctgaaacattcacctttcacgccgatatctgcactctgtccgagaaagaaaggcagattaagaaacagacagcactggtcgagctcgtgaagcataaaccaaaggctaccaaggagcagctgaaagccgtcatggacgatttcgcagcttttgtggaaaagtgttgcaaagccgacgataaggagacttgtttcgcagaagaggggaaaaagctcgtggctgccagccaggcagctctgggtctg

SEQ ID NO: 58 - DNA, 1755 bp, Artificial Sequence
  Synthetic construct
gacgctcacaagtctgaagtggcacataggttcaaagatctgggcgaagagaactttaaggccctcgtcctgatcgctttcgcacagtacctccagcagtctccctttgaagatcacgtgaaactggtcaatgaggtgaccgaatttgccaagacatgcgtggctgatgagagtgcagaaaactgtgacaaatcactgcatactctctttggagataagctgtgcaccgtcgccacactcagagagacttatggggaaatggctgactgttgcgcaaaacaggagcctgaacggaatgagtgtttcctccagcacaaggatgacaacccaaatctgccccgcctcgtgcgacctgaggtcgatgtgatgtgcaccgcctttcatgacaacgaagagacattcctgaagaaatacctgtatgaaattgctcgtaggcacccatacttttatgcccccgagctcctgttctttgcaaagagatacaaagctgccttcactgaatgttgccaggcagctgataaggccgcatgtctcctgcctaaactggacgagctccgggatgaaggtaaggcttccagcgccaaacagcgcctgaagtgcgcttctctccagaagtttggcgagcgagcattcaaagcctgggctgtggcccgtctcagtcagaggtttccaaaggcagaatttgctgaggtgtcaaaactggtgaccgacctcacaaaggtccatactgagtgttgccacggagatctgctggaatgtgccgacgatagagcagacctcgctaaatatatctgcgagaatcaggattccattagctctaagctgaaagaatgttgcgagaagcccctcctggaaaagagtcattgtatcgccgaggtggaaaacgacgagatgccagcagatctgccatcactcgctgccgactttgtggaatccaaagatgtctgcaagaattacgcagaggctaaagacgtgttcctggggatgtttctgtatgagtacgcccggcgtcaccccgattatagcgtcgtgctcctgctccgactggcaaagacctacgaaacaactctggagaaatgttgcgctgccgcagaccctcatgaatgttatgctaaggtgttcgatgagtttaagccactcgtcgaagagccccagaacctgattaaacagaattgcgaactgttcgagcagctcggtgaatacaagtttcagaacgccctgctcgtgcgttataccaaaaaggtccctcaggtgtctacaccaactctggtggaggtcagtaggaatctgggcaaagtgggatcaaagtgttgcaaacaccccgaggcaaagagaatgccttgtgctgaagattacctctccgtcgtgctgaaccagctctgcgtgctgcatgaaaagaccccagtcagcgaccgggtgacaaaatgttgcaccgaatctctggtcaatcgccgaccctgtttcagtgccctcgaagtggacgaaacttatgtgcctaaggagtttcaggctgaaacattcacctttcacgccgatatctgcactctgtccgagaaagaaaggcagattaagaaacagacagcactggtcgagctcgtgaagcataaaccaaaggctaccaaggagcagctgaaagccgtcatggacgatttcgcagcttttgtggaaaagtgttgcaaagccgacgataaggagacttgtttcgcagaagaggggaaaaagctcgtggctgccagccaggcagctctgggtctg

SEQ ID NO: 59 - DNA, 1755 bp, Artificial Sequence
  Synthetic construct
gacgctcacaagtctgaagtggcacataggttcaaagatctgggcgaagagaactttaaggccctcgtcctgatcgctttcgcacagtacctccagcagtctccctttgaagatcacgtgaaactggtcaatgaggtgaccgaatttgccaagacatgcgtggctgatgagagtgcagaaaactgtgacaaatcactgcatactctctttggagataagctgtgcaccgtcgccacactcagagagacttatggggaaatggctgactgttgcgcaaaacaggagcctgaacggaatgagtgtttcctccagcacaaggatgacaacccaaatctgccccgcctcgtgcgacctgaggtcgatgtgatgtgcaccgcctttcatgacaacgaagagacattcctgaagaaatacctgtatgaaattgctcgtaggcacccatacttttatgcccccgagctcctgttctttgcaaagagatacaaagctgccttcactgaatgttgccaggcagctgataaggccgcatgtctcctgcctaaactggacgagctccgggatgaaggtaaggcttccagcgccaaacagcgcctgaagtgcgcttctctccagaagtttggcgagcgagcattcaaagcctgggctgtggcccgtctcagtcagaggtttccaaaggcagaatttgctgaggtgtcaaaactggtgaccgacctcacaaaggtccatactgagtgttgccacggagatctgctggaatgtgccgacgatagagcagacctcgctaaatatatctgcgagaatcaggattccattagctctaagctgaaagaatgttgcgagaagcccctcctggaaaagagtcattgtatcgccgaggtggaaaacgacgagatgccagcagatctgccatcactcgctgccgactttgtggaatccaaagatgtctgcaagaattacgcagaggctaaagacgtgttcctggggatgtttctgtatgagtacgcccggcgtcaccccgattatagcgtcgtgctcctgctccgactggcaaagacctacgaaacaactctggagaaatgttgcgctgccgcagaccctcatgaatgttatgctaaggtgttcgatgagtttaagccactcgtcgaagagccccagaacctgattaaacagaattgcgaactgttcgagcagctcggtgaatacaagtttcagaacgccctgctcgtgcgttataccaaaaaggtccctcaggtgtctacaccaactctggtggaggtcagtaggaatctgggcaaagtgggatcaaagtgttgcaaacaccccgaggcaaagagaatgccttgtgctgaagattacctctccgtcgtgctgaaccagctctgcgtgctgcatgaaaagaccccagtcagcgaccgggtgacaaaatgttgcaccgaatctctggtcaatcgccgaccctgtttcagtgccctcgaagtggacgaaacttatgtgcctaaggagtttcaggctggaacattcacctttcacgccgatatctgcactctgtccgagaaagaaaggcagattaagaaacagacagcactggtcgagctcgtgaagcataaaccaaaggctaccaaggagcagctgaaagccgccatggacgatttcgcagcttttgtggaaaagtgttgcaaagccgacgataaggagacttgtttcgcagaagaggggaaaaagctcgtggctgccagccaggcagctctgggtctg

SEQ ID NO: 60 - protein, 7 aa, Artificial Sequence
  Synthetic construct
GSGGGSG

SEQ ID NO: 61 - protein, 15 aa, Artificial Sequence
  Synthetic construct
GSGGSGGGSGGSGGG

SEQ ID NO: 62 - protein, 40 aa, Artificial Sequence
  Synthetic construct
GSGGSGGGSGGGSGGGSGGGSGGGSGGGSGGGSGGGSGGG

SEQ ID NO: 63 - DNA, 21 bp, Artificial Sequence
  Synthetic construct
gggagcggtggtgggagtggc

SEQ ID NO: 64 - DNA, 45 bp, Artificial Sequence
  Synthetic construct
gggtctggcggttcagggggaggaagtggaggctcaggaggtggt

SEQ ID NO: 65 - DNA, 120 bp, Artificial Sequence
  Synthetic construct
ggttccggaggttctggcggtggatctgggggcggtagcggaggcggcagtggtggtggcagcgggggagggtcaggtgggggtagtggcggtggttctggaggtggttcaggaggagga

SEQ ID NO: 66 - protein, 721 aa, Artificial Sequence
  Synthetic construct
MFPAMPLSSLFVNGPRTLCGAELVDALQFVCGDRGFYFNKPTGYGSSSRAPQTGIVDECCFRSCDLRRLEMYCAPLKPAKSAGSGGSGGGSGGGSGGGSGGGSGGGSGGGSGGGSGGGSGGGDAHKSEVAHRFKDLGEENFKALVLIAFAQYLQQSPFEDHVKLVNEVTEFAKTCVADESAENCDKSLHTLFGDKLCTVATLRETYGEMADCCAKQEPERNECFLQHKDDNPNLPRLVRPEVDVMCTAFHDNEETFLKKYLYEIARRHPYFYAPELLFFAKRYKAAFTECCQAADKAACLLPKLDELRDEGKASSAKQRLKCASLQKFGERAFKAWAVARLSQRFPKAEFAEVSKLVTDLTKVHTECCHGDLLECADDRADLAKYICENQDSISSKLKECCEKPLLEKSHCIAEVENDEMPADLPSLAADFVESKDVCKNYAEAKDVFLGMFLYEYARRHPDYSVVLLLRLAKTYETTLEKCCAAADPHECYAKVFDEFKPLVEEPQNLIKQNCELFEQLGEYKFQNALLVRYTKKVPQVSTPTLVEVSRNLGKVGSKCCKHPEAKRMPCAEDYLSVVLNQLCVLHEKTPVSDRVTKCCTESLVNRRPCFSALEVDETYVPKEFQAETFTFHADICTLSEKERQIKKQTALVELVKHKPKATKEQLKAVMDDFAAFVEKCCKADDKETCFAEEGKKLVAASQAALGLGSGGSGSGHHHHHH

SEQ ID NO: 67 - protein, 1063 aa, Artificial Sequence
  Synthetic construct
MFPAMPLSSLFVNGPRTLCGAELVDALQFVCGDRGFYFNKPTGYGSSSRAPQTGIVDECCFRSCDLRRLEMYCAPLKPAGSGGSGGGSGGGSGGGSGGGSGGGSGGGSGGGSGGGSGGGDKTHTCPPCPAPELLGGPSVFLFPPKPKDTLMISRTPEVTCVVVDVSHEDPEVKFNWYVDGVEVHNAKTKPREEQYQSTYRVVSVLTVLHQDWLNGKEYKCKVSNKALPAPIEKTISKAKGQPREPQVYTLPPSREEMTKNQVSLTCLVKGFYPSDIAVEWESNGQPENNYKTTPPVLDSDGSFFLYSKLTVDKSRWQQGNVFSCSVMHEALHNHYTQKSLSLSPGGSGGSGGGSGGGSGGGSGGGSGGGSGGGSGGGSGGGSGGGAQVLRGTVTDFPGFDERADAETLRKAMKGLGTDEESILTLLTSRSNAQRQEISAAFKTLFGRDLLDDLKSELTGKFEKLIVALMKPSRLYDAYELKHALKGAGTNEKVLTEIIASRTPEELRAIKQVYEEEYGSSLEDDVVGDTSGYYQRMLVVLLQANRDPDAGIDEAQVEQDAQALFQAGELKWGTDEEKFITIFGTRSVSHLRKVFDKYMTISGFQIEETIDRETSGNLEQLLLAVVKSIRSIPAYLAETLYYAMKGAGTDDHTLIRVMVSRSEIDLFNIRKEFRKNFATSLYSMIKGDTSGDYKKALLLLSGEDDGSGGSGGGSGGGSGGGSGGGSGGGSGGGSGGGSGGGSGSGAQVLRGTVTDFPGFDERADAETLRKAMKGLGTDEESILTLLTSRSNAQRQEISAAFKTLFGRDLLDDLKSELTGKFEKLIVALMKPSRLYDAYELKHALKGAGTNEKVLTEIIASRTPEELRAIKQVYEEEYGSSLEDDVVGDTSGYYQRMLVVLLQANRDPDAGIDEAQVEQDAQALFQAGELKWGTDEEKFITIFGTRSVSHLRKVFDKYMTISGFQIEETIDRETSGNLEQLLLAVVKSIRSIPAYLAETLYYAMKGAGTDDHTLIRVMVSRSEIDLFNIRKEFRKNFATSLYSMIKGDTSGDYKKALLLLSGEDD

SEQ ID NO: 68 - protein, 683 aa, Artificial Sequence
  Synthetic construct
MFPAMPLSSLFVNGPRTLCGAELVDALQFVCGDRGFYFNKPTGYGSSSRRAPQTGIVDECCFRSCDLRRLEMYCAPLKPAKSAGSGGSGGGSGGSGGGDAHKSEVAHRFKDLGEENFKALVLIAFAQYLQQSPFEDHVKLVNEVTEFAKTCVADESAENCDKSLHTLFGDKLCTVATLRETYGEMADCCAKQEPERNECFLQHKDDNPNLPRLVRPEVDVMCTAFHDNEETFLKKYLYEIARRHPYFYAPELLFFAKRYKAAFTECCQAADKAACLLPKLDELRDEGKASSAKQRLKCASLQKFGERAFKAWAVARLSQRFPKAEFAEVSKLVTDLTKVHTECCHGDLLECADDRADLAKYICENQDSISSKLKECCEKPLLEKSHCIAEVENDEMPADLPSLAADFVESKDVCKNYAEAKDVFLGMFLYEYARRHPDYSVVLLLRLAKTYETTLEKCCAAADPHECYAKVFDEFKPLVEEPQNLIKQNCELFEQLGEYKFQNALLVRYTKKVPQVSTPTLVEVSRNLGKVGSKCCKHPEAKRMPCAEDYLSVVLNQLCVLHEKTPVSDRVTKCCTESLVNRRPCFSALEVDETYVPKEFQAETFTFHADICTLSEKERQIKKQTALVELVKHKPKATKEQLKAVMDDFAAFVEKCCKADDKETCFAEEGKKLVAASQAALGL

SEQ ID NO: 69 - protein, 680 aa, Artificial Sequence
  Synthetic construct
MFPAMPLSSLFVNGPRTLCGAELVDALQFVCGDRGFYFNKPTGYGSSSRAPQTGIVDECCFRSCDLRRLEMYCAPLKPAGGDAHKSEVAHRFKDLGEENFKALVLIAFAQYLQQSPFEDHVKLVNEVTEFAKTCVADESAENCDKSLHTLFGDKLCTVATLRETYGEMADCCAKQEPERNECFLQHKDDNPNLPRLVRPEVDVMCTAFHDNEETFLKKYLYEIARRHPYFYAPELLFFAKRYKAAFTECCQAADKAACLLPKLDELRDEGKASSAKQRLKCASLQKFGERAFKAWAVARLSQRFPKAEFAEVSKLVTDLTKVHTECCHGDLLECADDRADLAKYICENQDSISSKLKECCEKPLLEKSHCIAEVENDEMPADLPSLAADFVESKDVCKNYAEAKDVFLGMFLYEYARRHPDYSVVLLLRLAKTYETTLEKCCAAADPHECYAKVFDEFKPLVEEPQNLIKQNCELFEQLGEYKFQNALLVRYTKKVPQVSTPTLVEVSRNLGKVGSKCCKHPEAKRMPCAEDYLSVVLNQLCVLHEKTPVSDRVTKCCTESLVNRRPCFSALEVDETYVPKEFQAETFTFHADICTLSEKERQIKKQTALVELVKHKPKATKEQLKAVMDDFAAFVEKCCKADDKETCFAEEGKKLVAASQAALGLGSGGSGSGHHHHHH

SEQ ID NO: 70 - protein, 1077 aa, Artificial Sequence
  Synthetic construct
MFPAMPLSSLFVNGPRTLCGAELVDALQFVCGDRGFYFNKPTGYGSSSRAPQTGIVDECCFRSCDLRRLEMYCAPLKPAGSGGSGGGSGGGSGGGSGGGSGGGSGGGSGGGSGGGSGGGDAHKSEVAHRFKDLGEENFKALVLIAFAQYLQQSPFEDHVKLVNEVTEFAKTCVADESAENCDKSLHTLFGDKLCTVATLRETYGEMADCCAKQEPERNECFLQHKDDNPNLPRLVRPEVDVMCTAFHDNEETFLKKYLYEIARRHPYFYAPELLFFAKRYKAAFTECCQAADKAACLLPKLDELRDEGKASSAKQRLKCASLQKFGERAFKAWAVARLSQRFPKAEFAEVSKLVTDLTKVHTECCHGDLLECADDRADLAKYICENQDSISSKLKECCEKPLLEKSHCIAEVENDEMPADLPSLAADFVESKDVCKNYAEAKDVFLGMFLYEYARRHPDYSVVLLLRLAKTYETTLEKCCAAADPHECYAKVFDEFKPLVEEPQNLIKQNCELFEQLGEYKFQNALLVRYTKKVPQVSTPTLVEVSRNLGKVGSKCCKHPEAKRMPCAEDYLSVVLNQLCVLHEKTPVSDRVTKCCTESLVNRRPCFSALEVDETYVPKEFQAETFTFHADICTLSEKERQIKKQTALVELVKHKPKATKEQLKAVMDDFAAFVEKCCKADDKETCFAEEGKKLVAASQAALGLGSGGSGGGSGGGSGGGSGGGSGGGSGGGSGGGSGGGSGGGAQVLRGTVTDFPGFDERADAETLRKAMKGLGTDEESILTLLTSRSNAQRQEISAAFKTLFGRDLLDDLKSELTGKFEKLIVALMKPSRLYDAYELKHALKGAGTNEKVLTEIIASRTPEELRAIKQVYEEEYGSSLEDDVVGDTSGYYQRMLVVLLQANRDPDAGIDEAQVEQDAQALFQAGELKWGTDEEKFITIFGTRSVSHLRKVFDKYMTISGFQIEETIDRETSGNLEQLLLAVVKSIRSIPAYLAETLYYAMKGAGTDDHTLIRVMVSRSEIDLFNIRKEFRKNFATSLYSMIKGDTSGDYKKALLLLSGEDDGSGGSGSGHHHHHH

SEQ ID NO: 71 - protein, 708 aa, Artificial Sequence
  Synthetic construct
MFPAMPLSSLFVNGPRTLCGAELVDALQFVCGDRGFYFNKPTGYGSSSRRAPQTGIVDECCFRSCDLRRLEMYCAPLKPAKSAGSGGSGGGSGGGSGGGSGGGSGGGSGGGSGGGSGGGSGGGDKTHTCPPCPAPELLGGPSVFLFPPKPKDTLMISRTPEVTCVVVDVSHEDPEVKFNWYVDGVEVHNAKTKPREEQYQSTYRVVSVLTVLHQDWLNGKEYKCKVSNKALPAPIEKTISKAKGQPREPQVYTLPPSREEMTKNQVSLTCLVKGFYPSDIAVEWESNGQPENNYKTTPPVLDSDGSFFLYSKLTVDKSRWQQGNVFSCSVMHEALHNHYTQKSLSLSPGGSGGSGGGSGGGSGGGSGGGSGGGSGGGSGGGSGGGSGGGAQVLRGTVTDFPGFDERADAETLRKAMKGLGTDEESILTLLTSRSNAQRQEISAAFKTLFGRDLLDDLKSELTGKFEKLIVALMKPSRLYDAYELKHALKGAGTNEKVLTEIIASRTPEELRAIKQVYEEEYGSSLEDDVVGDTSGYYQRMLVVLLQANRDPDAGIDEAQVEQDAQALFQAGELKWGTDEEKFITIFGTRSVSHLRKVFDKYMTISGFQIEETIDRETSGNLEQLLLAVVKSIRSIPAYLAETLYYAMKGAGTDDHTLIRVMVSRSEIDLFNIRKEFRKNFATSLYSMIKGDTSGDYKKALLLLSGEDD

SEQ ID NO: 72 - protein, 345 aa, Artificial Sequence
  Synthetic construct
MFPAMPLSSLFVNGPRTLCGAELVDALQFVCGDRGFYFNKPTGYGSSSRAPQTGIVDECCFRSCDLRRLEMYCAPLKPAGSGGSGGGSGGGSGGGSGGGSGGGSGGGSGGGSGGGSGGGDKTHTCPPCPAPELLGGPSVFLFPPKPKDTLMISRTPEVTCVVVDVSHEDPEVKFNWYVDGVEVHNAKTKPREEQYQSTYRVVSVLTVLHQDWLNGKEYKCKVSNKALPAPIEKTISKAKGQPREPQVYTLPPSREEMTKNQVSLTCLVKGFYPSDIAVEWESNGQPENNYKTTPPVLDSDGSFFLYSKLTVDKSRWQQGNVFSCSVMHEALHNHYTQKSLSLSPG

SEQ ID NO: 73 - protein, 1017 aa, Artificial Sequence
  Synthetic construct
MFPAMPLSSLFVNGPRTLCGAELVDALQFVCGDRGFYFNKPTGYGSSSRRAPQTGIVDECCFRSCDLRRLEMYCAPLKPAKSAGSGGSGGGSGGSGGGDAHKSEVAHRFKDLGEENFKALVLIAFAQYLQQSPFEDHVKLVNEVTEFAKTCVADESAENCDKSLHTLFGDKLCTVATLRETYGEMADCCAKQEPERNECFLQHKDDNPNLPRLVRPEVDVMCTAFHDNEETFLKKYLYEIARRHPYFYAPELLFFAKRYKAAFTECCQAADKAACLLPKLDELRDEGKASSAKQRLKCASLQKFGERAFKAWAVARLSQRFPKAEFAEVSKLVTDLTKVHTECCHGDLLECADDRADLAKYICENQDSISSKLKECCEKPLLEKSHCIAEVENDEMPADLPSLAADFVESKDVCKNYAEAKDVFLGMFLYEYARRHPDYSVVLLLRLAKTYETTLEKCCAAADPHECYAKVFDEFKPLVEEPQNLIKQNCELFEQLGEYKFQNALLVRYTKKVPQVSTPTLVEVSRNLGKVGSKCCKHPEAKRMPCAEDYLSVVLNQLCVLHEKTPVSDRVTKCCTESLVNRRPCFSALEVDETYVPKEFQAETFTFHADICTLSEKERQIKKQTALVELVKHKPKATKEQLKAVMDDFAAFVEKCCKADDKETCFAEEGKKLVAASQAALGLGSGGSGGGSGGSGGGAQVLRGTVTDFPGFDERADAETLRKAMKGLGTDEESILTLLTSRSNAQRQEISAAFKTLFGRDLLDDLKSELTGKFEKLIVALMKPSRLYDAYELKHALKGAGTNEKVLTEIIASRTPEELRAIKQVYEEEYGSSLEDDVVGDTSGYYQRMLVVLLQANRDPDAGIDEAQVEQDAQALFQAGELKWGTDEEKFITIFGTRSVSHLRKVFDKYMTISGFQIEETIDRETSGNLEQLLLAVVKSIRSIPAYLAETLYYAMKGAGTDDHTLIRVMVSRSEIDLFNIRKEFRKNFATSLYSMIKGDTSGDYKKALLLLCGEDD

SEQ ID NO: 74 - protein, 1017 aa, Artificial Sequence
  Synthetic construct
MFPAMPLSSLFVNGPRTLCGAELVDALQFVCGDRGFYFNKPTGYGSSSRRAPQTGIVDECCFRSCDLRRLEMYCAPLKPAKSAGSGGSGGGSGGSGGGDAHKSEVAHRFKDLGEENFKALVLIAFAQYLQQSPFEDHVKLVNEVTEFAKTCVADESAENCDKSLHTLFGDKLCTVATLRETYGEMADCCAKQEPERNECFLQHKDDNPNLPRLVRPEVDVMCTAFHDNEETFLKKYLYEIARRHPYFYAPELLFFAKRYKAAFTECCQAADKAACLLPKLDELRDEGKASSAKQRLKCASLQKFGERAFKAWAVARLSQRFPKAEFAEVSKLVTDLTKVHTECCHGDLLECADDRADLAKYICENQDSISSKLKECCEKPLLEKSHCIAEVENDEMPADLPSLAADFVESKDVCKNYAEAKDVFLGMFLYEYARRHPDYSVVLLLRLAKTYETTLEKCCAAADPHECYAKVFDEFKPLVEEPQNLIKQNCELFEQLGEYKFQNALLVRYTKKVPQVSTPTLVEVSRNLGKVGSKCCKHPEAKRMPCAEDYLSVVLNQLCVLHEKTPVSDRVTKCCTESLVNRRPCFSALEVDETYVPKEFQAETFTFHADICTLSEKERQIKKQTALVELVKHKPKATKEQLKAVMDDFAAFVEKCCKADDKETCFAEEGKKLVAASQAALGLGSGGSGGGSGGSGGGAQVLRGTVTDFPGFDERADAETLRKAMKGLGTDEESILTLLTSRSNAQRQEISAAFKTLFGADLLDDLASELTGKFEKLIVALMKPSRLYDAYELKHALAGAGTNEKVLTEIIASRTPEELRAIKQVYEEEYGSSLAGDVVGDTSGYYQRMLVVLLQAARDPDAGIDEAQVEQDAQALFQAGELKWGTDEEKFITIFGTRSVSHLRKVFDKYMTISGFQIEETIDRETSGNLEQLLLAVVKSIRSIPAYLAETLYYAMKGAGTDDHTLIRVMVSRSEIDLFNIRKEFRKNFATSLYSMIKGDTSGDYKKALLLLCGEDD

SEQ ID NO: 75 - protein, 1017 aa, Artificial Sequence
  Synthetic construct
MFPAMPLSSLFVNGPRTLCGAELVDALQFVCGDRGFYFNKPTGYGSSSRRAPQTGIVDECCFRSCDLRRLEMYCAPLKPAKSAGSGGSGGGSGGSGGGDAHKSEVAHRFKDLGEENFKALVLIAFAQYLQQSPFEDHVKLVNEVTEFAKTCVADESAENCDKSLHTLFGDKLCTVATLRETYGEMADCCAKQEPERNECFLQHKDDNPNLPRLVRPEVDVMCTAFHDNEETFLKKYLYEIARRHPYFYAPELLFFAKRYKAAFTECCQAADKAACLLPKLDELRDEGKASSAKQRLKCASLQKFGERAFKAWAVARLSQRFPKAEFAEVSKLVTDLTKVHTECCHGDLLECADDRADLAKYICENQDSISSKLKECCEKPLLEKSHCIAEVENDEMPADLPSLAADFVESKDVCKNYAEAKDVFLGMFLYEYARRHPDYSVVLLLRLAKTYETTLEKCCAAADPHECYAKVFDEFKPLVEEPQNLIKQNCELFEQLGEYKFQNALLVRYTKKVPQVSTPTLVEVSRNLGKVGSKCCKHPEAKRMPCAEDYLSVVLNQLCVLHEKTPVSDRVTKCCTESLVNRRPCFSALEVDETYVPKEFQAGTFTFHADICTLSEKERQIKKQTALVELVKHKPKATKEQLKAAMDDFAAFVEKCCKADDKETCFAEEGKKLVAASQAALGLGSGGSGGGSGGSGGGAQVLRGTVTDFPGFDERADAETLRKAMKGLGTDEESILTLLTSRSNAQRQEISAAFKTLFGADLLDDLASELTGKFEKLIVALMKPSRLYDAYELKHALAGAGTNEKVLTEIIASRTPEELRAIKQVYEEEYGSSLAGDVVGDTSGYYQRMLVVLLQAARDPDAGIDEAQVEQDAQALFQAGELKWGTDEEKFITIFGTRSVSHLRKVFDKYMTISGFQIEETIDRETSGNLEQLLLAVVKSIRSIPAYLAETLYYAMKGAGTDDHTLIRVMVSRSEIDLFNIRKEFRKNFATSLYSMIKGDTSGDYKKALLLLCGEDD

SEQ ID NO: 76 - protein, 1063 aa, Artificial Sequence
  Synthetic construct
MFPAMPLSSLFVNGPRTLCGAELVDALQFVCGDRGFYFNKPTGYGSSSRAPQTGIVDECCFRSCDLRRLEMYCAPLKPAGSGGSGGGSGGGSGGGSGGGSGGGSGGGSGGGSGGGSGGGDAHKSEVAHRFKDLGEENFKALVLIAFAQYLQQSPFEDHVKLVNEVTEFAKTCVADESAENCDKSLHTLFGDKLCTVATLRETYGEMADCCAKQEPERNECFLQHKDDNPNLPRLVRPEVDVMCTAFHDNEETFLKKYLYEIARRHPYFYAPELLFFAKRYKAAFTECCQAADKAACLLPKLDELRDEGKASSAKQRLKCASLQKFGERAFKAWAVARLSQRFPKAEFAEVSKLVTDLTKVHTECCHGDLLECADDRADLAKYICENQDSISSKLKECCEKPLLEKSHCIAEVENDEMPADLPSLAADFVESKDVCKNYAEAKDVFLGMFLYEYARRHPDYSVVLLLRLAKTYETTLEKCCAAADPHECYAKVFDEFKPLVEEPQNLIKQNCELFEQLGEYKFQNALLVRYTKKVPQVSTPTLVEVSRNLGKVGSKCCKHPEAKRMPCAEDYLSVVLNQLCVLHEKTPVSDRVTKCCTESLVNRRPCFSALEVDETYVPKEFQAETFTFHADICTLSEKERQIKKQTALVELVKHKPKATKEQLKAVMDDFAAFVEKCCKADDKETCFAEEGKKLVAASQAALGLGSGGSGGGSGGGSGGGSGGGSGGGSGGGSGGGSGGGSGGGAQVLRGTVTDFPGFDERADAETLRKAMKGLGTDEESILTLLTSRSNAQRQEISAAFKTLFGRDLLDDLKSELTGKFEKLIVALMKPSRLYDAYELKHALKGAGTNEKVLTEIIASRTPEELRAIKQVYEEEYGSSLEDDVVGDTSGYYQRMLVVLLQANRDPDAGIDEAQVEQDAQALFQAGELKWGTDEEKFITIFGTRSVSHLRKVFDKYMTISGFQIEETIDRETSGNLEQLLLAVVKSIRSIPAYLAETLYYAMKGAGTDDHTLIRVMVSRSEIDLFNIRKEFRKNFATSLYSMIKGDTSGDYKKALLLLCGEDD

SEQ ID NO: 77 - protein, 1017 aa, Artificial Sequence
  Synthetic construct
MFPAMPLSSLFVNGPRTLCGAELVDALQFVCGDRGFYFNKPTGYGSSSRRAPQTGIVDECCFRSCDLRRLEMLCAPLKPAKSAGSGGSGGGSGGSGGGDAHKSEVAHRFKDLGEENFKALVLIAFAQYLQQSPFEDHVKLVNEVTEFAKTCVADESAENCDKSLHTLFGDKLCTVATLRETYGEMADCCAKQEPERNECFLQHKDDNPNLPRLVRPEVDVMCTAFHDNEETFLKKYLYEIARRHPYFYAPELLFFAKRYKAAFTECCQAADKAACLLPKLDELRDEGKASSAKQRLKCASLQKFGERAFKAWAVARLSQRFPKAEFAEVSKLVTDLTKVHTECCHGDLLECADDRADLAKYICENQDSISSKLKECCEKPLLEKSHCIAEVENDEMPADLPSLAADFVESKDVCKNYAEAKDVFLGMFLYEYARRHPDYSVVLLLRLAKTYETTLEKCCAAADPHECYAKVFDEFKPLVEEPQNLIKQNCELFEQLGEYKFQNALLVRYTKKVPQVSTPTLVEVSRNLGKVGSKCCKHPEAKRMPCAEDYLSVVLNQLCVLHEKTPVSDRVTKCCTESLVNRRPCFSALEVDETYVPKEFQAGTFTFHADICTLSEKERQIKKQTALVELVKHKPKATKEQLKAAMDDFAAFVEKCCKADDKETCFAEEGKKLVAASQAALGLGSGGSGGGSGGSGGGAQVLRGTVTDFPGFDERADAETLRKAMKGLGTDEESILTLLTSRSNAQRQEISAAFKTLFGADLLDDLASELTGKFEKLIVALMKPSRLYDAYELKHALAGAGTNEKVLTEIIASRTPEELRAIKQVYEEEYGSSLAGDVVGDTSGYYQRMLVVLLQAARDPDAGIDEAQVEQDAQALFQAGELKWGTDEEKFITIFGTRSVSHLRKVFDKYMTISGFQIEETIDRETSGNLEQLLLAVVKSIRSIPAYLAETLYYAMKGAGTDDHTLIRVMVSRSEIDLFNIRKEFRKNFATSLYSMIKGDTSGDYKKALLLLCGEDD

SEQ ID NO: 78 - protein, 1001 aa, Artificial Sequence
  Synthetic construct
MFPAMPLSSLFVNGPRTLCGAELVDALQFVCGDRGFYFNKPTGYGSSSRRAPQTGIVDECCFRSCDLRRLEMYCAPLKPAKSAGSGGGSGDAHKSEVAHRFKDLGEENFKALVLIAFAQYLQQSPFEDHVKLVNEVTEFAKTCVADESAENCDKSLHTLFGDKLCTVATLRETYGEMADCCAKQEPERNECFLQHKDDNPNLPRLVRPEVDVMCTAFHDNEETFLKKYLYEIARRHPYFYAPELLFFAKRYKAAFTECCQAADKAACLLPKLDELRDEGKASSAKQRLKCASLQKFGERAFKAWAVARLSQRFPKAEFAEVSKLVTDLTKVHTECCHGDLLECADDRADLAKYICENQDSISSKLKECCEKPLLEKSHCIAEVENDEMPADLPSLAADFVESKDVCKNYAEAKDVFLGMFLYEYARRHPDYSVVLLLRLAKTYETTLEKCCAAADPHECYAKVFDEFKPLVEEPQNLIKQNCELFEQLGEYKFQNALLVRYTKKVPQVSTPTLVEVSRNLGKVGSKCCKHPEAKRMPCAEDYLSVVLNQLCVLHEKTPVSDRVTKCCTESLVNRRPCFSALEVDETYVPKEFQAETFTFHADICTLSEKERQIKKQTALVELVKHKPKATKEQLKAVMDDFAAFVEKCCKADDKETCFAEEGKKLVAASQAALGLGSGGGSGAQVLRGTVTDFPGFDERADAETLRKAMKGLGTDEESILTLLTSRSNAQRQEISAAFKTLFGRDLLDDLKSELTGKFEKLIVALMKPSRLYDAYELKHALKGAGTNEKVLTEIIASRTPEELRAIKQVYEEEYGSSLEDDVVGDTSGYYQRMLVVLLQANRDPDAGIDEAQVEQDAQALFQAGELKWGTDEEKFITIFGTRSVSHLRKVFDKYMTISGFQIEETIDRETSGNLEQLLLAVVKSIRSIPAYLAETLYYAMKGAGTDDHTLIRVMVSRSEIDLFNIRKEFRKNFATSLYSMIKGDTSGDYKKALLLLCGEDD

SEQ ID NO: 79 - protein, 1013 aa, Artificial Sequence
  Synthetic construct
MFPAMPLSSLFVNGPRTLCGAELVDALQFVCGDRGFYFNKPTGYGSSSRAPQTGIVDECCFRSCDLRRLEMYCAPLKPAGSGGSGGGSGGSGGGDAHKSEVAHRFKDLGEENFKALVLIAFAQYLQQSPFEDHVKLVNEVTEFAKTCVADESAENCDKSLHTLFGDKLCTVATLRETYGEMADCCAKQEPERNECFLQHKDDNPNLPRLVRPEVDVMCTAFHDNEETFLKKYLYEIARRHPYFYAPELLFFAKRYKAAFTECCQAADKAACLLPKLDELRDEGKASSAKQRLKCASLQKFGERAFKAWAVARLSQRFPKAEFAEVSKLVTDLTKVHTECCHGDLLECADDRADLAKYICENQDSISSKLKECCEKPLLEKSHCIAEVENDEMPADLPSLAADFVESKDVCKNYAEAKDVFLGMFLYEYARRHPDYSVVLLLRLAKTYETTLEKCCAAADPHECYAKVFDEFKPLVEEPQNLIKQNCELFEQLGEYKFQNALLVRYTKKVPQVSTPTLVEVSRNLGKVGSKCCKHPEAKRMPCAEDYLSVVLNQLCVLHEKTPVSDRVTKCCTESLVNRRPCFSALEVDETYVPKEFQAGTFTFHADICTLSEKERQIKKQTALVELVKHKPKATKEQLKAAMDDFAAFVEKCCKADDKETCFAEEGKKLVAASQAALGLGSGGSGGGSGGSGGGAQVLRGTVTDFPGFDERADAETLRKAMKGLGTDEESILTLLTSRSNAQRQEISAAFKTLFGADLLDDLASELTGKFEKLIVALMKPSRLYDAYELKHALAGAGTNEKVLTEIIASRTPEELRAIKQVYEEEYGSSLAGDVVGDTSGYYQRMLVVLLQAARDPDAGIDEAQVEQDAQALFQAGELKWGTDEEKFITIFGTRSVSHLRKVFDKYMTISGFQIEETIDRETSGNLEQLLLAVVKSIRSIPAYLAETLYYAMKGAGTDDHTLIRVMVSRSEIDLFNIRKEFRKNFATSLYSMIKGDTSGDYKKALLLLCGEDD

SEQ ID NO: 80 - protein, 1017 aa, Artificial Sequence
  Synthetic construct
MFPAMPLSSLFVNGPRTLCGAELVDALQFVCGDRGFLFNKPTGAGSSSRRAPQTGIVDECCFRSCDLRRLEMYCAPLKPAKSAGSGGSGGGSGGSGGGDAHKSEVAHRFKDLGEENFKALVLIAFAQYLQQSPFEDHVKLVNEVTEFAKTCVADESAENCDKSLHTLFGDKLCTVATLRETYGEMADCCAKQEPERNECFLQHKDDNPNLPRLVRPEVDVMCTAFHDNEETFLKKYLYEIARRHPYFYAPELLFFAKRYKAAFTECCQAADKAACLLPKLDELRDEGKASSAKQRLKCASLQKFGERAFKAWAVARLSQRFPKAEFAEVSKLVTDLTKVHTECCHGDLLECADDRADLAKYICENQDSISSKLKECCEKPLLEKSHCIAEVENDEMPADLPSLAADFVESKDVCKNYAEAKDVFLGMFLYEYARRHPDYSVVLLLRLAKTYETTLEKCCAAADPHECYAKVFDEFKPLVEEPQNLIKQNCELFEQLGEYKFQNALLVRYTKKVPQVSTPTLVEVSRNLGKVGSKCCKHPEAKRMPCAEDYLSVVLNQLCVLHEKTPVSDRVTKCCTESLVNRRPCFSALEVDETYVPKEFQAGTFTFHADICTLSEKERQIKKQTALVELVKHKPKATKEQLKAAMDDFAAFVEKCCKADDKETCFAEEGKKLVAASQAALGLGSGGSGGGSGGSGGGAQVLRGTVTDFPGFDERADAETLRKAMKGLGTDEESILTLLTSRSNAQRQEISAAFKTLFGADLLDDLASELTGKFEKLIVALMKPSRLYDAYELKHALAGAGTNEKVLTEIIASRTPEELRAIKQVYEEEYGSSLAGDVVGDTSGYYQRMLVVLLQAARDPDAGIDEAQVEQDAQALFQAGELKWGTDEEKFITIFGTRSVSHLRKVFDKYMTISGFQIEETIDRETSGNLEQLLLAVVKSIRSIPAYLAETLYYAMKGAGTDDHTLIRVMVSRSEIDLFNIRKEFRKNFATSLYSMIKGDTSGDYKKALLLLCGEDD

SEQ ID NO: 81 - protein, 1017 aa, Artificial Sequence
  Synthetic construct
MFPAMPLSSLFVNGPRTLCGAELVDALQFVCGDRGFLFNKPTGYGSSSRRAPQTGIVDECCFRSCDLRRLEMYCAPLKPAKSAGSGGSGGGSGGSGGGDAHKSEVAHRFKDLGEENFKALVLIAFAQYLQQSPFEDHVKLVNEVTEFAKTCVADESAENCDKSLHTLFGDKLCTVATLRETYGEMADCCAKQEPERNECFLQHKDDNPNLPRLVRPEVDVMCTAFHDNEETFLKKYLYEIARRHPYFYAPELLFFAKRYKAAFTECCQAADKAACLLPKLDELRDEGKASSAKQRLKCASLQKFGERAFKAWAVARLSQRFPKAEFAEVSKLVTDLTKVHTECCHGDLLECADDRADLAKYICENQDSISSKLKECCEKPLLEKSHCIAEVENDEMPADLPSLAADFVESKDVCKNYAEAKDVFLGMFLYEYARRHPDYSVVLLLRLAKTYETTLEKCCAAADPHECYAKVFDEFKPLVEEPQNLIKQNCELFEQLGEYKFQNALLVRYTKKVPQVSTPTLVEVSRNLGKVGSKCCKHPEAKRMPCAEDYLSVVLNQLCVLHEKTPVSDRVTKCCTESLVNRRPCFSALEVDETYVPKEFQAGTFTFHADICTLSEKERQIKKQTALVELVKHKPKATKEQLKAAMDDFAAFVEKCCKADDKETCFAEEGKKLVAASQAALGLGSGGSGGGSGGSGGGAQVLRGTVTDFPGFDERADAETLRKAMKGLGTDEESILTLLTSRSNAQRQEISAAFKTLFGADLLDDLASELTGKFEKLIVALMKPSRLYDAYELKHALAGAGTNEKVLTEIIASRTPEELRAIKQVYEEEYGSSLAGDVVGDTSGYYQRMLVVLLQAARDPDAGIDEAQVEQDAQALFQAGELKWGTDEEKFITIFGTRSVSHLRKVFDKYMTISGFQIEETIDRETSGNLEQLLLAVVKSIRSIPAYLAETLYYAMKGAGTDDHTLIRVMVSRSEIDLFNIRKEFRKNFATSLYSMIKGDTSGDYKKALLLLCGEDD

SEQ ID NO: 82 - protein, 1017 aa, Artificial Sequence
  Synthetic construct
MFPAMPLSSLFVNGPRTLCGAELVDALQFVCGDRGFYFNKPTGAGSSSRRAPQTGIVDECCFRSCDLRRLEMYCAPLKPAKSAGSGGSGGGSGGSGGGDAHKSEVAHRFKDLGEENFKALVLIAFAQYLQQSPFEDHVKLVNEVTEFAKTCVADESAENCDKSLHTLFGDKLCTVATLRETYGEMADCCAKQEPERNECFLQHKDDNPNLPRLVRPEVDVMCTAFHDNEETFLKKYLYEIARRHPYFYAPELLFFAKRYKAAFTECCQAADKAACLLPKLDELRDEGKASSAKQRLKCASLQKFGERAFKAWAVARLSQRFPKAEFAEVSKLVTDLTKVHTECCHGDLLECADDRADLAKYICENQDSISSKLKECCEKPLLEKSHCIAEVENDEMPADLPSLAADFVESKDVCKNYAEAKDVFLGMFLYEYARRHPDYSVVLLLRLAKTYETTLEKCCAAADPHECYAKVFDEFKPLVEEPQNLIKQNCELFEQLGEYKFQNALLVRYTKKVPQVSTPTLVEVSRNLGKVGSKCCKHPEAKRMPCAEDYLSVVLNQLCVLHEKTPVSDRVTKCCTESLVNRRPCFSALEVDETYVPKEFQAGTFTFHADICTLSEKERQIKKQTALVELVKHKPKATKEQLKAAMDDFAAFVEKCCKADDKETCFAEEGKKLVAASQAALGLGSGGSGGGSGGSGGGAQVLRGTVTDFPGFDERADAETLRKAMKGLGTDEESILTLLTSRSNAQRQEISAAFKTLFGADLLDDLASELTGKFEKLIVALMKPSRLYDAYELKHALAGAGTNEKVLTEIIASRTPEELRAIKQVYEEEYGSSLAGDVVGDTSGYYQRMLVVLLQAARDPDAGIDEAQVEQDAQALFQAGELKWGTDEEKFITIFGTRSVSHLRKVFDKYMTISGFQIEETIDRETSGNLEQLLLAVVKSIRSIPAYLAETLYYAMKGAGTDDHTLIRVMVSRSEIDLFNIRKEFRKNFATSLYSMIKGDTSGDYKKALLLLCGEDD

SEQ ID NO: 83 - protein, 1001 aa, Artificial Sequence
  Synthetic construct
MFPAMPLSSLFVNGPRTLCGAELVDALQFVCGDRGFLFNKPTGYGSSSRRAPQTGIVDECCFRSCDLRRLEMYCAPLKPAKSAGSGGGSGDAHKSEVAHRFKDLGEENFKALVLIAFAQYLQQSPFEDHVKLVNEVTEFAKTCVADESAENCDKSLHTLFGDKLCTVATLRETYGEMADCCAKQEPERNECFLQHKDDNPNLPRLVRPEVDVMCTAFHDNEETFLKKYLYEIARRHPYFYAPELLFFAKRYKAAFTECCQAADKAACLLPKLDELRDEGKASSAKQRLKCASLQKFGERAFKAWAVARLSQRFPKAEFAEVSKLVTDLTKVHTECCHGDLLECADDRADLAKYICENQDSISSKLKECCEKPLLEKSHCIAEVENDEMPADLPSLAADFVESKDVCKNYAEAKDVFLGMFLYEYARRHPDYSVVLLLRLAKTYETTLEKCCAAADPHECYAKVFDEFKPLVEEPQNLIKQNCELFEQLGEYKFQNALLVRYTKKVPQVSTPTLVEVSRNLGKVGSKCCKHPEAKRMPCAEDYLSVVLNQLCVLHEKTPVSDRVTKCCTESLVNRRPCFSALEVDETYVPKEFQAETFTFHADICTLSEKERQIKKQTALVELVKHKPKATKEQLKAVMDDFAAFVEKCCKADDKETCFAEEGKKLVAASQAALGLGSGGGSGAQVLRGTVTDFPGFDERADAETLRKAMKGLGTDEESILTLLTSRSNAQRQEISAAFKTLFGADLLDDLASELTGKFEKLIVALMKPSRLYDAYELKHALAGAGTNEKVLTEIIASRTPEELRAIKQVYEEEYGSSLAGDVVGDTSGYYQRMLVVLLQAARDPDAGIDEAQVEQDAQALFQAGELKWGTDEEKFITIFGTRSVSHLRKVFDKYMTISGFQIEETIDRETSGNLEQLLLAVVKSIRSIPAYLAETLYYAMKGAGTDDHTLIRVMVSRSEIDLFNIRKEFRKNFATSLYSMIKGDTSGDYKKALLLLCGEDD

SEQ ID NO: 84 - protein, 1001 aa, Artificial Sequence
  Synthetic construct
MFPAMPLSSLFVNGPRTLCGAELVDALQFVCGDRGFYFNKPTGAGSSSRRAPQTGIVDECCFRSCDLRRLEMYCAPLKPAKSAGSGGGSGDAHKSEVAHRFKDLGEENFKALVLIAFAQYLQQSPFEDHVKLVNEVTEFAKTCVADESAENCDKSLHTLFGDKLCTVATLRETYGEMADCCAKQEPERNECFLQHKDDNPNLPRLVRPEVDVMCTAFHDNEETFLKKYLYEIARRHPYFYAPELLFFAKRYKAAFTECCQAADKAACLLPKLDELRDEGKASSAKQRLKCASLQKFGERAFKAWAVARLSQRFPKAEFAEVSKLVTDLTKVHTECCHGDLLECADDRADLAKYICENQDSISSKLKECCEKPLLEKSHCIAEVENDEMPADLPSLAADFVESKDVCKNYAEAKDVFLGMFLYEYARRHPDYSVVLLLRLAKTYETTLEKCCAAADPHECYAKVFDEFKPLVEEPQNLIKQNCELFEQLGEYKFQNALLVRYTKKVPQVSTPTLVEVSRNLGKVGSKCCKHPEAKRMPCAEDYLSVVLNQLCVLHEKTPVSDRVTKCCTESLVNRRPCFSALEVDETYVPKEFQAETFTFHADICTLSEKERQIKKQTALVELVKHKPKATKEQLKAVMDDFAAFVEKCCKADDKETCFAEEGKKLVAASQAALGLGSGGGSGAQVLRGTVTDFPGFDERADAETLRKAMKGLGTDEESILTLLTSRSNAQRQEISAAFKTLFGADLLDDLASELTGKFEKLIVALMKPSRLYDAYELKHALAGAGTNEKVLTEIIASRTPEELRAIKQVYEEEYGSSLAGDVVGDTSGYYQRMLVVLLQAARDPDAGIDEAQVEQDAQALFQAGELKWGTDEEKFITIFGTRSVSHLRKVFDKYMTISGFQIEETIDRETSGNLEQLLLAVVKSIRSIPAYLAETLYYAMKGAGTDDHTLIRVMVSRSEIDLFNIRKEFRKNFATSLYSMIKGDTSGDYKKALLLLCGEDD

SEQ ID NO: 85 - protein, 1001 aa, Artificial Sequence
  Synthetic construct
MFPAMPLSSLFVNGPRTLCGAELVDALQFVCGDRGFYFNKPTGYGSSSRRAPQTGIVDECCFRSCDLRRLEMLCAPLKPAKSAGSGGGSGDAHKSEVAHRFKDLGEENFKALVLIAFAQYLQQSPFEDHVKLVNEVTEFAKTCVADESAENCDKSLHTLFGDKLCTVATLRETYGEMADCCAKQEPERNECFLQHKDDNPNLPRLVRPEVDVMCTAFHDNEETFLKKYLYEIARRHPYFYAPELLFFAKRYKAAFTECCQAADKAACLLPKLDELRDEGKASSAKQRLKCASLQKFGERAFKAWAVARLSQRFPKAEFAEVSKLVTDLTKVHTECCHGDLLECADDRADLAKYICENQDSISSKLKECCEKPLLEKSHCIAEVENDEMPADLPSLAADFVESKDVCKNYAEAKDVFLGMFLYEYARRHPDYSVVLLLRLAKTYETTLEKCCAAADPHECYAKVFDEFKPLVEEPQNLIKQNCELFEQLGEYKFQNALLVRYTKKVPQVSTPTLVEVSRNLGKVGSKCCKHPEAKRMPCAEDYLSVVLNQLCVLHEKTPVSDRVTKCCTESLVNRRPCFSALEVDETYVPKEFQAETFTFHADICTLSEKERQIKKQTALVELVKHKPKATKEQLKAVMDDFAAFVEKCCKADDKETCFAEEGKKLVAASQAALGLGSGGGSGAQVLRGTVTDFPGFDERADAETLRKAMKGLGTDEESILTLLTSRSNAQRQEISAAFKTLFGADLLDDLASELTGKFEKLIVALMKPSRLYDAYELKHALAGAGTNEKVLTEIIASRTPEELRAIKQVYEEEYGSSLAGDVVGDTSGYYQRMLVVLLQAARDPDAGIDEAQVEQDAQALFQAGELKWGTDEEKFITIFGTRSVSHLRKVFDKYMTISGFQIEETIDRETSGNLEQLLLAVVKSIRSIPAYLAETLYYAMKGAGTDDHTLIRVMVSRSEIDLFNIRKEFRKNFATSLYSMIKGDTSGDYKKALLLLCGEDD

SEQ ID NO: 86 - protein, 997 aa, Artificial Sequence
  Synthetic construct
MFPAMPLSSLFVNGPRTLCGAELVDALQFVCGDRGFYFNKPTGYGSSSRAPQTGIVDECCFRSCDLRRLEMYCAPLKPAGSGGGSGDAHKSEVAHRFKDLGEENFKALVLIAFAQYLQQSPFEDHVKLVNEVTEFAKTCVADESAENCDKSLHTLFGDKLCTVATLRETYGEMADCCAKQEPERNECFLQHKDDNPNLPRLVRPEVDVMCTAFHDNEETFLKKYLYEIARRHPYFYAPELLFFAKRYKAAFTECCQAADKAACLLPKLDELRDEGKASSAKQRLKCASLQKFGERAFKAWAVARLSQRFPKAEFAEVSKLVTDLTKVHTECCHGDLLECADDRADLAKYICENQDSISSKLKECCEKPLLEKSHCIAEVENDEMPADLPSLAADFVESKDVCKNYAEAKDVFLGMFLYEYARRHPDYSVVLLLRLAKTYETTLEKCCAAADPHECYAKVFDEFKPLVEEPQNLIKQNCELFEQLGEYKFQNALLVRYTKKVPQVSTPTLVEVSRNLGKVGSKCCKHPEAKRMPCAEDYLSVVLNQLCVLHEKTPVSDRVTKCCTESLVNRRPCFSALEVDETYVPKEFQAETFTFHADICTLSEKERQIKKQTALVELVKHKPKATKEQLKAVMDDFAAFVEKCCKADDKETCFAEEGKKLVAASQAALGLGSGGGSGAQVLRGTVTDFPGFDERADAETLRKAMKGLGTDEESILTLLTSRSNAQRQEISAAFKTLFGADLLDDLASELTGKFEKLIVALMKPSRLYDAYELKHALAGAGTNEKVLTEIIASRTPEELRAIKQVYEEEYGSSLAGDVVGDTSGYYQRMLVVLLQAARDPDAGIDEAQVEQDAQALFQAGELKWGTDEEKFITIFGTRSVSHLRKVFDKYMTISGFQIEETIDRETSGNLEQLLLAVVKSIRSIPAYLAETLYYAMKGAGTDDHTLIRVMVSRSEIDLFNIRKEFRKNFATSLYSMIKGDTSGDYKKALLLLCGEDD

SEQ ID NO: 87 - DNA, 2046 bp, Artificial Sequence
  Synthetic construct
atgttcccagccatgcccttgtccagcctgtttgttaacggcccaagaacactttgtggagccgaactggtggatgctctccaattcgtttgcggcgaccgcggattctactttaacaagcccaccggttacgggtcttcaagccgggccccgcagactggcatcgtcgacgagtgctgttttagaagctgcgatctgcgacggttggagatgtattgtgcacctctgaagcccgcgggaggagacgctcacaagtctgaagtggcacataggttcaaagatctgggcgaagagaactttaaggccctcgtcctgatcgctttcgcacagtacctccagcagtctccctttgaagatcacgtgaaactggtcaatgaggtgaccgaatttgccaagacatgcgtggctgatgagagtgcagaaaactgtgacaaatcactgcatactctctttggagataagctgtgcaccgtcgccacactcagagagacttatggggaaatggctgactgttgcgcaaaacaggagcctgaacggaatgagtgtttcctccagcacaaggatgacaacccaaatctgccccgcctcgtgcgacctgaggtcgatgtgatgtgcaccgcctttcatgacaacgaagagacattcctgaagaaatacctgtatgaaattgctcgtaggcacccatacttttatgcccccgagctcctgttctttgcaaagagatacaaagctgccttcactgaatgttgccaggcagctgataaggccgcatgtctcctgcctaaactggacgagctccgggatgaaggtaaggcttccagcgccaaacagcgcctgaagtgcgcttctctccagaagtttggcgagcgagcattcaaagcctgggctgtggcccgtctcagtcagaggtttccaaaggcagaatttgctgaggtgtcaaaactggtgaccgacctcacaaaggtccatactgagtgttgccacggagatctgctggaatgtgccgacgatagagcagacctcgctaaatatatctgcgagaatcaggattccattagctctaagctgaaagaatgttgcgagaagcccctcctggaaaagagtcattgtatcgccgaggtggaaaacgacgagatgccagcagatctgccatcactcgctgccgactttgtggaatccaaagatgtctgcaagaattacgcagaggctaaagacgtgttcctggggatgtttctgtatgagtacgcccggcgtcaccccgattatagcgtcgtgctcctgctccgactggcaaagacctacgaaacaactctggagaaatgttgcgctgccgcagaccctcatgaatgttatgctaaggtgttcgatgagtttaagccactcgtcgaagagccccagaacctgattaaacagaattgcgaactgttcgagcagctcggtgaatacaagtttcagaacgccctgctcgtgcgttataccaaaaaggtccctcaggtgtctacaccaactctggtggaggtcagtaggaatctgggcaaagtgggatcaaagtgttgcaaacaccccgaggcaaagagaatgccttgtgctgaagattacctctccgtcgtgctgaaccagctctgcgtgctgcatgaaaagaccccagtcagcgaccgggtgacaaaatgttgcaccgaatctctggtcaatcgccgaccctgtttcagtgccctcgaagtggacgaaacttatgtgcctaaggagtttcaggctgaaacattcacctttcacgccgatatctgcactctgtccgagaaagaaaggcagattaagaaacagacagcactggtcgagctcgtgaagcataaaccaaaggctaccaaggagcagctgaaagccgtcatggacgatttcgcagcttttgtggaaaagtgttgcaaagccgacgataaggagacttgtttcgcagaagaggggaaaaagctcgtggctgccagccaggcagctctgggtctgggcagtggtggctcaggtagcggccaccatcaccatcaccactaatga

SEQ ID NO: 88 - DNA, 3237 bp, Artificial Sequence
  Synthetic construct
atgttcccagccatgcccttgtccagcctgtttgttaacggcccaagaacactttgtggagccgaactggtggatgctctccaattcgtttgcggcgaccgcggattctactttaacaagcccaccggttacgggtcttcaagccgggccccgcagactggcatcgtcgacgagtgctgttttagaagctgcgatctgcgacggttggagatgtattgtgcacctctgaagcccgcgggttccggaggttctggcggtggatctgggggcggtagcggaggcggcagtggtggtggcagcgggggagggtcaggtgggggtagtggcggtggttctggaggtggttcaggaggaggagacgctcacaagtctgaagtggcacataggttcaaagatctgggcgaagagaactttaaggccctcgtcctgatcgctttcgcacagtacctccagcagtctccctttgaagatcacgtgaaactggtcaatgaggtgaccgaatttgccaagacatgcgtggctgatgagagtgcagaaaactgtgacaaatcactgcatactctctttggagataagctgtgcaccgtcgccacactcagagagacttatggggaaatggctgactgttgcgcaaaacaggagcctgaacggaatgagtgtttcctccagcacaaggatgacaacccaaatctgccccgcctcgtgcgacctgaggtcgatgtgatgtgcaccgcctttcatgacaacgaagagacattcctgaagaaatacctgtatgaaattgctcgtaggcacccatacttttatgcccccgagctcctgttctttgcaaagagatacaaagctgccttcactgaatgttgccaggcagctgataaggccgcatgtctcctgcctaaactggacgagctccgggatgaaggtaaggcttccagcgccaaacagcgcctgaagtgcgcttctctccagaagtttggcgagcgagcattcaaagcctgggctgtggcccgtctcagtcagaggtttccaaaggcagaatttgctgaggtgtcaaaactggtgaccgacctcacaaaggtccatactgagtgttgccacggagatctgctggaatgtgccgacgatagagcagacctcgctaaatatatctgcgagaatcaggattccattagctctaagctgaaagaatgttgcgagaagcccctcctggaaaagagtcattgtatcgccgaggtggaaaacgacgagatgccagcagatctgccatcactcgctgccgactttgtggaatccaaagatgtctgcaagaattacgcagaggctaaagacgtgttcctggggatgtttctgtatgagtacgcccggcgtcaccccgattatagcgtcgtgctcctgctccgactggcaaagacctacgaaacaactctggagaaatgttgcgctgccgcagaccctcatgaatgttatgctaaggtgttcgatgagtttaagccactcgtcgaagagccccagaacctgattaaacagaattgcgaactgttcgagcagctcggtgaatacaagtttcagaacgccctgctcgtgcgttataccaaaaaggtccctcaggtgtctacaccaactctggtggaggtcagtaggaatctgggcaaagtgggatcaaagtgttgcaaacaccccgaggcaaagagaatgccttgtgctgaagattacctctccgtcgtgctgaaccagctctgcgtgctgcatgaaaagaccccagtcagcgaccgggtgacaaaatgttgcaccgaatctctggtcaatcgccgaccctgtttcagtgccctcgaagtggacgaaacttatgtgcctaaggagtttcaggctgaaacattcacctttcacgccgatatctgcactctgtccgagaaagaaaggcagattaagaaacagacagcactggtcgagctcgtgaagcataaaccaaaggctaccaaggagcagctgaaagccgtcatggacgatttcgcagcttttgtggaaaagtgttgcaaagccgacgataaggagacttgtttcgcagaagaggggaaaaagctcgtggctgccagccaggcagctctgggtctggggtctggtggatcagggggaggttcaggcgggggcagtggcgggggatctggaggtggcagtgggggcggttccggaggtggatcaggaggaggaagtggcggcggtagcggtggtggtgctcaagtcttgcgtggtacggtgacagacttcccaggcttcgatgaaagagcggacgcggaaacacttcgaaaggcgatgaaagggctcggtactgacgaagagtccattttgacccttcttacgagcaggtcaaacgctcagaggcaagaaatctctgcagcctttaagacactctttggacgtgaccttcttgatgacctcaaatctgagctgacgggaaagtttgagaaactcatcgtagctttgatgaagcccagccgattgtatgatgcttacgaactgaaacacgccctgaaaggagcgggaacgaacgagaaagttttgactgagatcatcgcatcgcggaccccggaagagctcagagccatcaaacaagtctacgaggaggagtacggatcgtcattggaagatgacgtggtgggggatacgtcgggttactaccaacgaatgcttgtcgtgcttttgcaggcaaatcgcgacccggatgcggggatcgacgaggcccaagtggagcaagatgcgcaagcactcttccaggccggtgaactcaaatgggggaccgatgaagagaagtttatcaccatctttggcacgaggagtgtaagtcatctgcgtaaagtattcgataagtatatgacaatctcagggtttcagattgaggagacaattgacagggaaacctccggtaacttggagcagctcttgcttgccgtcgtcaagtccattcgctcgatccctgcgtatctggctgaaacactgtattacgccatgaaaggggcaggcactgatgaccacaccttgattagagttatggtgtcgcgatcagaaattgacttgttcaatatccggaaagagttccggaagaatttcgcaacgagcctctatagcatgatcaaaggggacacttcgggagattacaagaaagcgttgctccttctttcaggagaggatgacggcagtggtggctcaggtagcggccaccatcaccatcaccactaatga

SEQ ID NO: 89 - DNA, 2130 bp, Artificial Sequence
  Synthetic construct
atgttcccagccatgcccttgtccagcctgtttgttaacggcccaagaacactttgtggagccgaactggtggatgctctccaattcgtttgcggcgaccgcggattctactttaacaagcccaccggttacgggtcttcaagccggagggccccgcagactggcatcgtcgacgagtgctgttttagaagctgcgatctgcgacggttggagatgtattgtgcacctctgaagcccgcgaaaagtgctggttccggaggttctggcggtggatctgggggcggtagcggaggcggcagtggtggtggcagcgggggagggtcaggtgggggtagtggcggtggttctggaggtggttcaggaggaggagataagacccatacatgccctccgtgccccgcaccggaactcttgggtggcccatcagtctttctgttcccgccaaagcccaaagacacactgatgatttcgcgcacgcccgaagtcacttgcgtcgtggtggatgtgtcgcatgaggacccggaggtcaagttcaactggtacgtcgatggtgtagaagtccacaacgccaagaccaagcctcgggaggagcagtatcagtccacctaccgggtagtgagcgtgcttacagtgctccatcaggactggctgaacggcaaagaatacaaatgcaaagtcagcaacaaagcgctgccagcgcccatcgagaaaacaattagcaaagcgaaagggcagcccagagaacctcaagtgtatacattgccgccgtcgcgggaggaaatgacaaagaatcaggtatccctgacgtgtcttgtgaaaggcttttacccatccgacattgcggtagagtgggagtcgaatgggcaacccgagaacaactataagacgactcccccagtcttggattcagacggctcttttttcttgtactcgaaactcacagtcgacaagtccagatggcagcaggggaacgtgttcagctgcagcgtgatgcacgaggcccttcacaaccactatacgcagaaatcattaagcttatcgcctggggggtctggtggatcagggggaggttcaggcgggggcagtggcgggggatctggaggtggcagtgggggcggttccggaggtggatcaggaggaggaagtggcggcggtagcggtggtggtgctcaagtcttgcgtggtacggtgacagacttcccaggcttcgatgaaagagcggacgcggaaacacttcgaaaggcgatgaaagggctcggtactgacgaagagtccattttgacccttcttacgagcaggtcaaacgctcagaggcaagaaatctctgcagcctttaagacactctttggacgtgaccttcttgatgacctcaaatctgagctgacgggaaagtttgagaaactcatcgtagctttgatgaagcccagccgattgtatgatgcttacgaactgaaacacgccctgaaaggagcgggaacgaacgagaaagttttgactgagatcatcgcatcgcggaccccggaagagctcagagccatcaaacaagtctacgaggaggagtacggatcgtcattggaagatgacgtggtgggggatacgtcgggttactaccaacgaatgcttgtcgtgcttttgcaggcaaatcgcgacccggatgcggggatcgacgaggcccaagtggagcaagatgcgcaagcactcttccaggccggtgaactcaaatgggggaccgatgaagagaagtttatcaccatctttggcacgaggagtgtaagtcatctgcgtaaagtattcgataagtatatgacaatctcagggtttcagattgaggagacaattgacagggaaacctccggtaacttggagcagctcttgcttgccgtcgtcaagtccattcgctcgatccctgcgtatctggctgaaacactgtattacgccatgaaaggggcaggcactgatgaccacaccttgattagagttatggtgtcgcgatcagaaattgacttgttcaatatccggaaagagttccggaagaatttcgcaacgagcctctatagcatgatcaaaggggacacttcgggagattacaagaaagcgttgctccttctttcaggagaggatgactaatga

SEQ ID NO: 90 - DNA, 1038 bp, Artificial Sequence
  Synthetic construct
atgttcccagccatgcccttgtccagcctgtttgttaacggcccaagaacactttgtggagccgaactggtggatgctctccaattcgtttgcggcgaccgcggattctactttaacaagcccaccggttacgggtcttcaagccgggccccgcagactggcatcgtcgacgagtgctgttttagaagctgcgatctgcgacggttggagatgtattgtgcacctctgaagcccgcgggttccggaggttctggcggtggatctgggggcggtagcggaggcggcagtggtggtggcagcgggggagggtcaggtgggggtagtggcggtggttctggaggtggttcaggaggaggagataagacccatacatgccctccgtgccccgcaccggaactcttgggtggcccatcagtctttctgttcccgccaaagcccaaagacacactgatgatttcgcgcacgcccgaagtcacttgcgtcgtggtggatgtgtcgcatgaggacccggaggtcaagttcaactggtacgtcgatggtgtagaagtccacaacgccaagaccaagcctcgggaggagcagtatcagtccacctaccgggtagtgagcgtgcttacagtgctccatcaggactggctgaacggcaaagaatacaaatgcaaagtcagcaacaaagcgctgccagcgcccatcgagaaaacaattagcaaagcgaaagggcagcccagagaacctcaagtgtatacattgccgccgtcgcgggaggaaatgacaaagaatcaggtatccctgacgtgtcttgtgaaaggcttttacccatccgacattgcggtagagtgggagtcgaatgggcaacccgagaacaactataagacgactcccccagtcttggattcagacggatcctttttcttgtactcgaaactcacagtcgacaagtccagatggcagcaggggaacgtgttcagctgcagcgtgatgcacgaggcccttcacaaccactatacgcagaaatcattaagcttatcgcctgggtaa

SEQ ID NO: 91 - DNA, 3053 bp, Artificial Sequence
  Synthetic construct
tgttcccagccatgcccttgtccagcctgtttgttaacggcccaagaacactttgtggagccgaactggtggatgctctccaattcgtttgcggcgaccgcggattctactttaacaagcccaccggttacgggtcttcaagccggagggccccgcagactggcatcgtcgacgagtgctgttttagaagctgcgatctgcgacggttggagatgtattgtgcacctctgaagcccgcgaaaagtgctggttccggagggagcggtggtgggagtggcggatctggtggaggagacgctcacaagtctgaagtggcacataggttcaaagatctgggcgaagagaactttaaggccctcgtcctgatcgctttcgcacagtacctccagcagtctccctttgaagatcacgtgaaactggtcaatgaggtgaccgaatttgccaagacatgcgtggctgatgagagtgcagaaaactgtgacaaatcactgcatactctctttggagataagctgtgcaccgtcgccacactcagagagacttatggggaaatggctgactgttgcgcaaaacaggagcctgaacggaatgagtgtttcctccagcacaaggatgacaacccaaatctgccccgcctcgtgcgacctgaggtcgatgtgatgtgcaccgcctttcatgacaacgaagagacattcctgaagaaatacctgtatgaaattgctcgtaggcacccatacttttatgcccccgagctcctgttctttgcaaagagatacaaagctgccttcactgaatgttgccaggcagctgataaggccgcatgtctcctgcctaaactggacgagctccgggatgaaggtaaggcttccagcgccaaacagcgcctgaagtgcgcttctctccagaagtttggcgagcgagcattcaaagcctgggctgtggcccgtctcagtcagaggtttccaaaggcagaatttgctgaggtgtcaaaactggtgaccgacctcacaaaggtccatactgagtgttgccacggagatctgctggaatgtgccgacgatagagcagacctcgctaaatatatctgcgagaatcaggattccattagctctaagctgaaagaatgttgcgagaagcccctcctggaaaagagtcattgtatcgccgaggtggaaaacgacgagatgccagcagatctgccatcactcgctgccgactttgtggaatccaaagatgtctgcaagaattacgcagaggctaaagacgtgttcctggggatgtttctgtatgagtacgcccggcgtcaccccgattatagcgtcgtgctcctgctccgactggcaaagacctacgaaacaactctggagaaatgttgcgctgccgcagaccctcatgaatgttatgctaaggtgttcgatgagtttaagccactcgtcgaagagccccagaacctgattaaacagaattgcgaactgttcgagcagctcggtgaatacaagtttcagaacgccctgctcgtgcgttataccaaaaaggtccctcaggtgtctacaccaactctggtggaggtcagtaggaatctgggcaaagtgggatcaaagtgttgcaaacaccccgaggcaaagagaatgccttgtgctgaagattacctctccgtcgtgctgaaccagctctgcgtgctgcatgaaaagaccccagtcagcgaccgggtgacaaaatgttgcaccgaatctctggtcaatcgccgaccctgtttcagtgccctcgaagtggacgaaacttatgtgcctaaggagtttcaggctgaaacattcacctttcacgccgatatctgcactctgtccgagaaagaaaggcagattaagaaacagacagcactggtcgagctcgtgaagcataaaccaaaggctaccaaggagcagctgaaagccgtcatggacgatttcgcagcttttgtggaaaagtgttgcaaagccgacgataaggagacttgtttcgcagaagaggggaaaaagctcgtggctgccagccaggcagctctgggtctggggtctggcggttcagggggaggaagtggaggctcaggaggtggtgctcaagtcttgcgtggtacggtgacagacttcccaggcttcgatgaaagagcggacgcggaaacacttcgaaaggcgatgaaagggctcggtactgacgaagagtccattttgacccttcttacgagcaggtcaaacgctcagaggcaagaaatctctgcagcctttaagacactctttggacgtgaccttcttgatgacctcaaatctgagctgacgggaaagtttgagaaactcatcgtagctttgatgaagcccagccgattgtatgatgcttacgaactgaaacacgccctgaaaggagcgggaacgaacgagaaagttttgactgagatcatcgcatcgcggaccccggaagagctcagagccatcaaacaagtctacgaggaggagtacggatcgtcattggaagatgacgtggtgggggatacgtcgggttactaccaacgaatgcttgtcgtgcttttgcaggcaaatcgcgacccggatgcggggatcgacgaggcccaagtggagcaagatgcgcaagcactcttccaggccggtgaactcaaatgggggaccgatgaagagaagtttatcaccatctttggcacgaggagtgtaagtcatctgcgtaaagtattcgataagtatatgacaatctcagggtttcagattgaggagacaattgacagggaaacctccggtaacttggagcagctcttgcttgccgtcgtcaagtccattcgctcgatccctgcgtatctggctgaaacactgtattacgccatgaaaggggcaggcactgatgaccacaccttgattagagttatggtgtcgcgatcagaaattgacttgttcaatatccggaaagagttccggaagaatttcgcaacgagcctctatagcatgatcaaaggggacacttcgggagattacaagaaagcgttgctccttctttgcggagaggatgactaa

SEQ ID NO: 92 - DNA, 3057 bp, Artificial Sequence
  Synthetic construct
atgttcccagccatgcccttgtccagcctgtttgttaacggcccaagaacactttgtggagccgaactggtggatgctctccaattcgtttgcggcgaccgcggattctactttaacaagcccaccggttacgggtcttcaagccggagggccccgcagactggcatcgtcgacgagtgctgttttagaagctgcgatctgcgacggttggagatgtattgtgcacctctgaagcccgcgaaaagtgctggttccggagggagcggtggtgggagtggcggatctggtggaggagacgctcacaagtctgaagtggcacataggttcaaagatctgggcgaagagaactttaaggccctcgtcctgatcgctttcgcacagtacctccagcagtctccctttgaagatcacgtgaaactggtcaatgaggtgaccgaatttgccaagacatgcgtggctgatgagagtgcagaaaactgtgacaaatcactgcatactctctttggagataagctgtgcaccgtcgccacactcagagagacttatggggaaatggctgactgttgcgcaaaacaggagcctgaacggaatgagtgtttcctccagcacaaggatgacaacccaaatctgccccgcctcgtgcgacctgaggtcgatgtgatgtgcaccgcctttcatgacaacgaagagacattcctgaagaaatacctgtatgaaattgctcgtaggcacccatacttttatgcccccgagctcctgttctttgcaaagagatacaaagctgccttcactgaatgttgccaggcagctgataaggccgcatgtctcctgcctaaactggacgagctccgggatgaaggtaaggcttccagcgccaaacagcgcctgaagtgcgcttctctccagaagtttggcgagcgagcattcaaagcctgggctgtggcccgtctcagtcagaggtttccaaaggcagaatttgctgaggtgtcaaaactggtgaccgacctcacaaaggtccatactgagtgttgccacggagatctgctggaatgtgccgacgatagagcagacctcgctaaatatatctgcgagaatcaggattccattagctctaagctgaaagaatgttgcgagaagcccctcctggaaaagagtcattgtatcgccgaggtggaaaacgacgagatgccagcagatctgccatcactcgctgccgactttgtggaatccaaagatgtctgcaagaattacgcagaggctaaagacgtgttcctggggatgtttctgtatgagtacgcccggcgtcaccccgattatagcgtcgtgctcctgctccgactggcaaagacctacgaaacaactctggagaaatgttgcgctgccgcagaccctcatgaatgttatgctaaggtgttcgatgagtttaagccactcgtcgaagagccccagaacctgattaaacagaattgcgaactgttcgagcagctcggtgaatacaagtttcagaacgccctgctcgtgcgttataccaaaaaggtccctcaggtgtctacaccaactctggtggaggtcagtaggaatctgggcaaagtgggatcaaagtgttgcaaacaccccgaggcaaagagaatgccttgtgctgaagattacctctccgtcgtgctgaaccagctctgcgtgctgcatgaaaagaccccagtcagcgaccgggtgacaaaatgttgcaccgaatctctggtcaatcgccgaccctgtttcagtgccctcgaagtggacgaaacttatgtgcctaaggagtttcaggctgaaacattcacctttcacgccgatatctgcactctgtccgagaaagaaaggcagattaagaaacagacagcactggtcgagctcgtgaagcataaaccaaaggctaccaaggagcagctgaaagccgtcatggacgatttcgcagcttttgtggaaaagtgttgcaaagccgacgataaggagacttgtttcgcagaagaggggaaaaagctcgtggctgccagccaggcagctctgggtctggggtctggcggttcagggggaggaagtggaggctcaggaggtggtgctcaagtcttgcgtggtacggtgacagacttcccaggcttcgatgaaagagcggacgcggaaacacttcgaaaggcgatgaaagggctcggtactgacgaagagtccattttgacccttcttacgagcaggtcaaacgctcagaggcaagaaatctctgcagcctttaagacactctttggagctgaccttcttgatgacctcgcatctgagctgacgggaaagtttgagaaactcatcgtagctttgatgaagcccagccgattgtatgatgcttacgaactgaaacacgccctggctggagcgggaacgaacgagaaagttttgactgagatcatcgcatcgcggaccccggaagagctcagagccatcaaacaagtctacgaggaggagtacggatcgtcattggcaggagacgtggtgggggatacgtcgggttactaccaacgaatgcttgtcgtgcttttgcaggcagctcgcgacccggatgcggggatcgacgaggcccaagtggagcaagatgcgcaagcactcttccaggccggtgaactcaaatgggggaccgatgaagagaagtttatcaccatctttggcacgaggagtgtaagtcatctgcgtaaagtattcgataagtatatgacaatctcagggtttcagattgaggagacaattgacagggaaacctccggtaacttggagcagctcttgcttgccgtcgtcaagtccattcgctcgatccctgcgtatctggctgaaacactgtattacgccatgaaaggggcaggcactgatgaccacaccttgattagagttatggtgtcgcgatcagaaattgacttgttcaatatccggaaagagttccggaagaatttcgcaacgagcctctatagcatgatcaaaggggacacttcgggagattacaagaaagcgttgctccttctttgcggagaggatgactaatga

SEQ ID NO: 93 - DNA, 3057 bp, Artificial Sequence
  Synthetic construct
atgttcccagccatgcccttgtccagcctgtttgttaacggcccaagaacactttgtggagccgaactggtggatgctctccaattcgtttgcggcgaccgcggattctactttaacaagcccaccggttacgggtcttcaagccggagggccccgcagactggcatcgtcgacgagtgctgttttagaagctgcgatctgcgacggttggagatgtattgtgcacctctgaagcccgcgaaaagtgctggttccggagggagcggtggtgggagtggcggatctggtggaggagacgctcacaagtctgaagtggcacataggttcaaagatctgggcgaagagaactttaaggccctcgtcctgatcgctttcgcacagtacctccagcagtctccctttgaagatcacgtgaaactggtcaatgaggtgaccgaatttgccaagacatgcgtggctgatgagagtgcagaaaactgtgacaaatcactgcatactctctttggagataagctgtgcaccgtcgccacactcagagagacttatggggaaatggctgactgttgcgcaaaacaggagcctgaacggaatgagtgtttcctccagcacaaggatgacaacccaaatctgccccgcctcgtgcgacctgaggtcgatgtgatgtgcaccgcctttcatgacaacgaagagacattcctgaagaaatacctgtatgaaattgctcgtaggcacccatacttttatgcccccgagctcctgttctttgcaaagagatacaaagctgccttcactgaatgttgccaggcagctgataaggccgcatgtctcctgcctaaactggacgagctccgggatgaaggtaaggcttccagcgccaaacagcgcctgaagtgcgcttctctccagaagtttggcgagcgagcattcaaagcctgggctgtggcccgtctcagtcagaggtttccaaaggcagaatttgctgaggtgtcaaaactggtgaccgacctcacaaaggtccatactgagtgttgccacggagatctgctggaatgtgccgacgatagagcagacctcgctaaatatatctgcgagaatcaggattccattagctctaagctgaaagaatgttgcgagaagcccctcctggaaaagagtcattgtatcgccgaggtggaaaacgacgagatgccagcagatctgccatcactcgctgccgactttgtggaatccaaagatgtctgcaagaattacgcagaggctaaagacgtgttcctggggatgtttctgtatgagtacgcccggcgtcaccccgattatagcgtcgtgctcctgctccgactggcaaagacctacgaaacaactctggagaaatgttgcgctgccgcagaccctcatgaatgttatgctaaggtgttcgatgagtttaagccactcgtcgaagagccccagaacctgattaaacagaattgcgaactgttcgagcagctcggtgaatacaagtttcagaacgccctgctcgtgcgttataccaaaaaggtccctcaggtgtctacaccaactctggtggaggtcagtaggaatctgggcaaagtgggatcaaagtgttgcaaacaccccgaggcaaagagaatgccttgtgctgaagattacctctccgtcgtgctgaaccagctctgcgtgctgcatgaaaagaccccagtcagcgaccgggtgacaaaatgttgcaccgaatctctggtcaatcgccgaccctgtttcagtgccctcgaagtggacgaaacttatgtgcctaaggagtttcaggctggaacattcacctttcacgccgatatctgcactctgtccgagaaagaaaggcagattaagaaacagacagcactggtcgagctcgtgaagcataaaccaaaggctaccaaggagcagctgaaagccgccatggacgatttcgcagcttttgtggaaaagtgttgcaaagccgacgataaggagacttgtttcgcagaagaggggaaaaagctcgtggctgccagccaggcagctctgggtctggggtctggcggttcagggggaggaagtggaggctcaggaggtggtgctcaagtcttgcgtggtacggtgacagacttcccaggcttcgatgaaagagcggacgcggaaacacttcgaaaggcgatgaaagggctcggtactgacgaagagtccattttgacccttcttacgagcaggtcaaacgctcagaggcaagaaatctctgcagcctttaagacactctttggagctgaccttcttgatgacctcgcatctgagctgacgggaaagtttgagaaactcatcgtagctttgatgaagcccagccgattgtatgatgcttacgaactgaaacacgccctggctggagcgggaacgaacgagaaagttttgactgagatcatcgcatcgcggaccccggaagagctcagagccatcaaacaagtctacgaggaggagtacggatcgtcattggcaggagacgtggtgggggatacgtcgggttactaccaacgaatgcttgtcgtgcttttgcaggcagctcgcgacccggatgcggggatcgacgaggcccaagtggagcaagatgcgcaagcactcttccaggccggtgaactcaaatgggggaccgatgaagagaagtttatcaccatctttggcacgaggagtgtaagtcatctgcgtaaagtattcgataagtatatgacaatctcagggtttcagattgaggagacaattgacagggaaacctccggtaacttggagcagctcttgcttgccgtcgtcaagtccattcgctcgatccctgcgtatctggctgaaacactgtattacgccatgaaaggggcaggcactgatgaccacaccttgattagagttatggtgtcgcgatcagaaattgacttgttcaatatccggaaagagttccggaagaatttcgcaacgagcctctatagcatgatcaaaggggacacttcgggagattacaagaaagcgttgctccttctttgcggagaggatgactaatga

SEQ ID NO: 94 - DNA, 3195 bp, Artificial Sequence
  Synthetic construct
atgttcccagccatgcccttgtccagcctgtttgttaacggcccaagaacactttgtggagccgaactggtggatgctctccaattcgtttgcggcgaccgcggattctactttaacaagcccaccggttacgggtcttcaagccgggccccgcagactggcatcgtcgacgagtgctgttttagaagctgcgatctgcgacggttggagatgtattgtgcacctctgaagcccgcgggttccggaggttctggcggtggatctgggggcggtagcggaggcggcagtggtggtggcagcgggggagggtcaggtgggggtagtggcggtggttctggaggtggttcaggaggaggagacgctcacaagtctgaagtggcacataggttcaaagatctgggcgaagagaactttaaggccctcgtcctgatcgctttcgcacagtacctccagcagtctccctttgaagatcacgtgaaactggtcaatgaggtgaccgaatttgccaagacatgcgtggctgatgagagtgcagaaaactgtgacaaatcactgcatactctctttggagataagctgtgcaccgtcgccacactcagagagacttatggggaaatggctgactgttgcgcaaaacaggagcctgaacggaatgagtgtttcctccagcacaaggatgacaacccaaatctgccccgcctcgtgcgacctgaggtcgatgtgatgtgcaccgcctttcatgacaacgaagagacattcctgaagaaatacctgtatgaaattgctcgtaggcacccatacttttatgcccccgagctcctgttctttgcaaagagatacaaagctgccttcactgaatgttgccaggcagctgataaggccgcatgtctcctgcctaaactggacgagctccgggatgaaggtaaggcttccagcgccaaacagcgcctgaagtgcgcttctctccagaagtttggcgagcgagcattcaaagcctgggctgtggcccgtctcagtcagaggtttccaaaggcagaatttgctgaggtgtcaaaactggtgaccgacctcacaaaggtccatactgagtgttgccacggagatctgctggaatgtgccgacgatagagcagacctcgctaaatatatctgcgagaatcaggattccattagctctaagctgaaagaatgttgcgagaagcccctcctggaaaagagtcattgtatcgccgaggtggaaaacgacgagatgccagcagatctgccatcactcgctgccgactttgtggaatccaaagatgtctgcaagaattacgcagaggctaaagacgtgttcctggggatgtttctgtatgagtacgcccggcgtcaccccgattatagcgtcgtgctcctgctccgactggcaaagacctacgaaacaactctggagaaatgttgcgctgccgcagaccctcatgaatgttatgctaaggtgttcgatgagtttaagccactcgtcgaagagccccagaacctgattaaacagaattgcgaactgttcgagcagctcggtgaatacaagtttcagaacgccctgctcgtgcgttataccaaaaaggtccctcaggtgtctacaccaactctggtggaggtcagtaggaatctgggcaaagtgggatcaaagtgttgcaaacaccccgaggcaaagagaatgccttgtgctgaagattacctctccgtcgtgctgaaccagctctgcgtgctgcatgaaaagaccccagtcagcgaccgggtgacaaaatgttgcaccgaatctctggtcaatcgccgaccctgtttcagtgccctcgaagtggacgaaacttatgtgcctaaggagtttcaggctgaaacattcacctttcacgccgatatctgcactctgtccgagaaagaaaggcagattaagaaacagacagcactggtcgagctcgtgaagcataaaccaaaggctaccaaggagcagctgaaagccgtcatggacgatttcgcagcttttgtggaaaagtgttgcaaagccgacgataaggagacttgtttcgcagaagaggggaaaaagctcgtggctgccagccaggcagctctgggtctggggtctggtggatcagggggaggttcaggcgggggcagtggcgggggatctggaggtggcagtgggggcggttccggaggtggatcaggaggaggaagtggcggcggtagcggtggtggtgctcaagtcttgcgtggtacggtgacagacttcccaggcttcgatgaaagagcggacgcggaaacacttcgaaaggcgatgaaagggctcggtactgacgaagagtccattttgacccttcttacgagcaggtcaaacgctcagaggcaagaaatctctgcagcctttaagacactctttggacgtgaccttcttgatgacctcaaatctgagctgacgggaaagtttgagaaactcatcgtagctttgatgaagcccagccgattgtatgatgcttacgaactgaaacacgccctgaaaggagcgggaacgaacgagaaagttttgactgagatcatcgcatcgcggaccccggaagagctcagagccatcaaacaagtctacgaggaggagtacggatcgtcattggaagatgacgtggtgggggatacgtcgggttactaccaacgaatgcttgtcgtgcttttgcaggcaaatcgcgacccggatgcggggatcgacgaggcccaagtggagcaagatgcgcaagcactcttccaggccggtgaactcaaatgggggaccgatgaagagaagtttatcaccatctttggcacgaggagtgtaagtcatctgcgtaaagtattcgataagtatatgacaatctcagggtttcagattgaggagacaattgacagggaaacctccggtaacttggagcagctcttgcttgccgtcgtcaagtccattcgctcgatccctgcgtatctggctgaaacactgtattacgccatgaaaggggcaggcactgatgaccacaccttgattagagttatggtgtcgcgatcagaaattgacttgttcaatatccggaaagagttccggaagaatttcgcaacgagcctctatagcatgatcaaaggggacacttcgggagattacaagaaagcgttgctccttctttgcggagaggatgactgataa

SEQ ID NO: 95 - DNA, 3057 bp, Artificial Sequence
  Synthetic construct
atgttcccagccatgcccttgtccagcctgtttgttaacggcccaagaacactttgtggagccgaactggtggatgctctccaattcgtttgcggcgaccgcggattctactttaacaagcccaccggttacgggtcttcaagccggagggccccgcagactggcatcgtcgacgagtgctgttttagaagctgcgatctgcgacggttggagatgttgtgtgcacctctgaagcccgcgaaaagtgctggttccggagggagcggtggtgggagtggcggatctggtggaggagacgctcacaagtctgaagtggcacataggttcaaagatctgggcgaagagaactttaaggccctcgtcctgatcgctttcgcacagtacctccagcagtctccctttgaagatcacgtgaaactggtcaatgaggtgaccgaatttgccaagacatgcgtggctgatgagagtgcagaaaactgtgacaaatcactgcatactctctttggagataagctgtgcaccgtcgccacactcagagagacttatggggaaatggctgactgttgcgcaaaacaggagcctgaacggaatgagtgtttcctccagcacaaggatgacaacccaaatctgccccgcctcgtgcgacctgaggtcgatgtgatgtgcaccgcctttcatgacaacgaagagacattcctgaagaaatacctgtatgaaattgctcgtaggcacccatacttttatgcccccgagctcctgttctttgcaaagagatacaaagctgccttcactgaatgttgccaggcagctgataaggccgcatgtctcctgcctaaactggacgagctccgggatgaaggtaaggcttccagcgccaaacagcgcctgaagtgcgcttctctccagaagtttggcgagcgagcattcaaagcctgggctgtggcccgtctcagtcagaggtttccaaaggcagaatttgctgaggtgtcaaaactggtgaccgacctcacaaaggtccatactgagtgttgccacggagatctgctggaatgtgccgacgatagagcagacctcgctaaatatatctgcgagaatcaggattccattagctctaagctgaaagaatgttgcgagaagcccctcctggaaaagagtcattgtatcgccgaggtggaaaacgacgagatgccagcagatctgccatcactcgctgccgactttgtggaatccaaagatgtctgcaagaattacgcagaggctaaagacgtgttcctggggatgtttctgtatgagtacgcccggcgtcaccccgattatagcgtcgtgctcctgctccgactggcaaagacctacgaaacaactctggagaaatgttgcgctgccgcagaccctcatgaatgttatgctaaggtgttcgatgagtttaagccactcgtcgaagagccccagaacctgattaaacagaattgcgaactgttcgagcagctcggtgaatacaagtttcagaacgccctgctcgtgcgttataccaaaaaggtccctcaggtgtctacaccaactctggtggaggtcagtaggaatctgggcaaagtgggatcaaagtgttgcaaacaccccgaggcaaagagaatgccttgtgctgaagattacctctccgtcgtgctgaaccagctctgcgtgctgcatgaaaagaccccagtcagcgaccgggtgacaaaatgttgcaccgaatctctggtcaatcgccgaccctgtttcagtgccctcgaagtggacgaaacttatgtgcctaaggagtttcaggctggaacattcacctttcacgccgatatctgcactctgtccgagaaagaaaggcagattaagaaacagacagcactggtcgagctcgtgaagcataaaccaaaggctaccaaggagcagctgaaagccgccatggacgatttcgcagcttttgtggaaaagtgttgcaaagccgacgataaggagacttgtttcgcagaagaggggaaaaagctcgtggctgccagccaggcagctctgggtctggggtctggcggttcagggggaggaagtggaggctcaggaggtggtgctcaagtcttgcgtggtacggtgacagacttcccaggcttcgatgaaagagcggacgcggaaacacttcgaaaggcgatgaaagggctcggtactgacgaagagtccattttgacccttcttacgagcaggtcaaacgctcagaggcaagaaatctctgcagcctttaagacactctttggagctgaccttcttgatgacctcgcatctgagctgacgggaaagtttgagaaactcatcgtagctttgatgaagcccagccgattgtatgatgcttacgaactgaaacacgccctggctggagcgggaacgaacgagaaagttttgactgagatcatcgcatcgcggaccccggaagagctcagagccatcaaacaagtctacgaggaggagtacggatcgtcattggcaggagacgtggtgggggatacgtcgggttactaccaacgaatgcttgtcgtgcttttgcaggcagctcgcgacccggatgcggggatcgacgaggcccaagtggagcaagatgcgcaagcactcttccaggccggtgaactcaaatgggggaccgatgaagagaagtttatcaccatctttggcacgaggagtgtaagtcatctgcgtaaagtattcgataagtatatgacaatctcagggtttcagattgaggagacaattgacagggaaacctccggtaacttggagcagctcttgcttgccgtcgtcaagtccattcgctcgatccctgcgtatctggctgaaacactgtattacgccatgaaaggggcaggcactgatgaccacaccttgattagagttatggtgtcgcgatcagaaattgacttgttcaatatccggaaagagttccggaagaatttcgcaacgagcctctatagcatgatcaaaggggacacttcgggagattacaagaaagcgttgctccttctttgcggagaggatgactaatga

SEQ ID NO: 96 - DNA, 3009 bp, Artificial Sequence
  Synthetic construct
atgttcccagccatgcccttgtccagcctgtttgttaacggcccaagaacactttgtggagccgaactggtggatgctctccaattcgtttgcggcgaccgcggattctactttaacaagcccaccggttacgggtcttcaagccggagggccccgcagactggcatcgtcgacgagtgctgttttagaagctgcgatctgcgacggttggagatgtattgtgcacctctgaagcccgcgaaaagtgctgggagcggtggtgggagtggcgacgctcacaagtctgaagtggcacataggttcaaagatctgggcgaagagaactttaaggccctcgtcctgatcgctttcgcacagtacctccagcagtctccctttgaagatcacgtgaaactggtcaatgaggtgaccgaatttgccaagacatgcgtggctgatgagagtgcagaaaactgtgacaaatcactgcatactctctttggagataagctgtgcaccgtcgccacactcagagagacttatggggaaatggctgactgttgcgcaaaacaggagcctgaacggaatgagtgtttcctccagcacaaggatgacaacccaaatctgccccgcctcgtgcgacctgaggtcgatgtgatgtgcaccgcctttcatgacaacgaagagacattcctgaagaaatacctgtatgaaattgctcgtaggcacccatacttttatgcccccgagctcctgttctttgcaaagagatacaaagctgccttcactgaatgttgccaggcagctgataaggccgcatgtctcctgcctaaactggacgagctccgggatgaaggtaaggcttccagcgccaaacagcgcctgaagtgcgcttctctccagaagtttggcgagcgagcattcaaagcctgggctgtggcccgtctcagtcagaggtttccaaaggcagaatttgctgaggtgtcaaaactggtgaccgacctcacaaaggtccatactgagtgttgccacggagatctgctggaatgtgccgacgatagagcagacctcgctaaatatatctgcgagaatcaggattccattagctctaagctgaaagaatgttgcgagaagcccctcctggaaaagagtcattgtatcgccgaggtggaaaacgacgagatgccagcagatctgccatcactcgctgccgactttgtggaatccaaagatgtctgcaagaattacgcagaggctaaagacgtgttcctggggatgtttctgtatgagtacgcccggcgtcaccccgattatagcgtcgtgctcctgctccgactggcaaagacctacgaaacaactctggagaaatgttgcgctgccgcagaccctcatgaatgttatgctaaggtgttcgatgagtttaagccactcgtcgaagagccccagaacctgattaaacagaattgcgaactgttcgagcagctcggtgaatacaagtttcagaacgccctgctcgtgcgttataccaaaaaggtccctcaggtgtctacaccaactctggtggaggtcagtaggaatctgggcaaagtgggatcaaagtgttgcaaacaccccgaggcaaagagaatgccttgtgctgaagattacctctccgtcgtgctgaaccagctctgcgtgctgcatgaaaagaccccagtcagcgaccgggtgacaaaatgttgcaccgaatctctggtcaatcgccgaccctgtttcagtgccctcgaagtggacgaaacttatgtgcctaaggagtttcaggctgaaacattcacctttcacgccgatatctgcactctgtccgagaaagaaaggcagattaagaaacagacagcactggtcgagctcgtgaagcataaaccaaaggctaccaaggagcagctgaaagccgtcatggacgatttcgcagcttttgtggaaaagtgttgcaaagccgacgataaggagacttgtttcgcagaagaggggaaaaagctcgtggctgccagccaggcagctctgggtctggggagcggtggtgggagtggcgctcaagtcttgcgtggtacggtgacagacttcccaggcttcgatgaaagagcggacgcggaaacacttcgaaaggcgatgaaagggctcggtactgacgaagagtccattttgacccttcttacgagcaggtcaaacgctcagaggcaagaaatctctgcagcctttaagacactctttggacgtgaccttcttgatgacctcaaatctgagctgacgggaaagtttgagaaactcatcgtagctttgatgaagcccagccgattgtatgatgcttacgaactgaaacacgccctgaaaggagcgggaacgaacgagaaagttttgactgagatcatcgcatcgcggaccccggaagagctcagagccatcaaacaagtctacgaggaggagtacggatcgtcattggaagatgacgtggtgggggatacgtcgggttactaccaacgaatgcttgtcgtgcttttgcaggcaaatcgcgacccggatgcggggatcgacgaggcccaagtggagcaagatgcgcaagcactcttccaggccggtgaactcaaatgggggaccgatgaagagaagtttatcaccatctttggcacgaggagtgtaagtcatctgcgtaaagtattcgataagtatatgacaatctcagggtttcagattgaggagacaattgacagggaaacctccggtaacttggagcagctcttgcttgccgtcgtcaagtccattcgctcgatccctgcgtatctggctgaaacactgtattacgccatgaaaggggcaggcactgatgaccacaccttgattagagttatggtgtcgcgatcagaaattgacttgttcaatatccggaaagagttccggaagaatttcgcaacgagcctctatagcatgatcaaaggggacacttcgggagattacaagaaagcgttgctccttctttgcggagaggatgactgataa

SEQ ID NO: 97 - DNA, 3045 bp, Artificial Sequence
  Syntehtic construct
atgttcccagccatgcccttgtccagcctgtttgttaacggcccaagaacactttgtggagccgaactggtggatgctctccaattcgtttgcggcgaccgcggattctactttaacaagcccaccggttacgggtcttcaagccgggccccgcagactggcatcgtcgacgagtgctgttttagaagctgcgatctgcgacggttggagatgtattgtgcacctctgaagcccgcgggttccggagggagcggtggtgggagtggcggatctggtggaggagacgctcacaagtctgaagtggcacataggttcaaagatctgggcgaagagaactttaaggccctcgtcctgatcgctttcgcacagtacctccagcagtctccctttgaagatcacgtgaaactggtcaatgaggtgaccgaatttgccaagacatgcgtggctgatgagagtgcagaaaactgtgacaaatcactgcatactctctttggagataagctgtgcaccgtcgccacactcagagagacttatggggaaatggctgactgttgcgcaaaacaggagcctgaacggaatgagtgtttcctccagcacaaggatgacaacccaaatctgccccgcctcgtgcgacctgaggtcgatgtgatgtgcaccgcctttcatgacaacgaagagacattcctgaagaaatacctgtatgaaattgctcgtaggcacccatacttttatgcccccgagctcctgttctttgcaaagagatacaaagctgccttcactgaatgttgccaggcagctgataaggccgcatgtctcctgcctaaactggacgagctccgggatgaaggtaaggcttccagcgccaaacagcgcctgaagtgcgcttctctccagaagtttggcgagcgagcattcaaagcctgggctgtggcccgtctcagtcagaggtttccaaaggcagaatttgctgaggtgtcaaaactggtgaccgacctcacaaaggtccatactgagtgttgccacggagatctgctggaatgtgccgacgatagagcagacctcgctaaatatatctgcgagaatcaggattccattagctctaagctgaaagaatgttgcgagaagcccctcctggaaaagagtcattgtatcgccgaggtggaaaacgacgagatgccagcagatctgccatcactcgctgccgactttgtggaatccaaagatgtctgcaagaattacgcagaggctaaagacgtgttcctggggatgtttctgtatgagtacgcccggcgtcaccccgattatagcgtcgtgctcctgctccgactggcaaagacctacgaaacaactctggagaaatgttgcgctgccgcagaccctcatgaatgttatgctaaggtgttcgatgagtttaagccactcgtcgaagagccccagaacctgattaaacagaattgcgaactgttcgagcagctcggtgaatacaagtttcagaacgccctgctcgtgcgttataccaaaaaggtccctcaggtgtctacaccaactctggtggaggtcagtaggaatctgggcaaagtgggatcaaagtgttgcaaacaccccgaggcaaagagaatgccttgtgctgaagattacctctccgtcgtgctgaaccagctctgcgtgctgcatgaaaagaccccagtcagcgaccgggtgacaaaatgttgcaccgaatctctggtcaatcgccgaccctgtttcagtgccctcgaagtggacgaaacttatgtgcctaaggagtttcaggctggaacattcacctttcacgccgatatctgcactctgtccgagaaagaaaggcagattaagaaacagacagcactggtcgagctcgtgaagcataaaccaaaggctaccaaggagcagctgaaagccgccatggacgatttcgcagcttttgtggaaaagtgttgcaaagccgacgataaggagacttgtttcgcagaagaggggaaaaagctcgtggctgccagccaggcagctctgggtctggggtctggcggttcagggggaggaagtggaggctcaggaggtggtgctcaagtcttgcgtggtacggtgacagacttcccaggcttcgatgaaagagcggacgcggaaacacttcgaaaggcgatgaaagggctcggtactgacgaagagtccattttgacccttcttacgagcaggtcaaacgctcagaggcaagaaatctctgcagcctttaagacactctttggagctgaccttcttgatgacctcgcatctgagctgacgggaaagtttgagaaactcatcgtagctttgatgaagcccagccgattgtatgatgcttacgaactgaaacacgccctggctggagcgggaacgaacgagaaagttttgactgagatcatcgcatcgcggaccccggaagagctcagagccatcaaacaagtctacgaggaggagtacggatcgtcattggcaggagacgtggtgggggatacgtcgggttactaccaacgaatgcttgtcgtgcttttgcaggcagctcgcgacccggatgcggggatcgacgaggcccaagtggagcaagatgcgcaagcactcttccaggccggtgaactcaaatgggggaccgatgaagagaagtttatcaccatctttggcacgaggagtgtaagtcatctgcgtaaagtattcgataagtatatgacaatctcagggtttcagattgaggagacaattgacagggaaacctccggtaacttggagcagctcttgcttgccgtcgtcaagtccattcgctcgatccctgcgtatctggctgaaacactgtattacgccatgaaaggggcaggcactgatgaccacaccttgattagagttatggtgtcgcgatcagaaattgacttgttcaatatccggaaagagttccggaagaatttcgcaacgagcctctatagcatgatcaaaggggacacttcgggagattacaagaaagcgttgctccttctttgcggagaggatgactaatga

SEQ ID NO: 98 - DNA, 3057 bp, Artificial Sequence
  Synthetic construct
atgttcccagccatgcccttgtccagcctgtttgttaacggcccaagaacactttgtggagccgaactggtggatgctctccaattcgtttgcggcgaccgcggattcctctttaacaagcccaccggtgccgggtcttcaagccggagggccccgcagactggcatcgtcgacgagtgctgttttagaagctgcgatctgcgacggttggagatgtattgtgcacctctgaagcccgcgaaaagtgctggttccggagggagcggtggtgggagtggcggatctggtggaggagacgctcacaagtctgaagtggcacataggttcaaagatctgggcgaagagaactttaaggccctcgtcctgatcgctttcgcacagtacctccagcagtctccctttgaagatcacgtgaaactggtcaatgaggtgaccgaatttgccaagacatgcgtggctgatgagagtgcagaaaactgtgacaaatcactgcatactctctttggagataagctgtgcaccgtcgccacactcagagagacttatggggaaatggctgactgttgcgcaaaacaggagcctgaacggaatgagtgtttcctccagcacaaggatgacaacccaaatctgccccgcctcgtgcgacctgaggtcgatgtgatgtgcaccgcctttcatgacaacgaagagacattcctgaagaaatacctgtatgaaattgctcgtaggcacccatacttttatgcccccgagctcctgttctttgcaaagagatacaaagctgccttcactgaatgttgccaggcagctgataaggccgcatgtctcctgcctaaactggacgagctccgggatgaaggtaaggcttccagcgccaaacagcgcctgaagtgcgcttctctccagaagtttggcgagcgagcattcaaagcctgggctgtggcccgtctcagtcagaggtttccaaaggcagaatttgctgaggtgtcaaaactggtgaccgacctcacaaaggtccatactgagtgttgccacggagatctgctggaatgtgccgacgatagagcagacctcgctaaatatatctgcgagaatcaggattccattagctctaagctgaaagaatgttgcgagaagcccctcctggaaaagagtcattgtatcgccgaggtggaaaacgacgagatgccagcagatctgccatcactcgctgccgactttgtggaatccaaagatgtctgcaagaattacgcagaggctaaagacgtgttcctggggatgtttctgtatgagtacgcccggcgtcaccccgattatagcgtcgtgctcctgctccgactggcaaagacctacgaaacaactctggagaaatgttgcgctgccgcagaccctcatgaatgttatgctaaggtgttcgatgagtttaagccactcgtcgaagagccccagaacctgattaaacagaattgcgaactgttcgagcagctcggtgaatacaagtttcagaacgccctgctcgtgcgttataccaaaaaggtccctcaggtgtctacaccaactctggtggaggtcagtaggaatctgggcaaagtgggatcaaagtgttgcaaacaccccgaggcaaagagaatgccttgtgctgaagattacctctccgtcgtgctgaaccagctctgcgtgctgcatgaaaagaccccagtcagcgaccgggtgacaaaatgttgcaccgaatctctggtcaatcgccgaccctgtttcagtgccctcgaagtggacgaaacttatgtgcctaaggagtttcaggctggaacattcacctttcacgccgatatctgcactctgtccgagaaagaaaggcagattaagaaacagacagcactggtcgagctcgtgaagcataaaccaaaggctaccaaggagcagctgaaagccgccatggacgatttcgcagcttttgtggaaaagtgttgcaaagccgacgataaggagacttgtttcgcagaagaggggaaaaagctcgtggctgccagccaggcagctctgggtctggggtctggcggttcagggggaggaagtggaggctcaggaggtggtgctcaagtcttgcgtggtacggtgacagacttcccaggcttcgatgaaagagcggacgcggaaacacttcgaaaggcgatgaaagggctcggtactgacgaagagtccattttgacccttcttacgagcaggtcaaacgctcagaggcaagaaatctctgcagcctttaagacactctttggagctgaccttcttgatgacctcgcatctgagctgacgggaaagtttgagaaactcatcgtagctttgatgaagcccagccgattgtatgatgcttacgaactgaaacacgccctggctggagcgggaacgaacgagaaagttttgactgagatcatcgcatcgcggaccccggaagagctcagagccatcaaacaagtctacgaggaggagtacggatcgtcattggcaggagacgtggtgggggatacgtcgggttactaccaacgaatgcttgtcgtgcttttgcaggcagctcgcgacccggatgcggggatcgacgaggcccaagtggagcaagatgcgcaagcactcttccaggccggtgaactcaaatgggggaccgatgaagagaagtttatcaccatctttggcacgaggagtgtaagtcatctgcgtaaagtattcgataagtatatgacaatctcagggtttcagattgaggagacaattgacagggaaacctccggtaacttggagcagctcttgcttgccgtcgtcaagtccattcgctcgatccctgcgtatctggctgaaacactgtattacgccatgaaaggggcaggcactgatgaccacaccttgattagagttatggtgtcgcgatcagaaattgacttgttcaatatccggaaagagttccggaagaatttcgcaacgagcctctatagcatgatcaaaggggacacttcgggagattacaagaaagcgttgctccttctttgcggagaggatgactaatga

SEQ ID NO: 99 - DNA, 3057 bp, Artificial Sequence
  Synthetic construct
atgttcccagccatgcccttgtccagcctgtttgttaacggcccaagaacactttgtggagccgaactggtggatgctctccaattcgtttgcggcgaccgcggattcctctttaacaagcccaccggttacgggtcttcaagccggagggccccgcagactggcatcgtcgacgagtgctgttttagaagctgcgatctgcgacggttggagatgtattgtgcacctctgaagcccgcgaaaagtgctggttccggagggagcggtggtgggagtggcggatctggtggaggagacgctcacaagtctgaagtggcacataggttcaaagatctgggcgaagagaactttaaggccctcgtcctgatcgctttcgcacagtacctccagcagtctccctttgaagatcacgtgaaactggtcaatgaggtgaccgaatttgccaagacatgcgtggctgatgagagtgcagaaaactgtgacaaatcactgcatactctctttggagataagctgtgcaccgtcgccacactcagagagacttatggggaaatggctgactgttgcgcaaaacaggagcctgaacggaatgagtgtttcctccagcacaaggatgacaacccaaatctgccccgcctcgtgcgacctgaggtcgatgtgatgtgcaccgcctttcatgacaacgaagagacattcctgaagaaatacctgtatgaaattgctcgtaggcacccatacttttatgcccccgagctcctgttctttgcaaagagatacaaagctgccttcactgaatgttgccaggcagctgataaggccgcatgtctcctgcctaaactggacgagctccgggatgaaggtaaggcttccagcgccaaacagcgcctgaagtgcgcttctctccagaagtttggcgagcgagcattcaaagcctgggctgtggcccgtctcagtcagaggtttccaaaggcagaatttgctgaggtgtcaaaactggtgaccgacctcacaaaggtccatactgagtgttgccacggagatctgctggaatgtgccgacgatagagcagacctcgctaaatatatctgcgagaatcaggattccattagctctaagctgaaagaatgttgcgagaagcccctcctggaaaagagtcattgtatcgccgaggtggaaaacgacgagatgccagcagatctgccatcactcgctgccgactttgtggaatccaaagatgtctgcaagaattacgcagaggctaaagacgtgttcctggggatgtttctgtatgagtacgcccggcgtcaccccgattatagcgtcgtgctcctgctccgactggcaaagacctacgaaacaactctggagaaatgttgcgctgccgcagaccctcatgaatgttatgctaaggtgttcgatgagtttaagccactcgtcgaagagccccagaacctgattaaacagaattgcgaactgttcgagcagctcggtgaatacaagtttcagaacgccctgctcgtgcgttataccaaaaaggtccctcaggtgtctacaccaactctggtggaggtcagtaggaatctgggcaaagtgggatcaaagtgttgcaaacaccccgaggcaaagagaatgccttgtgctgaagattacctctccgtcgtgctgaaccagctctgcgtgctgcatgaaaagaccccagtcagcgaccgggtgacaaaatgttgcaccgaatctctggtcaatcgccgaccctgtttcagtgccctcgaagtggacgaaacttatgtgcctaaggagtttcaggctggaacattcacctttcacgccgatatctgcactctgtccgagaaagaaaggcagattaagaaacagacagcactggtcgagctcgtgaagcataaaccaaaggctaccaaggagcagctgaaagccgccatggacgatttcgcagcttttgtggaaaagtgttgcaaagccgacgataaggagacttgtttcgcagaagaggggaaaaagctcgtggctgccagccaggcagctctgggtctggggtctggcggttcagggggaggaagtggaggctcaggaggtggtgctcaagtcttgcgtggtacggtgacagacttcccaggcttcgatgaaagagcggacgcggaaacacttcgaaaggcgatgaaagggctcggtactgacgaagagtccattttgacccttcttacgagcaggtcaaacgctcagaggcaagaaatctctgcagcctttaagacactctttggagctgaccttcttgatgacctcgcatctgagctgacgggaaagtttgagaaactcatcgtagctttgatgaagcccagccgattgtatgatgcttacgaactgaaacacgccctggctggagcgggaacgaacgagaaagttttgactgagatcatcgcatcgcggaccccggaagagctcagagccatcaaacaagtctacgaggaggagtacggatcgtcattggcaggagacgtggtgggggatacgtcgggttactaccaacgaatgcttgtcgtgcttttgcaggcagctcgcgacccggatgcggggatcgacgaggcccaagtggagcaagatgcgcaagcactcttccaggccggtgaactcaaatgggggaccgatgaagagaagtttatcaccatctttggcacgaggagtgtaagtcatctgcgtaaagtattcgataagtatatgacaatctcagggtttcagattgaggagacaattgacagggaaacctccggtaacttggagcagctcttgcttgccgtcgtcaagtccattcgctcgatccctgcgtatctggctgaaacactgtattacgccatgaaaggggcaggcactgatgaccacaccttgattagagttatggtgtcgcgatcagaaattgacttgttcaatatccggaaagagttccggaagaatttcgcaacgagcctctatagcatgatcaaaggggacacttcgggagattacaagaaagcgttgctccttctttgcggagaggatgactaatga

SEQ ID NO: 100 - DNA, 3057 bp, Artificial Sequence
  Synthetic construct
atgttcccagccatgcccttgtccagcctgtttgttaacggcccaagaacactttgtggagccgaactggtggatgctctccaattcgtttgcggcgaccgcggattctactttaacaagcccaccggtgccgggtcttcaagccggagggccccgcagactggcatcgtcgacgagtgctgttttagaagctgcgatctgcgacggttggagatgtattgtgcacctctgaagcccgcgaaaagtgctggttccggagggagcggtggtgggagtggcggatctggtggaggagacgctcacaagtctgaagtggcacataggttcaaagatctgggcgaagagaactttaaggccctcgtcctgatcgctttcgcacagtacctccagcagtctccctttgaagatcacgtgaaactggtcaatgaggtgaccgaatttgccaagacatgcgtggctgatgagagtgcagaaaactgtgacaaatcactgcatactctctttggagataagctgtgcaccgtcgccacactcagagagacttatggggaaatggctgactgttgcgcaaaacaggagcctgaacggaatgagtgtttcctccagcacaaggatgacaacccaaatctgccccgcctcgtgcgacctgaggtcgatgtgatgtgcaccgcctttcatgacaacgaagagacattcctgaagaaatacctgtatgaaattgctcgtaggcacccatacttttatgcccccgagctcctgttctttgcaaagagatacaaagctgccttcactgaatgttgccaggcagctgataaggccgcatgtctcctgcctaaactggacgagctccgggatgaaggtaaggcttccagcgccaaacagcgcctgaagtgcgcttctctccagaagtttggcgagcgagcattcaaagcctgggctgtggcccgtctcagtcagaggtttccaaaggcagaatttgctgaggtgtcaaaactggtgaccgacctcacaaaggtccatactgagtgttgccacggagatctgctggaatgtgccgacgatagagcagacctcgctaaatatatctgcgagaatcaggattccattagctctaagctgaaagaatgttgcgagaagcccctcctggaaaagagtcattgtatcgccgaggtggaaaacgacgagatgccagcagatctgccatcactcgctgccgactttgtggaatccaaagatgtctgcaagaattacgcagaggctaaagacgtgttcctggggatgtttctgtatgagtacgcccggcgtcaccccgattatagcgtcgtgctcctgctccgactggcaaagacctacgaaacaactctggagaaatgttgcgctgccgcagaccctcatgaatgttatgctaaggtgttcgatgagtttaagccactcgtcgaagagccccagaacctgattaaacagaattgcgaactgttcgagcagctcggtgaatacaagtttcagaacgccctgctcgtgcgttataccaaaaaggtccctcaggtgtctacaccaactctggtggaggtcagtaggaatctgggcaaagtgggatcaaagtgttgcaaacaccccgaggcaaagagaatgccttgtgctgaagattacctctccgtcgtgctgaaccagctctgcgtgctgcatgaaaagaccccagtcagcgaccgggtgacaaaatgttgcaccgaatctctggtcaatcgccgaccctgtttcagtgccctcgaagtggacgaaacttatgtgcctaaggagtttcaggctggaacattcacctttcacgccgatatctgcactctgtccgagaaagaaaggcagattaagaaacagacagcactggtcgagctcgtgaagcataaaccaaaggctaccaaggagcagctgaaagccgccatggacgatttcgcagcttttgtggaaaagtgttgcaaagccgacgataaggagacttgtttcgcagaagaggggaaaaagctcgtggctgccagccaggcagctctgggtctggggtctggcggttcagggggaggaagtggaggctcaggaggtggtgctcaagtcttgcgtggtacggtgacagacttcccaggcttcgatgaaagagcggacgcggaaacacttcgaaaggcgatgaaagggctcggtactgacgaagagtccattttgacccttcttacgagcaggtcaaacgctcagaggcaagaaatctctgcagcctttaagacactctttggagctgaccttcttgatgacctcgcatctgagctgacgggaaagtttgagaaactcatcgtagctttgatgaagcccagccgattgtatgatgcttacgaactgaaacacgccctggctggagcgggaacgaacgagaaagttttgactgagatcatcgcatcgcggaccccggaagagctcagagccatcaaacaagtctacgaggaggagtacggatcgtcattggcaggagacgtggtgggggatacgtcgggttactaccaacgaatgcttgtcgtgcttttgcaggcagctcgcgacccggatgcggggatcgacgaggcccaagtggagcaagatgcgcaagcactcttccaggccggtgaactcaaatgggggaccgatgaagagaagtttatcaccatctttggcacgaggagtgtaagtcatctgcgtaaagtattcgataagtatatgacaatctcagggtttcagattgaggagacaattgacagggaaacctccggtaacttggagcagctcttgcttgccgtcgtcaagtccattcgctcgatccctgcgtatctggctgaaacactgtattacgccatgaaaggggcaggcactgatgaccacaccttgattagagttatggtgtcgcgatcagaaattgacttgttcaatatccggaaagagttccggaagaatttcgcaacgagcctctatagcatgatcaaaggggacacttcgggagattacaagaaagcgttgctccttctttgcggagaggatgactaatga

SEQ ID NO: 101 - DNA, 3009 bp, Artificial Sequence
  Synthetic construct
atgttcccagccatgcccttgtccagcctgtttgttaacggcccaagaacactttgtggagccgaactggtggatgctctccaattcgtttgcggcgaccgcggattcctctttaacaagcccaccggttacgggtcttcaagccggagggccccgcagactggcatcgtcgacgagtgctgttttagaagctgcgatctgcgacggttggagatgtattgtgcacctctgaagcccgcgaaaagtgctgggagcggtggtgggagtggcgacgctcacaagtctgaagtggcacataggttcaaagatctgggcgaagagaactttaaggccctcgtcctgatcgctttcgcacagtacctccagcagtctccctttgaagatcacgtgaaactggtcaatgaggtgaccgaatttgccaagacatgcgtggctgatgagagtgcagaaaactgtgacaaatcactgcatactctctttggagataagctgtgcaccgtcgccacactcagagagacttatggggaaatggctgactgttgcgcaaaacaggagcctgaacggaatgagtgtttcctccagcacaaggatgacaacccaaatctgccccgcctcgtgcgacctgaggtcgatgtgatgtgcaccgcctttcatgacaacgaagagacattcctgaagaaatacctgtatgaaattgctcgtaggcacccatacttttatgcccccgagctcctgttctttgcaaagagatacaaagctgccttcactgaatgttgccaggcagctgataaggccgcatgtctcctgcctaaactggacgagctccgggatgaaggtaaggcttccagcgccaaacagcgcctgaagtgcgcttctctccagaagtttggcgagcgagcattcaaagcctgggctgtggcccgtctcagtcagaggtttccaaaggcagaatttgctgaggtgtcaaaactggtgaccgacctcacaaaggtccatactgagtgttgccacggagatctgctggaatgtgccgacgatagagcagacctcgctaaatatatctgcgagaatcaggattccattagctctaagctgaaagaatgttgcgagaagcccctcctggaaaagagtcattgtatcgccgaggtggaaaacgacgagatgccagcagatctgccatcactcgctgccgactttgtggaatccaaagatgtctgcaagaattacgcagaggctaaagacgtgttcctggggatgtttctgtatgagtacgcccggcgtcaccccgattatagcgtcgtgctcctgctccgactggcaaagacctacgaaacaactctggagaaatgttgcgctgccgcagaccctcatgaatgttatgctaaggtgttcgatgagtttaagccactcgtcgaagagccccagaacctgattaaacagaattgcgaactgttcgagcagctcggtgaatacaagtttcagaacgccctgctcgtgcgttataccaaaaaggtccctcaggtgtctacaccaactctggtggaggtcagtaggaatctgggcaaagtgggatcaaagtgttgcaaacaccccgaggcaaagagaatgccttgtgctgaagattacctctccgtcgtgctgaaccagctctgcgtgctgcatgaaaagaccccagtcagcgaccgggtgacaaaatgttgcaccgaatctctggtcaatcgccgaccctgtttcagtgccctcgaagtggacgaaacttatgtgcctaaggagtttcaggctgaaacattcacctttcacgccgatatctgcactctgtccgagaaagaaaggcagattaagaaacagacagcactggtcgagctcgtgaagcataaaccaaaggctaccaaggagcagctgaaagccgtcatggacgatttcgcagcttttgtggaaaagtgttgcaaagccgacgataaggagacttgtttcgcagaagaggggaaaaagctcgtggctgccagccaggcagctctgggtctggggagcggtggtgggagtggcgctcaagtcttgcgtggtacggtgacagacttcccaggcttcgatgaaagagcggacgcggaaacacttcgaaaggcgatgaaagggctcggtactgacgaagagtccattttgacccttcttacgagcaggtcaaacgctcagaggcaagaaatctctgcagcctttaagacactctttggagctgaccttcttgatgacctcgcatctgagctgacgggaaagtttgagaaactcatcgtagctttgatgaagcccagccgattgtatgatgcttacgaactgaaacacgccctggctggagcgggaacgaacgagaaagttttgactgagatcatcgcatcgcggaccccggaagagctcagagccatcaaacaagtctacgaggaggagtacggatcgtcattggcaggagacgtggtgggggatacgtcgggttactaccaacgaatgcttgtcgtgcttttgcaggcagctcgcgacccggatgcggggatcgacgaggcccaagtggagcaagatgcgcaagcactcttccaggccggtgaactcaaatgggggaccgatgaagagaagtttatcaccatctttggcacgaggagtgtaagtcatctgcgtaaagtattcgataagtatatgacaatctcagggtttcagattgaggagacaattgacagggaaacctccggtaacttggagcagctcttgcttgccgtcgtcaagtccattcgctcgatccctgcgtatctggctgaaacactgtattacgccatgaaaggggcaggcactgatgaccacaccttgattagagttatggtgtcgcgatcagaaattgacttgttcaatatccggaaagagttccggaagaatttcgcaacgagcctctatagcatgatcaaaggggacacttcgggagattacaagaaagcgttgctccttctttgcggagaggatgactgataa

SEQ ID NO: 102 - DNA, 3009 bp, Artificial Sequence
  Synthetic construct
atgttcccagccatgcccttgtccagcctgtttgttaacggcccaagaacactttgtggagccgaactggtggatgctctccaattcgtttgcggcgaccgcggattctactttaacaagcccaccggtgccgggtcttcaagccggagggccccgcagactggcatcgtcgacgagtgctgttttagaagctgcgatctgcgacggttggagatgtattgtgcacctctgaagcccgcgaaaagtgctgggagcggtggtgggagtggcgacgctcacaagtctgaagtggcacataggttcaaagatctgggcgaagagaactttaaggccctcgtcctgatcgctttcgcacagtacctccagcagtctccctttgaagatcacgtgaaactggtcaatgaggtgaccgaatttgccaagacatgcgtggctgatgagagtgcagaaaactgtgacaaatcactgcatactctctttggagataagctgtgcaccgtcgccacactcagagagacttatggggaaatggctgactgttgcgcaaaacaggagcctgaacggaatgagtgtttcctccagcacaaggatgacaacccaaatctgccccgcctcgtgcgacctgaggtcgatgtgatgtgcaccgcctttcatgacaacgaagagacattcctgaagaaatacctgtatgaaattgctcgtaggcacccatacttttatgcccccgagctcctgttctttgcaaagagatacaaagctgccttcactgaatgttgccaggcagctgataaggccgcatgtctcctgcctaaactggacgagctccgggatgaaggtaaggcttccagcgccaaacagcgcctgaagtgcgcttctctccagaagtttggcgagcgagcattcaaagcctgggctgtggcccgtctcagtcagaggtttccaaaggcagaatttgctgaggtgtcaaaactggtgaccgacctcacaaaggtccatactgagtgttgccacggagatctgctggaatgtgccgacgatagagcagacctcgctaaatatatctgcgagaatcaggattccattagctctaagctgaaagaatgttgcgagaagcccctcctggaaaagagtcattgtatcgccgaggtggaaaacgacgagatgccagcagatctgccatcactcgctgccgactttgtggaatccaaagatgtctgcaagaattacgcagaggctaaagacgtgttcctggggatgtttctgtatgagtacgcccggcgtcaccccgattatagcgtcgtgctcctgctccgactggcaaagacctacgaaacaactctggagaaatgttgcgctgccgcagaccctcatgaatgttatgctaaggtgttcgatgagtttaagccactcgtcgaagagccccagaacctgattaaacagaattgcgaactgttcgagcagctcggtgaatacaagtttcagaacgccctgctcgtgcgttataccaaaaaggtccctcaggtgtctacaccaactctggtggaggtcagtaggaatctgggcaaagtgggatcaaagtgttgcaaacaccccgaggcaaagagaatgccttgtgctgaagattacctctccgtcgtgctgaaccagctctgcgtgctgcatgaaaagaccccagtcagcgaccgggtgacaaaatgttgcaccgaatctctggtcaatcgccgaccctgtttcagtgccctcgaagtggacgaaacttatgtgcctaaggagtttcaggctgaaacattcacctttcacgccgatatctgcactctgtccgagaaagaaaggcagattaagaaacagacagcactggtcgagctcgtgaagcataaaccaaaggctaccaaggagcagctgaaagccgtcatggacgatttcgcagcttttgtggaaaagtgttgcaaagccgacgataaggagacttgtttcgcagaagaggggaaaaagctcgtggctgccagccaggcagctctgggtctggggagcggtggtgggagtggcgctcaagtcttgcgtggtacggtgacagacttcccaggcttcgatgaaagagcggacgcggaaacacttcgaaaggcgatgaaagggctcggtactgacgaagagtccattttgacccttcttacgagcaggtcaaacgctcagaggcaagaaatctctgcagcctttaagacactctttggagctgaccttcttgatgacctcgcatctgagctgacgggaaagtttgagaaactcatcgtagctttgatgaagcccagccgattgtatgatgcttacgaactgaaacacgccctggctggagcgggaacgaacgagaaagttttgactgagatcatcgcatcgcggaccccggaagagctcagagccatcaaacaagtctacgaggaggagtacggatcgtcattggcaggagacgtggtgggggatacgtcgggttactaccaacgaatgcttgtcgtgcttttgcaggcagctcgcgacccggatgcggggatcgacgaggcccaagtggagcaagatgcgcaagcactcttccaggccggtgaactcaaatgggggaccgatgaagagaagtttatcaccatctttggcacgaggagtgtaagtcatctgcgtaaagtattcgataagtatatgacaatctcagggtttcagattgaggagacaattgacagggaaacctccggtaacttggagcagctcttgcttgccgtcgtcaagtccattcgctcgatccctgcgtatctggctgaaacactgtattacgccatgaaaggggcaggcactgatgaccacaccttgattagagttatggtgtcgcgatcagaaattgacttgttcaatatccggaaagagttccggaagaatttcgcaacgagcctctatagcatgatcaaaggggacacttcgggagattacaagaaagcgttgctccttctttgcggagaggatgactgataa

SEQ ID NO: 103 - DNA, 3009 bp, Artificial Sequence
  Synthetic construct
atgttcccagccatgcccttgtccagcctgtttgttaacggcccaagaacactttgtggagccgaactggtggatgctctccaattcgtttgcggcgaccgcggattctactttaacaagcccaccggttacgggtcttcaagccggagggccccgcagactggcatcgtcgacgagtgctgttttagaagctgcgatctgcgacggttggagatgttgtgtgcacctctgaagcccgcgaaaagtgctgggagcggtggtgggagtggcgacgctcacaagtctgaagtggcacataggttcaaagatctgggcgaagagaactttaaggccctcgtcctgatcgctttcgcacagtacctccagcagtctccctttgaagatcacgtgaaactggtcaatgaggtgaccgaatttgccaagacatgcgtggctgatgagagtgcagaaaactgtgacaaatcactgcatactctctttggagataagctgtgcaccgtcgccacactcagagagacttatggggaaatggctgactgttgcgcaaaacaggagcctgaacggaatgagtgtttcctccagcacaaggatgacaacccaaatctgccccgcctcgtgcgacctgaggtcgatgtgatgtgcaccgcctttcatgacaacgaagagacattcctgaagaaatacctgtatgaaattgctcgtaggcacccatacttttatgcccccgagctcctgttctttgcaaagagatacaaagctgccttcactgaatgttgccaggcagctgataaggccgcatgtctcctgcctaaactggacgagctccgggatgaaggtaaggcttccagcgccaaacagcgcctgaagtgcgcttctctccagaagtttggcgagcgagcattcaaagcctgggctgtggcccgtctcagtcagaggtttccaaaggcagaatttgctgaggtgtcaaaactggtgaccgacctcacaaaggtccatactgagtgttgccacggagatctgctggaatgtgccgacgatagagcagacctcgctaaatatatctgcgagaatcaggattccattagctctaagctgaaagaatgttgcgagaagcccctcctggaaaagagtcattgtatcgccgaggtggaaaacgacgagatgccagcagatctgccatcactcgctgccgactttgtggaatccaaagatgtctgcaagaattacgcagaggctaaagacgtgttcctggggatgtttctgtatgagtacgcccggcgtcaccccgattatagcgtcgtgctcctgctccgactggcaaagacctacgaaacaactctggagaaatgttgcgctgccgcagaccctcatgaatgttatgctaaggtgttcgatgagtttaagccactcgtcgaagagccccagaacctgattaaacagaattgcgaactgttcgagcagctcggtgaatacaagtttcagaacgccctgctcgtgcgttataccaaaaaggtccctcaggtgtctacaccaactctggtggaggtcagtaggaatctgggcaaagtgggatcaaagtgttgcaaacaccccgaggcaaagagaatgccttgtgctgaagattacctctccgtcgtgctgaaccagctctgcgtgctgcatgaaaagaccccagtcagcgaccgggtgacaaaatgttgcaccgaatctctggtcaatcgccgaccctgtttcagtgccctcgaagtggacgaaacttatgtgcctaaggagtttcaggctgaaacattcacctttcacgccgatatctgcactctgtccgagaaagaaaggcagattaagaaacagacagcactggtcgagctcgtgaagcataaaccaaaggctaccaaggagcagctgaaagccgtcatggacgatttcgcagcttttgtggaaaagtgttgcaaagccgacgataaggagacttgtttcgcagaagaggggaaaaagctcgtggctgccagccaggcagctctgggtctggggagcggtggtgggagtggcgctcaagtcttgcgtggtacggtgacagacttcccaggcttcgatgaaagagcggacgcggaaacacttcgaaaggcgatgaaagggctcggtactgacgaagagtccattttgacccttcttacgagcaggtcaaacgctcagaggcaagaaatctctgcagcctttaagacactctttggagctgaccttcttgatgacctcgcatctgagctgacgggaaagtttgagaaactcatcgtagctttgatgaagcccagccgattgtatgatgcttacgaactgaaacacgccctggctggagcgggaacgaacgagaaagttttgactgagatcatcgcatcgcggaccccggaagagctcagagccatcaaacaagtctacgaggaggagtacggatcgtcattggcaggagacgtggtgggggatacgtcgggttactaccaacgaatgcttgtcgtgcttttgcaggcagctcgcgacccggatgcggggatcgacgaggcccaagtggagcaagatgcgcaagcactcttccaggccggtgaactcaaatgggggaccgatgaagagaagtttatcaccatctttggcacgaggagtgtaagtcatctgcgtaaagtattcgataagtatatgacaatctcagggtttcagattgaggagacaattgacagggaaacctccggtaacttggagcagctcttgcttgccgtcgtcaagtccattcgctcgatccctgcgtatctggctgaaacactgtattacgccatgaaaggggcaggcactgatgaccacaccttgattagagttatggtgtcgcgatcagaaattgacttgttcaatatccggaaagagttccggaagaatttcgcaacgagcctctatagcatgatcaaaggggacacttcgggagattacaagaaagcgttgctccttctttgcggagaggatgactgataa

SEQ ID NO: 104 - DNA, 2997 bp, Artificial Sequence
  Synthetic construct
atgttcccagccatgcccttgtccagcctgtttgttaacggcccaagaacactttgtggagccgaactggtggatgctctccaattcgtttgcggcgaccgcggattctactttaacaagcccaccggttacgggtcttcaagccgggccccgcagactggcatcgtcgacgagtgctgttttagaagctgcgatctgcgacggttggagatgtattgtgcacctctgaagcccgcggggagcggtggtgggagtggcgacgctcacaagtctgaagtggcacataggttcaaagatctgggcgaagagaactttaaggccctcgtcctgatcgctttcgcacagtacctccagcagtctccctttgaagatcacgtgaaactggtcaatgaggtgaccgaatttgccaagacatgcgtggctgatgagagtgcagaaaactgtgacaaatcactgcatactctctttggagataagctgtgcaccgtcgccacactcagagagacttatggggaaatggctgactgttgcgcaaaacaggagcctgaacggaatgagtgtttcctccagcacaaggatgacaacccaaatctgccccgcctcgtgcgacctgaggtcgatgtgatgtgcaccgcctttcatgacaacgaagagacattcctgaagaaatacctgtatgaaattgctcgtaggcacccatacttttatgcccccgagctcctgttctttgcaaagagatacaaagctgccttcactgaatgttgccaggcagctgataaggccgcatgtctcctgcctaaactggacgagctccgggatgaaggtaaggcttccagcgccaaacagcgcctgaagtgcgcttctctccagaagtttggcgagcgagcattcaaagcctgggctgtggcccgtctcagtcagaggtttccaaaggcagaatttgctgaggtgtcaaaactggtgaccgacctcacaaaggtccatactgagtgttgccacggagatctgctggaatgtgccgacgatagagcagacctcgctaaatatatctgcgagaatcaggattccattagctctaagctgaaagaatgttgcgagaagcccctcctggaaaagagtcattgtatcgccgaggtggaaaacgacgagatgccagcagatctgccatcactcgctgccgactttgtggaatccaaagatgtctgcaagaattacgcagaggctaaagacgtgttcctggggatgtttctgtatgagtacgcccggcgtcaccccgattatagcgtcgtgctcctgctccgactggcaaagacctacgaaacaactctggagaaatgttgcgctgccgcagaccctcatgaatgttatgctaaggtgttcgatgagtttaagccactcgtcgaagagccccagaacctgattaaacagaattgcgaactgttcgagcagctcggtgaatacaagtttcagaacgccctgctcgtgcgttataccaaaaaggtccctcaggtgtctacaccaactctggtggaggtcagtaggaatctgggcaaagtgggatcaaagtgttgcaaacaccccgaggcaaagagaatgccttgtgctgaagattacctctccgtcgtgctgaaccagctctgcgtgctgcatgaaaagaccccagtcagcgaccgggtgacaaaatgttgcaccgaatctctggtcaatcgccgaccctgtttcagtgccctcgaagtggacgaaacttatgtgcctaaggagtttcaggctgaaacattcacctttcacgccgatatctgcactctgtccgagaaagaaaggcagattaagaaacagacagcactggtcgagctcgtgaagcataaaccaaaggctaccaaggagcagctgaaagccgtcatggacgatttcgcagcttttgtggaaaagtgttgcaaagccgacgataaggagacttgtttcgcagaagaggggaaaaagctcgtggctgccagccaggcagctctgggtctggggagcggtggtgggagtggcgctcaagtcttgcgtggtacggtgacagacttcccaggcttcgatgaaagagcggacgcggaaacacttcgaaaggcgatgaaagggctcggtactgacgaagagtccattttgacccttcttacgagcaggtcaaacgctcagaggcaagaaatctctgcagcctttaagacactctttggagctgaccttcttgatgacctcgcatctgagctgacgggaaagtttgagaaactcatcgtagctttgatgaagcccagccgattgtatgatgcttacgaactgaaacacgccctggctggagcgggaacgaacgagaaagttttgactgagatcatcgcatcgcggaccccggaagagctcagagccatcaaacaagtctacgaggaggagtacggatcgtcattggcaggagacgtggtgggggatacgtcgggttactaccaacgaatgcttgtcgtgcttttgcaggcagctcgcgacccggatgcggggatcgacgaggcccaagtggagcaagatgcgcaagcactcttccaggccggtgaactcaaatgggggaccgatgaagagaagtttatcaccatctttggcacgaggagtgtaagtcatctgcgtaaagtattcgataagtatatgacaatctcagggtttcagattgaggagacaattgacagggaaacctccggtaacttggagcagctcttgcttgccgtcgtcaagtccattcgctcgatccctgcgtatctggctgaaacactgtattacgccatgaaaggggcaggcactgatgaccacaccttgattagagttatggtgtcgcgatcagaaattgacttgttcaatatccggaaagagttccggaagaatttcgcaacgagcctctatagcatgatcaaaggggacacttcgggagattacaagaaagcgttgctccttctttgcggagaggatgactgataa

SEQ ID NO: 105 - protein, 21 aa, Artificial Sequence
  Synthetic construct
MAWRLWWLLLLLLLLWPMVWA

SEQ ID NO: 106 - DNA, 63 bp, Artificial Sequence
  Synthetic construct
atggcctggcggctgtggtggctgctgctcctgctcctgttgctttggcctatggtgtgggcc

SEQ ID NO: 107 - protein, 683 aa, Artificial Sequence
  Synthetic construct
MFPAMPLSSLFVNGPRTLCGAELVDALQFVCGDRGFYFNKPTGYGSSSRRAPQTGIVDECCFRSCDLRRLEMYCAPLKPAKSAGSGGSGGGSGGSGGGDAHKSEVAHRFKDLGEENFKALVLIAFAQYLQQSPFEDHVKLVNEVTEFAKTCVADESAENCDKSLHTLFGDKLCTVATLRETYGEMADCCAKQEPERNECFLQHKDDNPNLPRLVRPEVDVMCTAFHDNEETFLKKYLYEIARRHPYFYAPELLFFAKRYKAAFTECCQAADKAACLLPKLDELRDEGKASSAKQRLKCASLQKFGERAFKAWAVARLSQRFPKAEFAEVSKLVTDLTKVHTECCHGDLLECADDRADLAKYICENQDSISSKLKECCEKPLLEKSHCIAEVENDEMPADLPSLAADFVESKDVCKNYAEAKDVFLGMFLYEYARRHPDYSVVLLLRLAKTYETTLEKCCAAADPHECYAKVFDEFKPLVEEPQNLIKQNCELFEQLGEYKFQNALLVRYTKKVPQVSTPTLVEVSRNLGKVGSKCCKHPEAKRMPCAEDYLSVVLNQLCVLHEKTPVSDRVTKCCTESLVNRRPCFSALEVDETYVPKEFQAGTFTFHADICTLSEKERQIKKQTALVELVKHKPKATKEQLKAAMDDFAAFVEKCCKADDKETCFAEEGKKLVAASQAALGL

SEQ ID NO: 108 - protein, 1001 aa, Artificial Sequence
  Synthetic construct
MFPAMPLSSLFVNGPRTLCGAELVDALQFVCGDRGFLFNKPTGAGSSSRRAPQTGIVDECCFRSCDLRRLEMYCAPLKPAKSAGSGGGSGDAHKSEVAHRFKDLGEENFKALVLIAFAQYLQQSPFEDHVKLVNEVTEFAKTCVADESAENCDKSLHTLFGDKLCTVATLRETYGEMADCCAKQEPERNECFLQHKDDNPNLPRLVRPEVDVMCTAFHDNEETFLKKYLYEIARRHPYFYAPELLFFAKRYKAAFTECCQAADKAACLLPKLDELRDEGKASSAKQRLKCASLQKFGERAFKAWAVARLSQRFPKAEFAEVSKLVTDLTKVHTECCHGDLLECADDRADLAKYICENQDSISSKLKECCEKPLLEKSHCIAEVENDEMPADLPSLAADFVESKDVCKNYAEAKDVFLGMFLYEYARRHPDYSVVLLLRLAKTYETTLEKCCAAADPHECYAKVFDEFKPLVEEPQNLIKQNCELFEQLGEYKFQNALLVRYTKKVPQVSTPTLVEVSRNLGKVGSKCCKHPEAKRMPCAEDYLSVVLNQLCVLHEKTPVSDRVTKCCTESLVNRRPCFSALEVDETYVPKEFQAGTFTFHADICTLSEKERQIKKQTALVELVKHKPKATKEQLKAAMDDFAAFVEKCCKADDKETCFAEEGKKLVAASQAALGLGSGGGSGAQVLRGTVTDFPGFDERADAETLRKAMKGLGTDEESILTLLTSRSNAQRQEISAAFKTLFGADLLDDLASELTGKFEKLIVALMKPSRLYDAYELKHALAGAGTNEKVLTEIIASRTPEELRAIKQVYEEEYGSSLAGDVVGDTSGYYQRMLVVLLQAARDPDAGIDEAQVEQDAQALFQAGELKWGTDEEKFITIFGTRSVSHLRKVFDKYMTISGFQIEETIDRETSGNLEQLLLAVVKSIRSIPAYLAETLYYAMKGAGTDDHTLIRVMVSRSEIDLFNIRKEFRKNFATSLYSMIKGDTSGDYKKALLLLCGEDD

SEQ ID NO: 109 - protein, 675 aa, Artificial Sequence
  Synthetic construct
MFPAMPLSSLFVNGPRTLCGAELVDALQFVCGDRGFYFNKPTGAGSSSRRAPQTGIVDECCFRSCDLRRLEMYCAPLKPAKSAGSGGGSGDAHKSEVAHRFKDLGEENFKALVLIAFAQYLQQSPFEDHVKLVNEVTEFAKTCVADESAENCDKSLHTLFGDKLCTVATLRETYGEMADCCAKQEPERNECFLQHKDDNPNLPRLVRPEVDVMCTAFHDNEETFLKKYLYEIARRHPYFYAPELLFFAKRYKAAFTECCQAADKAACLLPKLDELRDEGKASSAKQRLKCASLQKFGERAFKAWAVARLSQRFPKAEFAEVSKLVTDLTKVHTECCHGDLLECADDRADLAKYICENQDSISSKLKECCEKPLLEKSHCIAEVENDEMPADLPSLAADFVESKDVCKNYAEAKDVFLGMFLYEYARRHPDYSVVLLLRLAKTYETTLEKCCAAADPHECYAKVFDEFKPLVEEPQNLIKQNCELFEQLGEYKFQNALLVRYTKKVPQVSTPTLVEVSRNLGKVGSKCCKHPEAKRMPCAEDYLSVVLNQLCVLHEKTPVSDRVTKCCTESLVNRRPCFSALEVDETYVPKEFQAETFTFHADICTLSEKERQIKKQTALVELVKHKPKATKEQLKAVMDDFAAFVEKCCKADDKETCFAEEGKKLVAASQAALGL

SEQ ID NO: 110 - protein, 985 aa, Artificial Sequence
  Synthetic construct
TGSHLVKCAEKEKTFCVNGGECFMVKDLSNPSRYLCKCQPGFTGARCTENVPMKVQNQEKAEELYQKGSGGGSGDAHKSEVAHRFKDLGEENFKALVLIAFAQYLQQSPFEDHVKLVNEVTEFAKTCVADESAENCDKSLHTLFGDKLCTVATLRETYGEMADCCAKQEPERNECFLQHKDDNPNLPRLVRPEVDVMCTAFHDNEETFLKKYLYEIARRHPYFYAPELLFFAKRYKAAFTECCQAADKAACLLPKLDELRDEGKASSAKQRLKCASLQKFGERAFKAWAVARLSQRFPKAEFAEVSKLVTDLTKVHTECCHGDLLECADDRADLAKYICENQDSISSKLKECCEKPLLEKSHCIAEVENDEMPADLPSLAADFVESKDVCKNYAEAKDVFLGMFLYEYARRHPDYSVVLLLRLAKTYETTLEKCCAAADPHECYAKVFDEFKPLVEEPQNLIKQNCELFEQLGEYKFQNALLVRYTKKVPQVSTPTLVEVSRNLGKVGSKCCKHPEAKRMPCAEDYLSVVLNQLCVLHEKTPVSDRVTKCCTESLVNRRPCFSALEVDETYVPKEFQAETFTFHADICTLSEKERQIKKQTALVELVKHKPKATKEQLKAVMDDFAAFVEKCCKADDKETCFAEEGKKLVAASQAALGLGSGGGSGAQVLRGTVTDFPGFDERADAETLRKAMKGLGTDEESILTLLTSRSNAQRQEISAAFKTLFGADLLDDLASELTGKFEKLIVALMKPSRLYDAYELKHALAGAGTNEKVLTEIIASRTPEELRAIKQVYEEEYGSSLAGDVVGDTSGYYQRMLVVLLQAARDPDAGIDEAQVEQDAQALFQAGELKWGTDEEKFITIFGTRSVSHLRKVFDKYMTISGFQIEETIDRETSGNLEQLLLAVVKSIRSIPAYLAETLYYAMKGAGTDDHTLIRVMVSRSEIDLFNIRKEFRKNFATSLYSMIKGDTSGDYKKALLLLCGEDD

SEQ ID NO: 111 - DNA, 2055 bp, Artificial Sequence
  Synthetic construct
atgttcccagccatgcccttgtccagcctgtttgttaacggcccaagaacactttgtggagccgaactggtggatgctctccaattcgtttgcggcgaccgcggattctactttaacaagcccaccggttacgggtcttcaagccggagggccccgcagactggcatcgtcgacgagtgctgttttagaagctgcgatctgcgacggttggagatgtattgtgcacctctgaagcccgcgaaaagtgctggttccggagggagcggtggtgggagtggcggatctggtggaggagacgctcacaagtctgaagtggcacataggttcaaagatctgggcgaagagaactttaaggccctcgtcctgatcgctttcgcacagtacctccagcagtctccctttgaagatcacgtgaaactggtcaatgaggtgaccgaatttgccaagacatgcgtggctgatgagagtgcagaaaactgtgacaaatcactgcatactctctttggagataagctgtgcaccgtcgccacactcagagagacttatggggaaatggctgactgttgcgcaaaacaggagcctgaacggaatgagtgtttcctccagcacaaggatgacaacccaaatctgccccgcctcgtgcgacctgaggtcgatgtgatgtgcaccgcctttcatgacaacgaagagacattcctgaagaaatacctgtatgaaattgctcgtaggcacccatacttttatgcccccgagctcctgttctttgcaaagagatacaaagctgccttcactgaatgttgccaggcagctgataaggccgcatgtctcctgcctaaactggacgagctccgggatgaaggtaaggcttccagcgccaaacagcgcctgaagtgcgcttctctccagaagtttggcgagcgagcattcaaagcctgggctgtggcccgtctcagtcagaggtttccaaaggcagaatttgctgaggtgtcaaaactggtgaccgacctcacaaaggtccatactgagtgttgccacggagatctgctggaatgtgccgacgatagagcagacctcgctaaatatatctgcgagaatcaggattccattagctctaagctgaaagaatgttgcgagaagcccctcctggaaaagagtcattgtatcgccgaggtggaaaacgacgagatgccagcagatctgccatcactcgctgccgactttgtggaatccaaagatgtctgcaagaattacgcagaggctaaagacgtgttcctggggatgtttctgtatgagtacgcccggcgtcaccccgattatagcgtcgtgctcctgctccgactggcaaagacctacgaaacaactctggagaaatgttgcgctgccgcagaccctcatgaatgttatgctaaggtgttcgatgagtttaagccactcgtcgaagagccccagaacctgattaaacagaattgcgaactgttcgagcagctcggtgaatacaagtttcagaacgccctgctcgtgcgttataccaaaaaggtccctcaggtgtctacaccaactctggtggaggtcagtaggaatctgggcaaagtgggatcaaagtgttgcaaacaccccgaggcaaagagaatgccttgtgctgaagattacctctccgtcgtgctgaaccagctctgcgtgctgcatgaaaagaccccagtcagcgaccgggtgacaaaatgttgcaccgaatctctggtcaatcgccgaccctgtttcagtgccctcgaagtggacgaaacttatgtgcctaaggagtttcaggctggaacattcacctttcacgccgatatctgcactctgtccgagaaagaaaggcagattaagaaacagacagcactggtcgagctcgtgaagcataaaccaaaggctaccaaggagcagctgaaagccgccatggacgatttcgcagcttttgtggaaaagtgttgcaaagccgacgataaggagacttgtttcgcagaagaggggaaaaagctcgtggctgccagccaggcagctctgggtctgtaatga

SEQ ID NO: 112 - DNA, 3009 bp, Artificial Sequence
  Synthetic construct
atgttcccagccatgcccttgtccagcctgtttgttaacggcccaagaacactttgtggagccgaactggtggatgctctccaattcgtttgcggcgaccgcggattcctctttaacaagcccaccggtgccgggtcttcaagccggagggccccgcagactggcatcgtcgacgagtgctgttttagaagctgcgatctgcgacggttggagatgtattgtgcacctctgaagcccgcgaaaagtgctgggagcggtggtgggagtggcgacgctcacaagtctgaagtggcacataggttcaaagatctgggcgaagagaactttaaggccctcgtcctgatcgctttcgcacagtacctccagcagtctccctttgaagatcacgtgaaactggtcaatgaggtgaccgaatttgccaagacatgcgtggctgatgagagtgcagaaaactgtgacaaatcactgcatactctctttggagataagctgtgcaccgtcgccacactcagagagacttatggggaaatggctgactgttgcgcaaaacaggagcctgaacggaatgagtgtttcctccagcacaaggatgacaacccaaatctgccccgcctcgtgcgacctgaggtcgatgtgatgtgcaccgcctttcatgacaacgaagagacattcctgaagaaatacctgtatgaaattgctcgtaggcacccatacttttatgcccccgagctcctgttctttgcaaagagatacaaagctgccttcactgaatgttgccaggcagctgataaggccgcatgtctcctgcctaaactggacgagctccgggatgaaggtaaggcttccagcgccaaacagcgcctgaagtgcgcttctctccagaagtttggcgagcgagcattcaaagcctgggctgtggcccgtctcagtcagaggtttccaaaggcagaatttgctgaggtgtcaaaactggtgaccgacctcacaaaggtccatactgagtgttgccacggagatctgctggaatgtgccgacgatagagcagacctcgctaaatatatctgcgagaatcaggattccattagctctaagctgaaagaatgttgcgagaagcccctcctggaaaagagtcattgtatcgccgaggtggaaaacgacgagatgccagcagatctgccatcactcgctgccgactttgtggaatccaaagatgtctgcaagaattacgcagaggctaaagacgtgttcctggggatgtttctgtatgagtacgcccggcgtcaccccgattatagcgtcgtgctcctgctccgactggcaaagacctacgaaacaactctggagaaatgttgcgctgccgcagaccctcatgaatgttatgctaaggtgttcgatgagtttaagccactcgtcgaagagccccagaacctgattaaacagaattgcgaactgttcgagcagctcggtgaatacaagtttcagaacgccctgctcgtgcgttataccaaaaaggtccctcaggtgtctacaccaactctggtggaggtcagtaggaatctgggcaaagtgggatcaaagtgttgcaaacaccccgaggcaaagagaatgccttgtgctgaagattacctctccgtcgtgctgaaccagctctgcgtgctgcatgaaaagaccccagtcagcgaccgggtgacaaaatgttgcaccgaatctctggtcaatcgccgaccctgtttcagtgccctcgaagtggacgaaacttatgtgcctaaggagtttcaggctggaacattcacctttcacgccgatatctgcactctgtccgagaaagaaaggcagattaagaaacagacagcactggtcgagctcgtgaagcataaaccaaaggctaccaaggagcagctgaaagccgccatggacgatttcgcagcttttgtggaaaagtgttgcaaagccgacgataaggagacttgtttcgcagaagaggggaaaaagctcgtggctgccagccaggcagctctgggtctggggagcggtggtgggagtggcgctcaagtcttgcgtggtacggtgacagacttcccaggcttcgatgaaagagcggacgcggaaacacttcgaaaggcgatgaaagggctcggtactgacgaagagtccattttgacccttcttacgagcaggtcaaacgctcagaggcaagaaatctctgcagcctttaagacactctttggagctgaccttcttgatgacctcgcatctgagctgacgggaaagtttgagaaactcatcgtagctttgatgaagcccagccgattgtatgatgcttacgaactgaaacacgccctggctggagcgggaacgaacgagaaagttttgactgagatcatcgcatcgcggaccccggaagagctcagagccatcaaacaagtctacgaggaggagtacggatcgtcattggcaggagacgtggtgggggatacgtcgggttactaccaacgaatgcttgtcgtgcttttgcaggcagctcgcgacccggatgcggggatcgacgaggcccaagtggagcaagatgcgcaagcactcttccaggccggtgaactcaaatgggggaccgatgaagagaagtttatcaccatctttggcacgaggagtgtaagtcatctgcgtaaagtattcgataagtatatgacaatctcagggtttcagattgaggagacaattgacagggaaacctccggtaacttggagcagctcttgcttgccgtcgtcaagtccattcgctcgatccctgcgtatctggctgaaacactgtattacgccatgaaaggggcaggcactgatgaccacaccttgattagagttatggtgtcgcgatcagaaattgacttgttcaatatccggaaagagttccggaagaatttcgcaacgagcctctatagcatgatcaaaggggacacttcgggagattacaagaaagcgttgctccttctttgcggagaggatgactaatga

SEQ ID NO: 113 - DNA, 2037 bp, Artificial Sequence
  Synthetic construct
atgttcccagccatgcccttgtccagcctgtttgttaacggcccaagaacactttgtggagccgaactggtggatgctctccaattcgtttgcggcgaccgcggattctactttaacaagcccaccggtgccgggtcttcaagccggagggccccgcagactggcatcgtcgacgagtgctgttttagaagctgcgatctgcgacggttggagatgtattgtgcacctctgaagcccgcgaaaagtgctgggagcggtggtgggagtggcgacgctcacaagtctgaagtggcacataggttcaaagatctgggcgaagagaactttaaggccctcgtcctgatcgctttcgcacagtacctccagcagtctccctttgaagatcacgtgaaactggtcaatgaggtgaccgaatttgccaagacatgcgtggctgatgagagtgcagaaaactgtgacaaatcactgcatactctctttggagataagctgtgcaccgtcgccacactcagagagacttatggggaaatggctgactgttgcgcaaaacaggagcctgaacggaatgagtgtttcctccagcacaaggatgacaacccaaatctgccccgcctcgtgcgacctgaggtcgatgtgatgtgcaccgcctttcatgacaacgaagagacattcctgaagaaatacctgtatgaaattgctcgtaggcacccatacttttatgcccccgagctcctgttctttgcaaagagatacaaagctgccttcactgaatgttgccaggcagctgataaggccgcatgtctcctgcctaaactggacgagctccgggatgaaggtaaggcttccagcgccaaacagcgcctgaagtgcgcttctctccagaagtttggcgagcgagcattcaaagcctgggctgtggcccgtctcagtcagaggtttccaaaggcagaatttgctgaggtgtcaaaactggtgaccgacctcacaaaggtccatactgagtgttgccacggagatctgctggaatgtgccgacgatagagcagacctcgctaaatatatctgcgagaatcaggattccattagctctaagctgaaagaatgttgcgagaagcccctcctggaaaagagtcattgtatcgccgaggtggaaaacgacgagatgccagcagatctgccatcactcgctgccgactttgtggaatccaaagatgtctgcaagaattacgcagaggctaaagacgtgttcctggggatgtttctgtatgagtacgcccggcgtcaccccgattatagcgtcgtgctcctgctccgactggcaaagacctacgaaacaactctggagaaatgttgcgctgccgcagaccctcatgaatgttatgctaaggtgttcgatgagtttaagccactcgtcgaagagccccagaacctgattaaacagaattgcgaactgttcgagcagctcggtgaatacaagtttcagaacgccctgctcgtgcgttataccaaaaaggtccctcaggtgtctacaccaactctggtggaggtcagtaggaatctgggcaaagtgggatcaaagtgttgcaaacaccccgaggcaaagagaatgccttgtgctgaagattacctctccgtcgtgctgaaccagctctgcgtgctgcatgaaaagaccccagtcagcgaccgggtgacaaaatgttgcaccgaatctctggtcaatcgccgaccctgtttcagtgccctcgaagtggacgaaacttatgtgcctaaggagtttcaggctgaaacattcacctttcacgccgatatctgcactctgtccgagaaagaaaggcagattaagaaacagacagcactggtcgagctcgtgaagcataaaccaaaggctaccaaggagcagctgaaagccgtcatggacgatttcgcagcttttgtggaaaagtgttgcaaagccgacgataaggagacttgtttcgcagaagaggggaaaaagctcgtggctgccagccaggcagctctgggtctgtaatgaggatcc

SEQ ID NO: 114 - DNA, 2961 bp, Artificial Sequence
  Synthetic construct
accggtagccaccttgtgaaatgtgcggagaaagaaaagacattctgtgttaatggcggggagtgcttcatggtaaaagacctgtcgaatccgtcaagatatctctgcaaatgccagcccggttttacgggagcccgatgtaccgagaacgtgcctatgaaagtccaaaaccaggaaaaggcagaagaattgtaccaaaaggggagcggtggtgggagtggcgacgctcacaagtctgaagtggcacataggttcaaagatctgggcgaagagaactttaaggccctcgtcctgatcgctttcgcacagtacctccagcagtctccctttgaagatcacgtgaaactggtcaatgaggtgaccgaatttgccaagacatgcgtggctgatgagagtgcagaaaactgtgacaaatcactgcatactctctttggagataagctgtgcaccgtcgccacactcagagagacttatggggaaatggctgactgttgcgcaaaacaggagcctgaacggaatgagtgtttcctccagcacaaggatgacaacccaaatctgccccgcctcgtgcgacctgaggtcgatgtgatgtgcaccgcctttcatgacaacgaagagacattcctgaagaaatacctgtatgaaattgctcgtaggcacccatacttttatgcccccgagctcctgttctttgcaaagagatacaaagctgccttcactgaatgttgccaggcagctgataaggccgcatgtctcctgcctaaactggacgagctccgggatgaaggtaaggcttccagcgccaaacagcgcctgaagtgcgcttctctccagaagtttggcgagcgagcattcaaagcctgggctgtggcccgtctcagtcagaggtttccaaaggcagaatttgctgaggtgtcaaaactggtgaccgacctcacaaaggtccatactgagtgttgccacggagatctgctggaatgtgccgacgatagagcagacctcgctaaatatatctgcgagaatcaggattccattagctctaagctgaaagaatgttgcgagaagcccctcctggaaaagagtcattgtatcgccgaggtggaaaacgacgagatgccagcagatctgccatcactcgctgccgactttgtggaatccaaagatgtctgcaagaattacgcagaggctaaagacgtgttcctggggatgtttctgtatgagtacgcccggcgtcaccccgattatagcgtcgtgctcctgctccgactggcaaagacctacgaaacaactctggagaaatgttgcgctgccgcagaccctcatgaatgttatgctaaggtgttcgatgagtttaagccactcgtcgaagagccccagaacctgattaaacagaattgcgaactgttcgagcagctcggtgaatacaagtttcagaacgccctgctcgtgcgttataccaaaaaggtccctcaggtgtctacaccaactctggtggaggtcagtaggaatctgggcaaagtgggatcaaagtgttgcaaacaccccgaggcaaagagaatgccttgtgctgaagattacctctccgtcgtgctgaaccagctctgcgtgctgcatgaaaagaccccagtcagcgaccgggtgacaaaatgttgcaccgaatctctggtcaatcgccgaccctgtttcagtgccctcgaagtggacgaaacttatgtgcctaaggagtttcaggctgaaacattcacctttcacgccgatatctgcactctgtccgagaaagaaaggcagattaagaaacagacagcactggtcgagctcgtgaagcataaaccaaaggctaccaaggagcagctgaaagccgtcatggacgatttcgcagcttttgtggaaaagtgttgcaaagccgacgataaggagacttgtttcgcagaagaggggaaaaagctcgtggctgccagccaggcagctctgggtctggggagcggtggtgggagtggcgctcaagtcttgcgtggtacggtgacagacttcccaggcttcgatgaaagagcggacgcggaaacacttcgaaaggcgatgaaagggctcggtactgacgaagagtccattttgacccttcttacgagcaggtcaaacgctcagaggcaagaaatctctgcagcctttaagacactctttggagctgaccttcttgatgacctcgcatctgagctgacgggaaagtttgagaaactcatcgtagctttgatgaagcccagccgattgtatgatgcttacgaactgaaacacgccctggctggagcgggaacgaacgagaaagttttgactgagatcatcgcatcgcggaccccggaagagctcagagccatcaaacaagtctacgaggaggagtacggatcgtcattggcaggagacgtggtgggggatacgtcgggttactaccaacgaatgcttgtcgtgcttttgcaggcagctcgcgacccggatgcggggatcgacgaggcccaagtggagcaagatgcgcaagcactcttccaggccggtgaactcaaatgggggaccgatgaagagaagtttatcaccatctttggcacgaggagtgtaagtcatctgcgtaaagtattcgataagtatatgacaatctcagggtttcagattgaggagacaattgacagggaaacctccggtaacttggagcagctcttgcttgccgtcgtcaagtccattcgctcgatccctgcgtatctggctgaaacactgtattacgccatgaaaggggcaggcactgatgaccacaccttgattagagttatggtgtcgcgatcagaaattgacttgttcaatatccggaaagagttccggaagaatttcgcaacgagcctctatagcatgatcaaaggggacacttcgggagattacaagaaagcgttgctccttctttgcggagaggatgactgataa

SEQ ID NO: 115 - DNA, 678 bp, Artificial Sequence
  Synthetic construct
gataagacccatacatgccctccgtgccccgcaccggaactcttgggtggcccatcagtctttctgttcccgccaaagcccaaagacacactgatgatttcgcgcacgcccgaagtcacttgcgtcgtggtggatgtgtcgcatgaggacccggaggtcaagttcaactggtacgtcgatggtgtagaagtccacaacgccaagaccaagcctcgggaggagcagtatcagtccacctaccgggtagtgagcgtgcttacagtgctccatcaggactggctgaacggcaaagaatacaaatgcaaagtcagcaacaaagcgctgccagcgcccatcgagaaaacaattagcaaagcgaaagggcagcccagagaacctcaagtgtatacattgccgccgtcgcgggaggaaatgacaaagaatcaggtatccctgacgtgtcttgtgaaaggcttttacccatccgacattgcggtagagtgggagtcgaatgggcaacccgagaacaactataagacgactcccccagtcttggattcagacggatcctttttcttgtactcgaaactcacagtcgacaagtccagatggcagcaggggaacgtgttcagctgcagcgtgatgcacgaggcccttcacaaccactatacgcagaaatcattaagcttatcgcctggg

SEQ ID NO: 116 - protein, 1001 aa, Artificial Sequence
  Synthetic construct
MFPAMPLSSLFVNGPRTLCGAELVDALQFVCGDRGFYFNKPTGAGSSSRRAPQTGIVDECCFRSCDLRRLEMYCAPLKPAKSAGSGGGSGDAHKSEVAHRFKDLGEENFKALVLIAFAQYLQQSPFEDHVKLVNEVTEFAKTCVADESAENCDKSLHTLFGDKLCTVATLRETYGEMADCCAKQEPERNECFLQHKDDNPNLPRLVRPEVDVMCTAFHDNEETFLKKYLYEIARRHPYFYAPELLFFAKRYKAAFTECCQAADKAACLLPKLDELRDEGKASSAKQRLKCASLQKFGERAFKAWAVARLSQRFPKAEFAEVSKLVTDLTKVHTECCHGDLLECADDRADLAKYICENQDSISSKLKECCEKPLLEKSHCIAEVENDEMPADLPSLAADFVESKDVCKNYAEAKDVFLGMFLYEYARRHPDYSVVLLLRLAKTYETTLEKCCAAADPHECYAKVFDEFKPLVEEPQNLIKQNCELFEQLGEYKFQNALLVRYTKKVPQVSTPTLVEVSRNLGKVGSKCCKHPEAKRMPCAEDYLSVVLNQLCVLHEKTPVSDRVTKCCTESLVNRRPCFSALEVDETYVPKEFQAETFTFHADICTLSEKERQIKKQTALVELVKHKPKATKEQLKAVMDDFAAFVEKCCKADDKETCFAEEGKKLVAASQAALGLGSGGGSGAQVLRGTVTDFPGFDERADAETLRKAMKGLGTDEESILTLLTSRSNAQRQEISAAFKTLFGRDLLDDLKSELTGKFEKLIVALMKPSRLYDAYELKHALKGAGTNEKVLTEIIASRTPEELRAIKQVYEEEYGSSLEDDVVGDTSGYYQRMLVVLLQANRDPDAGIDEAQVEQDAQALFQAGELKWGTDEEKFITIFGTRSVSHLRKVFDKYMTISGFQIEETIDRETSGNLEQLLLAVVKSIRSIPAYLAETLYYAMKGAGTDDHTLIRVMVSRSEIDLFNIRKEFRKNFATSLYSMIKGDTSGDYKKALLLLCGEDD

SEQ ID NO: 117 - DNA, 3009 bp, Artificial Sequence
  Synthetic construct
atgttcccagccatgcccttgtccagcctgtttgttaacggcccaagaacactttgtggagccgaactggtggatgctctccaattcgtttgcggcgaccgcggattctactttaacaagcccaccggtgccgggtcttcaagccggagggccccgcagactggcatcgtcgacgagtgctgttttagaagctgcgatctgcgacggttggagatgtattgtgcacctctgaagcccgcgaaaagtgctgggagcggtggtgggagtggcgacgctcacaagtctgaagtggcacataggttcaaagatctgggcgaagagaactttaaggccctcgtcctgatcgctttcgcacagtacctccagcagtctccctttgaagatcacgtgaaactggtcaatgaggtgaccgaatttgccaagacatgcgtggctgatgagagtgcagaaaactgtgacaaatcactgcatactctctttggagataagctgtgcaccgtcgccacactcagagagacttatggggaaatggctgactgttgcgcaaaacaggagcctgaacggaatgagtgtttcctccagcacaaggatgacaacccaaatctgccccgcctcgtgcgacctgaggtcgatgtgatgtgcaccgcctttcatgacaacgaagagacattcctgaagaaatacctgtatgaaattgctcgtaggcacccatacttttatgcccccgagctcctgttctttgcaaagagatacaaagctgccttcactgaatgttgccaggcagctgataaggccgcatgtctcctgcctaaactggacgagctccgggatgaaggtaaggcttccagcgccaaacagcgcctgaagtgcgcttctctccagaagtttggcgagcgagcattcaaagcctgggctgtggcccgtctcagtcagaggtttccaaaggcagaatttgctgaggtgtcaaaactggtgaccgacctcacaaaggtccatactgagtgttgccacggagatctgctggaatgtgccgacgatagagcagacctcgctaaatatatctgcgagaatcaggattccattagctctaagctgaaagaatgttgcgagaagcccctcctggaaaagagtcattgtatcgccgaggtggaaaacgacgagatgccagcagatctgccatcactcgctgccgactttgtggaatccaaagatgtctgcaagaattacgcagaggctaaagacgtgttcctggggatgtttctgtatgagtacgcccggcgtcaccccgattatagcgtcgtgctcctgctccgactggcaaagacctacgaaacaactctggagaaatgttgcgctgccgcagaccctcatgaatgttatgctaaggtgttcgatgagtttaagccactcgtcgaagagccccagaacctgattaaacagaattgcgaactgttcgagcagctcggtgaatacaagtttcagaacgccctgctcgtgcgttataccaaaaaggtccctcaggtgtctacaccaactctggtggaggtcagtaggaatctgggcaaagtgggatcaaagtgttgcaaacaccccgaggcaaagagaatgccttgtgctgaagattacctctccgtcgtgctgaaccagctctgcgtgctgcatgaaaagaccccagtcagcgaccgggtgacaaaatgttgcaccgaatctctggtcaatcgccgaccctgtttcagtgccctcgaagtggacgaaacttatgtgcctaaggagtttcaggctgaaacattcacctttcacgccgatatctgcactctgtccgagaaagaaaggcagattaagaaacagacagcactggtcgagctcgtgaagcataaaccaaaggctaccaaggagcagctgaaagccgtcatggacgatttcgcagcttttgtggaaaagtgttgcaaagccgacgataaggagacttgtttcgcagaagaggggaaaaagctcgtggctgccagccaggcagctctgggtctggggagcggtggtgggagtggcgctcaagtcttgcgtggtacggtgacagacttcccaggcttcgatgaaagagcggacgcggaaacacttcgaaaggcgatgaaagggctcggtactgacgaagagtccattttgacccttcttacgagcaggtcaaacgctcagaggcaagaaatctctgcagcctttaagacactctttggacgtgaccttcttgatgacctcaaatctgagctgacgggaaagtttgagaaactcatcgtagctttgatgaagcccagccgattgtatgatgcttacgaactgaaacacgccctgaaaggagcgggaacgaacgagaaagttttgactgagatcatcgcatcgcggaccccggaagagctcagagccatcaaacaagtctacgaggaggagtacggatcgtcattggaagatgacgtggtgggggatacgtcgggttactaccaacgaatgcttgtcgtgcttttgcaggcaaatcgcgacccggatgcggggatcgacgaggcccaagtggagcaagatgcgcaagcactcttccaggccggtgaactcaaatgggggaccgatgaagagaagtttatcaccatctttggcacgaggagtgtaagtcatctgcgtaaagtattcgataagtatatgacaatctcagggtttcagattgaggagacaattgacagggaaacctccggtaacttggagcagctcttgcttgccgtcgtcaagtccattcgctcgatccctgcgtatctggctgaaacactgtattacgccatgaaaggggcaggcactgatgaccacaccttgattagagttatggtgtcgcgatcagaaattgacttgttcaatatccggaaagagttccggaagaatttcgcaacgagcctctatagcatgatcaaaggggacacttcgggagattacaagaaagcgttgctccttctttgcggagaggatgactgataa

SEQ ID NO: 118 - protein, 988 aa, Artificial Sequence
  Synthetic construct
GPRTLCGAELVDALQFVCGDRGFYFNKPTGAGSSSRRAPQTGIVDECCFRSCDLRRLEMYCAPLKPAKSAGSGGGSGDAHKSEVAHRFKDLGEENFKALVLIAFAQYLQQSPFEDHVKLVNEVTEFAKTCVADESAENCDKSLHTLFGDKLCTVATLRETYGEMADCCAKQEPERNECFLQHKDDNPNLPRLVRPEVDVMCTAFHDNEETFLKKYLYEIARRHPYFYAPELLFFAKRYKAAFTECCQAADKAACLLPKLDELRDEGKASSAKQRLKCASLQKFGERAFKAWAVARLSQRFPKAEFAEVSKLVTDLTKVHTECCHGDLLECADDRADLAKYICENQDSISSKLKECCEKPLLEKSHCIAEVENDEMPADLPSLAADFVESKDVCKNYAEAKDVFLGMFLYEYARRHPDYSVVLLLRLAKTYETTLEKCCAAADPHECYAKVFDEFKPLVEEPQNLIKQNCELFEQLGEYKFQNALLVRYTKKVPQVSTPTLVEVSRNLGKVGSKCCKHPEAKRMPCAEDYLSVVLNQLCVLHEKTPVSDRVTKCCTESLVNRRPCFSALEVDETYVPKEFQAETFTFHADICTLSEKERQIKKQTALVELVKHKPKATKEQLKAVMDDFAAFVEKCCKADDKETCFAEEGKKLVAASQAALGLGSGGGSGAQVLRGTVTDFPGFDERADAETLRKAMKGLGTDEESILTLLTSRSNAQRQEISAAFKTLFGADLLDDLASELTGKFEKLIVALMKPSRLYDAYELKHALAGAGTNEKVLTEIIASRTPEELRAIKQVYEEEYGSSLAGDVVGDTSGYYQRMLVVLLQAARDPDAGIDEAQVEQDAQALFQAGELKWGTDEEKFITIFGTRSVSHLRKVFDKYMTISGFQIEETIDRETSGNLEQLLLAVVKSIRSIPAYLAETLYYAMKGAGTDDHTLIRVMVSRSEIDLFNIRKEFRKNFATSLYSMIKGDTSGDYKKALLLLAGEDD

SEQ ID NO: 119 - DNA, 3043 bp, Artificial Sequence
  Synthetic construct
atggcctggcggctgtggtggctgctgctcctgctcctgttgctttggcctatggtgtgggccggcccaagaacactttgtggagccgaactggtggatgctctccaattcgtttgcggcgaccgcggattctactttaacaagcccaccggtgccgggtcttcaagccggagggccccgcagactggcatcgtcgacgagtgctgttttagaagctgcgatctgcgacggttggagatgtattgtgcacctctgaagcccgcgaaaagtgctgggagcggtggtgggagtggcgacgctcacaagtctgaagtggcacataggttcaaagatctgggcgaagagaactttaaggccctcgtcctgatcgctttcgcacagtacctccagcagtctccctttgaagatcacgtgaaactggtcaatgaggtgaccgaatttgccaagacatgcgtggctgatgagagtgcagaaaactgtgacaaatcactgcatactctctttggagataagctgtgcaccgtcgccacactcagagagacttatggggaaatggctgactgttgcgcaaaacaggagcctgaacggaatgagtgtttcctccagcacaaggatgacaacccaaatctgccccgcctcgtgcgacctgaggtcgatgtgatgtgcaccgcctttcatgacaacgaagagacattcctgaagaaatacctgtatgaaattgctcgtaggcacccatacttttatgcccccgagctcctgttctttgcaaagagatacaaagctgccttcactgaatgttgccaggcagctgataaggccgcatgtctcctgcctaaactggacgagctccgggatgaaggtaaggcttccagcgccaaacagcgcctgaagtgcgcttctctccagaagtttggcgagcgagcattcaaagcctgggctgtggcccgtctcagtcagaggtttccaaaggcagaatttgctgaggtgtcaaaactggtgaccgacctcacaaaggtccatactgagtgttgccacggagatctgctggaatgtgccgacgatagagcagacctcgctaaatatatctgcgagaatcaggattccattagctctaagctgaaagaatgttgcgagaagcccctcctggaaaagagtcattgtatcgccgaggtggaaaacgacgagatgccagcagatctgccatcactcgctgccgactttgtggaatccaaagatgtctgcaagaattacgcagaggctaaagacgtgttcctggggatgtttctgtatgagtacgcccggcgtcaccccgattatagcgtcgtgctcctgctccgactggcaaagacctacgaaacaactctggagaaatgttgcgctgccgcagaccctcatgaatgttatgctaaggtgttcgatgagtttaagccactcgtcgaagagccccagaacctgattaaacagaattgcgaactgttcgagcagctcggtgaatacaagtttcagaacgccctgctcgtgcgttataccaaaaaggtccctcaggtgtctacaccaactctggtggaggtcagtaggaatctgggcaaagtgggatcaaagtgttgcaaacaccccgaggcaaagagaatgccttgtgctgaagattacctctccgtcgtgctgaaccagctctgcgtgctgcatgaaaagaccccagtcagcgaccgggtgacaaaatgttgcaccgaatctctggtcaatcgccgaccctgtttcagtgccctcgaagtggacgaaacttatgtgcctaaggagtttcaggctgaaacattcacctttcacgccgatatctgcactctgtccgagaaagaaaggcagattaagaaacagacagcactggtcgagctcgtgaagcataaaccaaaggctaccaaggagcagctgaaagccgtcatggacgatttcgcagcttttgtggaaaagtgttgcaaagccgacgataaggagacttgtttcgcagaagaggggaaaaagctcgtggctgccagccaggcagctctgggtctggggagcggtggtgggagtggcgctcaagtcttgcgtggtacggtgacagacttcccaggcttcgatgaaagagcggacgcggaaacacttcgaaaggcgatgaaagggctcggtactgacgaagagtccattttgacccttcttacgagcaggtcaaacgctcagaggcaagaaatctctgcagcctttaagacactctttggagctgaccttcttgatgacctcgcatctgagctgacgggaaagtttgagaaactcatcgtagctttgatgaagcccagccgattgtatgatgcttacgaactgaaacacgccctggctggagcgggaacgaacgagaaagttttgactgagatcatcgcatcgcggaccccggaagagctcagagccatcaaacaagtctacgaggaggagtacggatcgtcattggcaggagacgtggtgggggatacgtcgggttactaccaacgaatgcttgtcgtgcttttgcaggcagctcgcgacccggatgcggggatcgacgaggcccaagtggagcaagatgcgcaagcactcttccaggccggtgaactcaaatgggggaccgatgaagagaagtttatcaccatctttggcacgaggagtgtaagtcatctgcgtaaagtattcgataagtatatgacaatctcagggtttcagattgaggagacaattgacagggaaacctccggtaacttggagcagctcttgcttgccgtcgtcaagtccattcgctcgatccctgcgtatctggctgaaacactgtattacgccatgaaaggggcaggcactgatgaccacaccttgattagagttatggtgtcgcgatcagaaattgacttgttcaatatccggaaagagttccggaagaatttcgcaacgagcctctatagcatgatcaaaggggacacttcgggagattacaagaaagcgttgctccttcttgccggagaggatgactgataaggatcctagc

SEQ ID NO: 120 - protein, 70 aa, Artificial Sequence
  Synthetic construct
GPRTLCGAELVDALQFVCGDRGFYFNKPTGAGSSSRRAPQTGIVDECCFRSCDLRRLEMYCAPLKPAKSA

SEQ ID NO: 121 - DNA, 210 bp, Artificial Sequence
  Synthetic construct
ggcccaagaacactttgtggagccgaactggtggatgctctccaattcgtttgcggcgaccgcggattctactttaacaagcccaccggtgccgggtcttcaagccggagggccccgcagactggcatcgtcgacgagtgctgttttagaagctgcgatctgcgacggttggagatgtattgtgcacctctgaagcccgcgaaaagtgct

SEQ ID NO: 122 - protein, 319 aa, Artificial Sequence
  Synthetic construct
AQVLRGTVTDFPGFDERADAETLRKAMKGLGTDEESILTLLTSRSNAQRQEISAAFKTLFGADLLDDLASELTGKFEKLIVALMKPSRLYDAYELKHALAGAGTNEKVLTEIIASRTPEELRAIKQVYEEEYGSSLAGDVVGDTSGYYQRMLVVLLQAARDPDAGIDEAQVEQDAQALFQAGELKWGTDEEKFITIFGTRSVSHLRKVFDKYMTISGFQIEETIDRETSGNLEQLLLAVVKSIRSIPAYLAETLYYAMKGAGTDDHTLIRVMVSRSEIDLFNIRKEFRKNFATSLYSMIKGDTSGDYKKALLLLAGEDD

SEQ ID NO: 123 - DNA, 957 bp, Artificial Sequence
  Synthetic construct
gctcaagtcttgcgtggtacggtgacagacttcccaggcttcgatgaaagagcggacgcggaaacacttcgaaaggcgatgaaagggctcggtactgacgaagagtccattttgacccttcttacgagcaggtcaaacgctcagaggcaagaaatctctgcagcctttaagacactctttggagctgaccttcttgatgacctcgcatctgagctgacgggaaagtttgagaaactcatcgtagctttgatgaagcccagccgattgtatgatgcttacgaactgaaacacgccctggctggagcgggaacgaacgagaaagttttgactgagatcatcgcatcgcggaccccggaagagctcagagccatcaaacaagtctacgaggaggagtacggatcgtcattggcaggagacgtggtgggggatacgtcgggttactaccaacgaatgcttgtcgtgcttttgcaggcagctcgcgacccggatgcggggatcgacgaggcccaagtggagcaagatgcgcaagcactcttccaggccggtgaactcaaatgggggaccgatgaagagaagtttatcaccatctttggcacgaggagtgtaagtcatctgcgtaaagtattcgataagtatatgacaatctcagggtttcagattgaggagacaattgacagggaaacctccggtaacttggagcagctcttgcttgccgtcgtcaagtccattcgctcgatccctgcgtatctggctgaaacactgtattacgccatgaaaggggcaggcactgatgaccacaccttgattagagttatggtgtcgcgatcagaaattgacttgttcaatatccggaaagagttccggaagaatttcgcaacgagcctctatagcatgatcaaaggggacacttcgggagattacaagaaagcgttgctccttcttgccggagaggatgac

SEQ ID NO: 124 - protein, 585 aa, Artificial Sequence; identical to SEQ ID NO: 55
  Synthetic construct

SEQ ID NO: 125 - DNA, 1755 bp, Artificial Sequence; identical to SEQ ID NO: 58
  Synthetic construct

SEQ ID NO: 126 - protein, 7 aa, Artificial Sequence
  Synthetic construct
GEGGGEG

SEQ ID NO: 127 - protein, 7 aa, Artificial Sequence
  Synthetic construct
AAALAAA

SEQ ID NO: 128 - protein, 245 aa, Artificial Sequence
  Synthetic construct
EVQLQQSGPELVKPGASMKISCKASGYSFTGYTMKWVKQSHGKNLEWIGLINPYNGGTSYNQKFKGKATLTVDKSSSTAYMELLSLTSDDSAVYYCAREGDYDGAMDYWGQGTSVTVSGGGGSGGGGSGGGGSGGGGSGGSDIQMTQSPSSLSASLGGKVTITCKSSQDINKYIAWYQHKPGKGPGLLIHYTSTLQPGIPSRFSGSGSGRDYSFSISNLDPENIAAYYCLQYDNLYTFGGGTRLE

SEQ ID NO: 129 - protein, 249 aa, Artificial Sequence
  Synthetic construct
LESGGGLVQPGGSLRLSCAGSGFTFSSYAMSWVRQAPGKGLEWVSSISGSGGSTYYADSVKGRFTISRDNSKKTLYLQMNSLRAEDTAVYYCARKRGRTTVSWGLVYFDYWGQGTVVTVSSGGGGSGGGGSGGGGSGGGGSGGSELTQSPGTLSLSPGERATLSCRASHSVSRAYLAWYQQKPGQAPRLLIYGTSSRATGIPDRFSGSGSGTDFTLTISRLEPEDFAVYYCQQYGGSPWFGQGTKVELK

SEQ ID NO: 130 - protein, 251 aa, Artificial Sequence
  Synthetic construct
LEQSGGGVVQPGGSLRLSCTASGFTFSSYGMHWVRQAPGKGLEWVTFIRYDGSSKYSADSVKGRFTISRDNSKNTLFLQMNSLRAEDTAVYYCARARWRDYYYYMDVWGKGTTVTVSSGGGGSGGGGSGGGGSGGGGSGGSELTQEPSVSGAPGQRVTISCTGSSSNIGAGYDVHWYQQLPGTAPKLLIYGNSNRPSGVPDRFSGSKSGTSASLAITGLQAEDEADYYCQSYDSSLSGVVFGGGTKLTVLG

SEQ ID NO: 131 - protein, 252 aa, Artificial Sequence
  Synthetic construct
EVQLVESGGGLVQPGGSLRLSCSASGFTFSSYAMHWVRQAPGKGLEYVSAISSNGGSTYYADSVKGRFTISRDNSKNTLYLQMSSLRAEDTAVYYCVKITGAYSSSWYYDNWFDPWGQGTLVTVSSGGGGSGGGGSGGGGSGGSSYELTQPPSVSVSPGQTASITCSGDKLGDKYACWYQQKPGQSPVLVIYQDSKRPSGIPERFSGSNSGNTATLTISGTQAMDEADYYCQAWDSSTAVFGGGTKLTVLGQ

SEQ ID NO: 132 - protein, 247 aa, Artificial Sequence
  Synthetic construct
EVQLVESGGGVVQPGGSLRLFCAASGFTFDGYAMHWVRQAPGKGLEWVSLISGDGGSTYYADSVKGRFTISRDNSKNSLYLQMNSLRAEDTALYYCAKGKVTTIYDRFDIWGQGTMVTVSSGGGGSGGGGSGGGGSGGSDIQMTQSPSSLSASVGDRVTITCRASQGISNYLAWYQQKPGKVPKSLIYAASTLQSGVPSRFSGSGSGTDFTLTISSLQPEDVATYYCQKYNSAPRTFGPGTKLEIKR

SEQ ID NO: 133 - protein, 243 aa, Artificial Sequence
  Synthetic construct
EVQLVESGGGLVQPGGSLRLSCAASGFTFSSYSMNWVRQAPGKGLEWVSYISSTIITIYYADSVKGRFTISRDNAKNSLYLQMNSLRAEDTAVYYCARGDSSEAFDIWGQGTMVTVSLGGGGSGGGGSGGGGSGGSSYELTQPSSVSVSPGQTARITCSGDLLAKKYARWFQQKPGQAPILVIFKDTERPSGIPERFSGSSSGTTVTLTISGAQVEDEADYYCYSASDNNGRVFGGGTKLTVL

SEQ ID NO: 134 - protein, 256 aa, Artificial Sequence
  Synthetic construct
EVQLVESGGGLVKPGGSLRLSCAASGFTFSKAWMSWVRQAPGKGLEWVGRIKSKTDGGTTDYAAPVKGRLTISRDSSKNTLYLRMNSLKTEDTAVYYCTTGITMIIVVITTSSKRTSFEYWGQGTLVTVSSGGGGSGGGGSGGGGSGGSDIQMTQSPSSLSASVGDRVTITCRASQSISNYLNWYQQKPGKAPNLLIYAASSLQSGVPSRFSGSGSGTDFTLTISGLQAEDFATYYCQQSYSALTFGPGTKVDIRR

SEQ ID NO: 135 - protein, 229 aa, Artificial Sequence
  Synthetic construct
GLVKPSQTLSLTCAISGDSVSSNSAAWNCIRPVPSRGLEWLGRTTYRSKWYNDYAVSVKSRITINPDTSKNQFSLQLNSVTPEDTAVYYCASTTLNWGYEKDDAFDIWGQGTMVTVSSGGGGSGGGGSGGGGSGGSQAVLTQPASLSASPGASASLTCTLRSGINVCTPRIYWQGSGVPSRFSGSKNASANAGILLISGLQSEDEADYYCMIWHSSALVFGGGTKLTVL

SEQ ID NO: 136 - protein, 244 aa, Artificial Sequence
  Syntehtic construct
LESGGGLVQPGGSLRLSCAGSGFTFSSYAMSWVRQAPGKGLEWVSSISGSGGSTYYADSVKGRFTISRDNSKKTLYLQMNSLRAEDTAVYYCARKRGRTTVSWGLVYFDYWGQGTVVTVSSGGGGSGGGGSGGGGSGGSELTQSPGTLSLSPGERATLSCRASHSVSRAYLAWYQQKPGQAPRLLIYGTSSRATGIPDRFSGSGSGTDFTLTISRLEPEDFAVYYCQQYGGSPWFGQGTKVELK

SEQ ID NO: 137 - protein, 20 aa, Artificial Sequence
  Synthetic construct
ASPAAPAPASPAAPAPSAPA

SEQ ID NO: 138 - protein, 107 aa, Artificial Sequence
  Synthetic construct
DIQMTQSPSSLSASVGDRVTITCRASQWIGSQLSWYQQKPGKAPKLLIMWRSSLQSGVPSRFSGSGSGTDFTLTISSLQPEDFATYYCAQGAALPRTFGQGTKVEIK